European Patent Application EP 4 596 687 A1, published August 6, 2025. Title: Herpes simplex virus targeted to IL13RA2, and anti-IL13RA2 antibody or antigen-binding fragment thereof. Applicant: 国立大学法人　東京大学. The sequence listing filed with the application follows.

SEQUENCE LISTING (30 sequences)

SEQ ID NO: 1 - protein, 5 aa, synthetic construct
RHGIH

SEQ ID NO: 2 - protein, 16 aa, synthetic construct
VIWAGGSTNYNSALMS

SEQ ID NO: 3 - protein, 8 aa, synthetic construct
DHFDSFDY

SEQ ID NO: 4 - protein, 12 aa, synthetic construct
TASSSVSSSYLH

SEQ ID NO: 5 - protein, 7 aa, synthetic construct
STSNLAS

SEQ ID NO: 6 - protein, 9 aa, synthetic construct
HQYHRSPLT

SEQ ID NO: 7 - protein, 251 aa, synthetic construct
DIVLTQTPAIMSASLGERVTMTCTASSSVSSSYLHWYQQKPGSSPKLWIYSTSNLASGVPLRFSGSGSGTSYSLTISSMEAEDAATYYCHQYHRSPLTFGAGTKLELKRAASGGGGSGGGGSGGGGSEVKLEESGPGLVAPSQSLSIACTVSGFSLTRHGIHWVRQPPGKNLEWLGVIWAGGSTNYNSALMSRLSIIKDNSKSQVFLKMNSLQTVDTAMYYCARDHFDSFDYWGQGTTLTVSSAGGGGSGS

SEQ ID NO: 8 - protein, 110 aa, synthetic construct
DIVLTQTPAIMSASLGERVTMTCTASSSVSSSYLHWYQQKPGSSPKLWIYSTSNLASGVPLRFSGSGSGTSYSLTISSMEAEDAATYYCHQYHRSPLTFGAGTKLELKRA

SEQ ID NO: 9 - protein, 17 aa, synthetic construct
ASGGGGSGGGGSGGGGS

SEQ ID NO: 10 - protein, 117 aa, synthetic construct
EVKLEESGPGLVAPSQSLSIACTVSGFSLTRHGIHWVRQPPGKNLEWLGVIWAGGSTNYNSALMSRLSIIKDNSKSQVFLKMNSLQTVDTAMYYCARDHFDSFDYWGQGTTLTVSSA

SEQ ID NO: 11 - protein, 7 aa, synthetic construct
GGGGSGS

SEQ ID NO: 12 - protein, 369 aa, Human alphaherpesvirus 1
KYALADASLKMADPNRFRGKDLPVLDQLTDPPGVRRVYHIQAGLPDPFQPPSLPITVYYAVLERACRSVLLNAPSEAPQIVRGASEDVRKQPYNLTIAWFRMGGNCAIPITVMEYTECSYNKSLGACPIRTQPRWNYYDSFSAVSEDNLGFLMHAPAFETAGTYLRLVKINDWTEITQFILEHRAKGSCKYALPLRIPPSACLSPQAYQQGVTVDSIGMLPRFIPENQRTVAVYSLKIAGWHGPKAPYTSTLLPPELSETPNATQPELAPEDPEDSALLEDPVGTVAPQIPPNWHIPSIQDAATPYHPPATPNNMGLIAGAVGGSLLAALVICGIVYWMHRRTRKAPKRIRLPHIREDDQPSSHQPLFY

SEQ ID NO: 13 - protein, 904 aa, Human alphaherpesvirus 1
MHQGAPSWGRRWFVVWALLGLTLGVLVASAAPSSPGTPGVAAATQAANGGPATPAPPALGAAPTGDPKPKKNKKPKNPTPPRPAGDNATVAAGHATLREHLRDIKAENTDANFYVCPPPTGATVVQFEQPRRCPTRPEGQNYTEGIAVVFKENIAPYKFKATMYYKDVTVSQVWFGHRYSQFMGIFEDRAPVPFEEVIDKINAKGVCRSTAKYVRNNLETTAFHRDDHETDMELKPANAATRTSRGWHTTDLKYNPSRVEAFHRYGTTVNCIVEEVDARSVYPYDEFVLATGDFVYMSPFYGYREGSHTEHTSYAADRFKQVDGFYARDLTTKARATAPTTRNLLTTPKFTVAWDWVPKRPSVCTMTKWQEVDEMLRSEYGGSFRFSSDAISTTFTTNLTEYPLSRVDLGDCIGKDARDAMDRIFARRYNATHIKVGQPQYYLANGGFLIAYQPLLSNTLAELYVREHLREQSRKPPNPTPPPPGASANASVERIKTTSSIEFARLQFTYNHIQRHVNDMLGRVAIAWCELQNHELTLWNEARKLNPNAIASVTVGRRVSARMLGDVMAVSTCVPVAADNVIVQNSMRISSRPGACYSRPLVSFRYEDQGPLVEGQLGENNELRLTRDAIEPCTVGHRRYFTFGGGYVYFEEYAYSHQLSRADITTVSTFIDLNITMLEDHEFVPLEVYTRHEIKDSGLLDYTEVQRRNQLHDLRFADIDTVIHADANAAMFAGLGAFFEGMGDLGRAVGKVVMGIVGGVVSAVSGVSSFMSNPFGALAVGLLVLAGLAAAFFAFRYVMRLQSNPMKALYPLTTKELKNPTNPDASGEGEEGGDFDEAKLAEAREMIRYMALVSAMERTEHKAKKKGTSALLSAKVTDMVMRKRRNTNYTQVPNKDGDADEDDL

SEQ ID NO: 14 - protein, 338 aa, Human alphaherpesvirus 1
MLAVRSLQHLSTVVLITAYGLVLVWYTVFGASPLHRCIYAVRPTGTNNDTALVWMKMNQTLLFLGAPTHPPNGGWRNHAHICYANLIAGRVVPFQVPPDATNRRIMNVHEAVNCLETLWYTRVRLVVVGWFLYLAFVALHQRRCMFGVVSPAHKMVAPATYLLNYAGRIVSSVFLQYPYTKITRLLCELSVQRQNLVQLFETDPVTFLYHRPAIGVIVGCELMLRFVAVGLIVGTAFISRGACAITYPLFLTITTWCFVSTIGLTELYCILRRGPAPKNADKAAAPGRSKGLSGVCGRCCSIILSGIAMRLCYIAVVAGVVLVALHYEQEIQRRLFDV

SEQ ID NO: 15 - protein, 222 aa, Human alphaherpesvirus 1
MTMRDDLPLVDRDLVDEAAFGGEEGELPLEEQFSLSSYGTSDFFVSSAYSRLPPHTQPVFSKRVILFLWSFLVLKPLEMVAAGMYYGLTGRVVAPACILAAIVGYYVTWAVRALLLYVNIKRDRLPLSAPVFWGMSVFLGGTALCALFAAAHETFSPDGLFHFIATNQMLPPTDPLRTRALGIACAAGASMWVAAADSFAASANFFLARFWTRAILNAPVAF

SEQ ID NO: 16 - protein, 269 aa, Human alphaherpesvirus 1
MAARTRSLVERRRVLMAGVRSHTRFYKALAKEVREFHATKICGTLLTLLSGSLQGRSVFEATRVTLICEVDLGPRRPDCICVFEFANDKTLGGVCVIIELKTCKYISSGDTASKREQRATGMKQLRHSLKLLQSLAPPGDKIVYLCPVLVFVAQRTLRVSRVTRLVPQKVSGNITAVVRMLQSLSTYTVPMEPRTQRARRRRGGAARGSASRPKRSHSGARDPPEPAARQVPPADQTPASTEGGGVLKRIAALFCVPVATKTKPRAASE

SEQ ID NO: 17 - protein, 380 aa, Homo sapiens
  SIGNAL 1..26
MAFVCLAIGCLYTFLISTTFGCTSSSDTEIKVNPPQDFEIVDPGYLGYLYLQWQPPLSLDHFKECTVEYELKYRNIGSETWKTIITKNLHYKDGFDLNKGIEAKIHTLLPWQCTNGSEVQSSWAETTYWISPQGIPETKVQDMDCVYYNWQYLLCSWKPGIGVLLDTNYNLFYWYEGLDHALQCVDYIKADGQNIGCRFPYLEASDYKDFYICVNGSSENKPIRSSYFTFQLQNIVKPLPPVYLTFTRESSCEIKLKWSIPLGPIPARCFDYEIEIREDDTTLVTATVENETYTLKTTNETRQLCFVVRSKVNIYCSDDGIWSEWSDKQCWEGEDLSKKTLLRFWLPFGFILILVIFVTGLLLRKPNTYPKMIPEFFCDT

SEQ ID NO: 18 - DNA, 33 bp, synthetic construct
  source 1..33: mol_type = other DNA
ggaagatctgayattgtgmtsacmcarwctmca

SEQ ID NO: 19 - DNA, 29 bp, synthetic construct
  source 1..29: mol_type = other DNA
ccgaattcggatacagttggtgcagcatc

SEQ ID NO: 20 - DNA, 29 bp, synthetic construct
  source 1..29: mol_type = other DNA
ggaagatctsargtnmagctgsagsagtc

SEQ ID NO: 21 - DNA, 32 bp, synthetic construct
  source 1..32: mol_type = other DNA
ggaagatctsargtnmagctgsagsagtcwgg

SEQ ID NO: 22 - DNA, 35 bp, synthetic construct
  source 1..35: mol_type = other DNA
ccgaattcatagacagatgggggtgtcgttttggc

SEQ ID NO: 23 - DNA, 48 bp, synthetic construct
  source 1..48: mol_type = other DNA
aagaattcgctagcggtggtggtggatccggccctgtgcctccctcta

SEQ ID NO: 24 - DNA, 48 bp, synthetic construct
  source 1..48: mol_type = other DNA
ccgggatcctgaacctccaccaccgttgaactgtccctcgcgaaaaag

SEQ ID NO: 25 - DNA, 114 bp, synthetic construct
  source 1..114: mol_type = other DNA
cccttaaggtctcttttgtgtggtgcgttccggtatggcgcttttgttgaccacggtcattgctctcacttgccttggcggctttgcctccccaggccctgtgcctccctctac

SEQ ID NO: 26 - DNA, 40 bp, synthetic construct
  source 1..40: mol_type = other DNA
ttggatccggtaccgttgaactgtccctcgcgaaaaagtt

SEQ ID NO: 27 - DNA, 31 bp, synthetic construct
  source 1..31: mol_type = other DNA
atcggatcccggcgcgtgtaccacatccagg

SEQ ID NO: 28 - DNA, 22 bp, synthetic construct
  source 1..22: mol_type = other DNA
tccggacgtcttcggaggcccc

SEQ ID NO: 29 - DNA, 152011 bp, Human alphaherpesvirus 1
  source 1..152011: mol_type = genomic DNA
gcagcccgggccccccgcgggcgcgcgcgcgcgcaaaaaaggcgggcggcggtccgggcggcgtgcgcgcgcgcggcgggcgtggggggcggggccgcgggagcgggggaggagcgggggaggagcggggggaggagcggggggaggagcggggggaggagcggggggaggagcggggggaggagcggggggaggagcggggggaggagcggggggaggagcggggggaggagcggggggaggagcggggggaggagcggggggaggagcggggggaggagcggggggaggagcggggggaggagcgggggaggagcggccagaccccggaaacgggccccccccaaaacacaccccccgggggtcgcgcgcggccctttaaaggcgggcggcgggcagcccgggccccccgcggccgagactagcgagttagacaggcaagcactactcgcctctgcacgcacatgcttgcctgtcaaactctaccaccccggcacgctctctgtctccatggcccgccgccgccatcgcggcccccgccgcccccggccgcccgggcccacgggcgcggtcccaaccgcacagtcccaggtaacctccacgcccaactcggaacccgtggtcaggagcgcgcccgcggccgccccgccgccgccccccgccagtgggcccccgccttcttgttcgctgctgctgcgccagtggctccacgttcccgagtccgcgtccgacgacgacgacgacgactggccggacagccccccgcccgagccggcgccagaggcccggcccaccgccgccgccccccgcccccggtccccaccgcccggcgcgggcccggggggcggggctaacccctcccaccccccctcacgccccttccgccttccgccgcgcctcgccctccgcctgcgcgtcaccgcagagcacctggcgcgcctgcgcctgcgacgcgcgggcggggagggggcgccgaagccccccgcgacccccgcgacccccgcgacccccacgcgggtgcgcttctcgccccacgtccgggtgcgccacctggtggtctgggcctcggccgcccgcctggcgcgccgcggctcgtgggcccgcgagcgggccgaccgggctcggttccggcgccgggtggcggaggccgaggcggtcatcgggccgtgcctggggcccgaggcccgtgcccgggccctggcccgcggagccggcccggcgaactcggtctaacgttacacccgaggcggcctgggtcttccgcggagctcccgggagctccgcaccaagccgctctccggagagacgatggcaggagccgcgcatatatacgcttggagccggcccgcccccgaggcgggcccgccctcggagggcgggactggccaatcggcggccgccagcgcggcggggcccggccaaccagcgtccgccgagtcgtcggggcccggcccactgggcggtaactcccgcccagtgggccgggccgcccacttcccggtatggtaattaaaaacttgcagaggccttgttccgcttcccggtatggtaattagaaactcattaatgggcggccccggccgcccttcccgcttccggcaattcccgcggcccttaatgggcaaccccggtattccccgcctcccgcgccgcgcgtaaccactcccctggggttccgggttatgttaattgcttttttggcggaacacacggcccctcgcgcattggcccgcgggtcgctcaatgaacccgcattggtcccctggggttccgggtatggtaatgagtttcttcgggaaggcgggaagccccggggcaccgacgcaggccaagcccctgttgcgtcggcgggaggggcatgctaatggggttctttgggggacaccgggttggtcccccaaatcgggggccgggccgtgcatgctaatgatattctttgggggcgccgggttggtccccggggacggggccgccccgcggtgggcctgcctcccctgggacgcgcggccattgggggaatcgtcactgccgcccctttggggaggggaaaggcgtggggtataagttagccctggcccgacggtctggtcgcatttgcacctcggcactcggagcgagacgcagcagccaggcagactcgggccgccccctctccgcatcaccacagaagccccgcctacgttgcgacccccagggaccctccgtcagcgaccctccagccgcatacgacccccatggagccccgccccggagcgagtacccgccggcctgagggccgcccccagcgcgaggtgaggggccgggcgccatgtctggggcgccatgttggggggcgccatgttggggggcgccatgttgggggacccccgacccttacactggaaccggccgccatgttgggggacccccactcatacacgggagccgggcgccatgttggggcgccatgttagggggcgtggaaccccgtgacactatatatacagggaccgggggcgccatgttagggggcgcggaaccccctgaccctatatatacagggaccggggtcgccctgttaggggtcgccatgtgaccccctgactttatatatacagacccccaacacctacacatggcccctttgactcagacgcagggcccggggtcgccgtgggacccccctgactcatacacagagacacgcccccacaacaaacacacagggaccggggtcgccgtgttagggggcgtggtccccactgactcatacgcagggcccccttactcacacgcatctaggggggtggggaggagccgcccgccatatttgggggacgccgtgggacccccgactccggtgcgtctggagggcgggagaagagggaagaagaggggtcgggatccaaaggacggacccagaccacctttggttgcagacccctttctcccccctcttccgaggccagcaggggggcaggactttgtgaggcggggggggagggggaactcgtgggcgctgattgacgcgggaaatccccccattcttacccgcccccccttttttcccctcagcccgccccggatgtctgggtgtttccctgcgaccgagacctgccggacagcagcgactcggaggcggagaccgaagtgggggggcggggggacgccgaccaccatgacgacgactccgcctccgaggcggacagcacggacacggaactgttcgagacggggctgctggggccgcagggcgtggatgggggggcggtctcgggggggagccccccccgcgaggaagaccccggcagttgcgggggcgccccccctcgagaggacggggggagcgacgagggcgacgtgtgcgccgtgtgcacggatgagatcgcgccccacctgcgctgcgacaccttcccgtgcatgcaccgcttctgcatcccgtgcatgaaaacctggatgcaattgcgcaacacctgcccgctgtgcaacgccaagctggtgtacctgatagtgggcgtgacgcccagcgggtcgttcagcaccatcccgatcgtgaacgacccccagacccgcatggaggccgaggaggccgtcagggcgggcacggccgtggactttatctggacgggcaatcagcggttcgccccgcggtacctgaccctgggggggcacacggtgagggccctgtcgcccacccaccctgagcccaccacggacgaggatgacgacgacctggacgacggtgaggcgggggggcggcgaggaccctgggggaggaggaggaggggggggggagggaggaataggcgggcgggcgggcgaggaaagggcgggccggggagggggcgtaacctgatcgcgccccccgttgtctcttgcagcagactacgtaccgcccgccccccgccggacgccccgcgcccccccacgcagaggcgccgccgcgccccccgtgacgggcggggcgtctcacgcagccccccagccggccgcggctcggacagcgcccccctcggcgcccatcgggccacacggcagcagtaacactaacaccaccaccaacagcagcggcggcggcggctcccgccagtcgcgagccgcggtgccgcggggggcgtctggcccctccgggggggttggggttgttgaagcggaggcggggcggccgaggggccggacgggcccccttgtcaacagacccgccccccttgcaaacaacagagaccccatagtgatcagcgactcccccccggcctctccccacaggccccccgcggcgcccatgccaggctccgccccccgccccggtccccccgcgtccgcggccgcgtcgggccccgcgcgcccccgcgcggccgtggccccgtgtgtgcgggcgccgcctccggggcccggcccccgcgccccggcccccggggcggagccggccgcccgccccgcggacgcgcgccgtgtgccccagtcgcactcgtccctggctcaggccgcgaaccaagaacagagtctgtgccgggcgcgtgcgacggtggcgcgcggctcgggggggccgggcgtggagggtggacacgggccctcccgcggcgccgccccctccggcgccgccccctccggcgcccccccgctcccctccgccgcctctgtcgagcaggaggcggcggtgcgtccgaggaagaggcgcgggtcgggccaggaaaacccctccccccagtccacgcgtccccccctcgcgccggcaggggccaagagggcggcgacgcaccccccctccgactcagggccgggggggcgcggccagggagggcccgggacccccctgacgtcctcggcggcctccgcctcttcctcctccgcctcttcctcctcggccccgactcccgcgggggccacctcttccgccaccggggccgcgtcctcctccgcttccgcctcctcgggcggggccgtcggtgccctgggagggagacaagaggaaacctccctcggcccccgcgctgcttctgggccgcgggggccgaggaagtgtgcccggaagacgcgccacgcggagacttccggggccgtccccgcgggcggcctcacgcgctacctgcccatctcgggggtctctagcgtggtcgccctgtcgccttacgtgaacaagacgatcacgggggactgcctgcccatcctggacatggagacggggaacatcggggcgtacgtggtcctggtggaccagacgggaaacatggcgacccggctgcgggccgcggtccccggctggagccgccgcaccctgctccccgagaccgcgggtaaccacgtgacgccccccgagtacccgacggcccccgcgtcggagtggaacagcctctggatgacccccgtggggaacatgctgttcgaccagggcaccctagtgggcgccctggacttccgcagcctgcggtctcggcacccgtggtccggggagcagggggcgtcgacccgggacgagggaaaacaataagggacgcccccgtgtttgtggggaggggggggtcgggcgctgggtggtctctggccgcgcccactacaccagccaatccgtgtcggggaggtggaaagtgaaagacacgggcaccacacaccagcgggtcttttgtgttggccctaataaaaaaaactcaggggatttttgctgtctgttgggaaataaaggtttacttttgtatcttttccctgtctgtgttggatgtatcgcgggggtgcgtgggagtgggggtgcgtgggagtgggggtgcgtgggagtgggggtgcgtgggagtgggggtgcgtgggagtgggggtgcgtgggagtgggggtgcgtgggagtgggggtgcgtgggagtgggggtgcgtgggagtgggggtgccatgttgggcaggctctggtgttaaccacagagccgcggcccgggctgcctgaccaccgatccccgaaagcatcctgccactggcatggagccagaaccacagtgggttgggtgtgggtgttaagtttccgcgagcgcctgcccgcccggactgacctggcctctggccgccacaaagggcgggggggggggttaactacactatagggcaacaaaggatgggaggggtagcggggcgggacggggcgcccaaaagggggtcggccacaccacagacgtgggtgttggggggtggggcggaggggtggggggggagacagaaacaggaacatagttagaaaacaagaatgcggtgcagccagagaatcacaggagacgaggggatgggcgtgttggttaccaacccacacccaggcatgctcggtggtatgaaggagggggggcggtgtttcttagagaccgccgggggacgtggggttggtgtgcaaaggcacgcgcacccgcgccggccaggtgggccggtaccccatccccccctcccccgacccttcccacccccgcgtgccagagatcaccccggtcccccggcacccgccactcctccatatcctcgctttaggaacaactttaggggggggtacacacgcgccgtgcatttccttccacaccccccccctcccccgcactccccccccccaggcagtaagacccaagcatagagagccaggcacaaaaacacaggcggggtgggacacatgccttcttggagtacgtgggtcattggcgtggggggttacagcgacaccggccgaccccctggcggtcttccagccggcccttagataagggggcagttggtggtcggacgggtaagtaacagagtctaactaagggtgggagggggggaaaataacgggctggtgtgctgtaacacgagcccacccgcgagtggcgtggccgaccttagcctctggggcgccccctgtcgtttgggtccccccccctctattggggagaagcaggtgtctaacctacctggaaacgcggcgtctttgttgaacgacaccggggcgccctcgacgagtgggataacgggggaggaagggagggaggagggtactgggggtgaagggggggggggagaagcgagaacaggaaaggcgacggagcccggcagaacaccgaggaaaaaaaaaccacagcgcatgcgccgggccgttgtggggccccgggccggggccccttgggtccgccggggccccgggccgggccgccacgggggccggccgttggcggtaaccccgagtgttcatctcaggccccgggccgggaacccggaaaagcctccggggggcctttttcgcgtcgcgtgccggcgagcgggtccggacggggcccggaccgccgcggtcgggggcccctcgtcccgggccgtacgcggccttcgccccgtgaggggacagacgaacgaaacattccggcgacggaacgaaaaacaccccagacgggttaaagaaacagaaaccgcaacccccaccacccccgaaacggggaaaacgaaaaaacagaccagcggccggccggcgcttagggggaggatgtcgccgacgccccttggccgccccggctgcaggggggcccggagagccgcggcacccggacgcgcccggaaagtctttcgcaccaccggcgatcggcacggccgcgcccccgcttttataaaggctcagatgacgcagcaaaaacaggccacagcaccacatgggtaggtgatgtaattttattttcctcgtctgcggcctaatggatttccgggcgcggtgcccctgtctgcagagcacttaacggattgatatctcgcgggcacgcgcgcccttaatggaccggcgcggggcggggggccggatacccacacgggcgggggggggtgtcgcgggccgtctgctggcccgcggccacataaacaatgactcggggcctttctgcctctgccgcttgtgtgtgcgcgcgccggctctgcggtgtcggcggcggcggcggcggtggccgccgtgttcggtctcggtagccggccggcgggtggactcgcggggggccggagggtggaaggcaggggggtgtaggatgggtatcaggacttccacttcccgtccttccatcccccgttcccctcggttgttcctcgcctcccccaacaccccgccgctttccgttggggttgttattgttgtcgggatcgtgcgggccgggggtcgccggggcaggggcgggggcgtgggcgggggtgctcgtcgatcgaccgggctcagtgggggcgtggggtgggtgggagaaggcgaggagactggggtgggggtgtcggtgggtggttgttttttgtggttgttttttgtgtctgtttccgtcccccgtcacccccctccctccgtcccctccgtccccccgtcgcgggtgtttgtgtttgtttattccgacatcggtttatttaaaataaacacagccgttctgcgtgtctgttcttgcgtgtggctgggggcttatatgtggggtcccgggggcgggatggggtttagcggcggggggcggcgcgccggacggggcgctggagataacggcccccggggaacgggggaccggggctgggtatcccgaggtgggtgggtgggcggcggtggccgggccgggccgggccgggccgggtgggcggggtttggaaaaacgaggaggaggaggagaaggcggggggggagacggggggaaagcaaggacacggcccggggggtgggagcgcgggccgggccgctcgtaagagccgcgacccggccgccggggagcgttgtcgccgtcggtctgccggcccccgtccctcccttttttgaccaaccagcgccctcccccccaccaccattcctactaccaccaccaccaccacccccaccaccgacacctcccgcgcacccccgcccacatccccccaccccgcaccacgagcacggggtgggggtagcaggggatcaaaggggggcaaagccggcggggcggttcgggggggcgggagaccgagtaggcccgcccatacgcggcccctcccggcagccacgccccccagcgtcgggtgtcacggggaaagagcaggggagagggggggagaggggagagggggggagaggggagagggggggagaggggagagggggggagaggggagagggggggagaggggagagggggggagaggggagagggggggagaggggagagggggggagaggggagagggggggagaggggagagggggggagagggggtatataaaccaacgaaaagcgcgggaacggggatacggggcttgtgtggcacgacgtcgtggttgtgttactgggcaaacacttggggactgtaggtttctgtgggtgccgaccctaggcgctatggggattttgggttgggtcgggcttattgccgttggggttttgtgtgtgcgggggggcttgtcttcaaccgaatatgttattcggagtcgggtggctcgagaggtgggggatatattaaaggtgccttgtgtgccgctcccgtctgacgatcttgattggcgttacgagaccccctcggctataaactatgctttgatagacggtatatttttgcgttatcactgtcccggattggacacggtcttgtgggataggcatgcccagaaggcatattgggttaacccctttttatttgtggcgggttttctggaggacttgagtcaccccgcgtttcctgccaacacccaggaaacagaaacgcgcttggccctttataaagagatacgccaggcgctggacagtcgcaagcaggccgccagccacacacctgtgaaggctgggtgtgtgaactttgactattcgcgcacccgccgctgtgtagggcgacaggatttgggacctaccaacggaacgtctggacggaccccggttctgccgccggacgatgaagcgggcctgcaaccgaagcccctcaccacgccgccgcccatcatcgccacgtcggaccccaccccgcgacgggacgccgccacaaaaagcagacgccgacgaccccactcccggcgcctctaacgatgcctcgacggaaacccgtccgggttcggggggcgaaccggccgcctgtcgctcgtcagggccggcgggcgctcctcgccgccctagaggctgtcccgctggtgtgacgttttcctcgtccgcgccccccgaccctcccatggatttaacaaacgggggggtgtcgcctgcggcgacctcggcgcctctggactggaccacgtttcggcgtgtgtttctgatcgacgacgcgtggcggcccctgatggagcctgagctggcgaaccccttaaccgcccacctcctggccgaatataatcgtcggtgccagaccgaagaggtgctgccgccgcgggaggatgtgttttcgtggactcgttattgcacccccgacgaggtgcgcgtggttatcatcggccaggacccatatcaccaccccggccaggcgcacggacttgcgtttagcgtgcgcgcgaacgtgccgcctcccccgagtcttcggaatgtcttggtggccgtcaagaactgttatcccgaggcacggatgagcggccacggttgcctggaaaagtgggcgcgggacggcgtcctgttactaaacacgaccctgaccgtcaagcgcggggcggcggcgtcccactctagaatcggttgggaccgcttcgtgggcggagttatccgccggttggccgcgcgccgccccggcctggtgtttatgctctggggcgcacacgcccagaatgccatcaggccggaccctcgggtccattgcgtcctcaagttttcgcacccgtcgcccctctccaaggttccgttcggaacctgccagcatttcctcgtggcgaaccgatacctcgagacccggtcgatttcacccatcgactggtcggtttgaaaggcatcgacgtccggggtttttgtcggtgggggcttttgggtatttccgatgaataaagacggttaatggttaaacctctggtctcatacgggtcggtgatgtcgggcgtcgggggagagggagttccctctgcgcttgcgattctagcctcgtggggctggacgttcgacacgccaaaccacgagtcggggatatcgccagatacgactcccgcagattccattcggggggccgctgtggcctcacctaaccaacctttacacgggggcccggaacgggaggccacagcgccgtctttctccccaacgcgcgcggatgacggcccgccctgtaccgacgggccctacgtgacgtttgataccctgtttatggtgtcgtcgatcgacgaattagggcgtcgccagctcacggacaccatccgcaaggacctgcggttgtcgctggccaagtttagcattgcgtgcaccaagacctcctcgttttcgggaaacgccccgcgccaccacagacgcggggcgttccagcgcggcacgcgggcgccgcgcagcaacaaaagcctccagatgtttgtgttgtgcaaacgcgcccacgccgctcgagtgcgagagcagcttcgggtcgttattcagtcccgcaagccgcgcaagtattacacgcgatcttcggacgggcggctctgccccgccgtccccgtgttcgtccacgagttcgtctcgtccgagccaatgcgcctccaccgagataacgtcatgctggcctcgggggccgagtaaccgccccccccccatgccaccctcactgcccgtcgcgcgtgtttgatgttaataaataacacataaatttggctggttgtttgttgtctttaatggaccgcccgcaagggggggggggcgtttcagtgtcgggtgacgagcgcgatccggccgggatcctaggaccccaaaagtttgtctgcgtattccagggtggggctcagttgaatctcccgcagcacctctaccagcaggtccgcggtgggctggagaaactcggccgtcccggggcaggcggttgtcgggggtggaggcgcggcgcccaccccgtgtgccgcgcctggcgtctcctctgggggcgacccgtaaatggttgcagtgatgtaaatggtgtccgcggtccagaccacggtcaaaatgccggccgtggcgctccgggcgctttcgccgcgcgaggagctgacccaggagtcgaacggatacgcgtacatatgggcgtcccacccgcgttcgagcttctggttgctgtcccggcctataaagcggtaggcacaaaattcggcgcgacagtcgataatcaccaacagcccaatgggggtgtgctggataacaacgcctccgcgcggcaggcggtcctggcgctcccggccccgtaccatgatcgcgcgggtgccgtactcaaaaacatgcaccacctgcgcggcgtcgggcagtgcgctggtcagcgaggccctggcgtggcataggctatacgcgatggtcgtctgtggattggacatctcgcggtgggtagtgagtcccccgggccgggttcggtggaactgtaaggggacggcgggttaatagacaatgaccacgttcggatcgcgcagagccgatagtatgtgctcactaatgacgtcatcgcgctcgtggcgctcccggagcggatttaagttcatgcgaaggaattcggaggaggtggtgcgggacatggccacgtacgcgctgttgaggcgcaggttgccgggcgtaaagcagatggcgaccttgtccaggctaaggccctgggagcgcgtgatggtcatggcaagcttggagctgatgccgtagtcggcgtttatggccatggccagctccgtagagtcaatggactcgacaaactcgctgatgttggtgttgacgacggacatgaagccgtgttggtcccgcaagaccacgtaaggcaggggggcctcttccagtaactcggccacgttggccgtcgcgtgccgcctccgcagctcgtccgcaaaggcaaacacccgtgtgtacgtgtatcccatgagcgtataattgtccgtctgcagggcgacggacatcagccccccgcgcggcgagccggtcagcatctcgcagccccggaagataacgttgtccacgtacgtgctaaagggggcgacttcaaatgcctccccgaagagctcttggaggattcggaatctcccgaggaaggcccgcttcagcagcgcaaactgggtgtgaacggcggcggtggtctccggttccccgggggtgtagtggcagtaaaacacgtcgagctgttgttcgtccagccccgcgaaaataacgtcgaggtcgtcgtcgggaaaatcgtccgggcccccgtcccgcggccccagttgcttaaaatcaaacgcacgctcgccgggggcgcctgcgtcggccattaccgacgcctgcgtcggcacccccgaagatttggggcgcagagacagaatctccgccgttagttctcccatgcgggcgtacgcgagggtcctctgggtcgcatccaggcccgggcgctgcagaaagttgtaaaaggagataagcccgctaaatatgagccgcgacaggaacctgtaggcaaactccaccgaagtctccccctgagtctttacaaagctgtcgtcacgcaacactgcctcgaaggcccggaacgtcccactaaacccaaaaaccagttttcgcaggcgcgcggtcaccgcgatctggctgttgaggacgtaagtgacgtcgttgcgggccacgaccagctgctgtttgctgtgcacctcgcagcgcatgtgccccgcgtcctggtcctggctctgcgagtagttggtgatgcggctggcgttggccgtgagccacttttcaatagtcaggccgggctggtgtgtcagccgtcggtattcgtcaaactccttgaccgacacgaacgtaagcacggggagggtgaacacgacgaactccccctcacgggtcaccttcaggtaggcgtggagcttggccatgtacgcgctcacctctttgtgggaggagaacagccgcgtccagccggggaggttggcggggttggtgatgtagttttccgggacgacgaagcgatccacgaactgcatgtgctcctcggtgatgggcaggccgtactccagcaccttcatgaggttaccgaactcgtgctcgacgcaccgtttgttgttaataaaaatggcccagctatacgagaggcgggcgtactcgcgcagcgtgcggttgcagatgaggtacgtgagcacgttctcgctctggcggacggaacaccgcagtttctggtgctcgaaggtcgactccagggacgccgtctgcgtcggcgagcccacacacaccaacacgggccgcaggcgggccgcgtactggggggtgtggtacagggcgttaatcatccaccagcaatacaccacggccgtgaggaggtgacgcccaaggagcccggcctcgtcgatgacgatcacgttgctgcgggtaaaggccggcagcgccccgtgggtggccggggccaaccgcgtcagggcgccctcggccaaccccagggtccgttccagggcggccagggcgcgaaactcgttccgcaactcctcgcccccggaggcggccagggcgcgcttcgtgaggtccaaaatcacctcccagtagtacgtcagatctcgtcgctgcaggtcctccagcgaggcggggttgctggtcagggtgtacgggtactgtcccagttgggcctggacgtgattcccgcgaaacccaaattcatgaaagatggtgttgatgggtcggctgagaaaggcgcccgagagtttggcgtacatgttttgggccgcaatgcgcgtggcgcccgtcaccacacagtccaagacctcgttgattgtctgcacgcacgtgctctttccggagccagcgttgccggtgataagatacaccgcgaacggaaactccctgaggggcaggcctgcgggggactctaaggccgccacgtcccggaaccactgcagacggggcacttgcgctccgtcgagctgttgttgcgagagctctcggatgcgcttaaggattggctgcaccccgtgcatagacgtaaaatttaaaaaggcctcggccctccctggaacggctggtcggtccccgggttgctgaaggtgcggcgggccgggtttctgtccgtctagctggcgctccccgccggccgccgccatgaccgcaccacgctcgtgggcccccactacgcgtgcgcggggggacacggaagcgctgtgctcccccgaggacggctgggtaaaggttcaccccacccccggtacgatgctgttccgtgagattctccacgggcagctggggtataccgagggccagggggtgtacaacgtcgtccggtccagcgaggcgaccacccggcagctgcaggcggcgatctttcacgcgctcctcaacgccaccacttaccgggacctcgaggcggactggctcggccacgtggcggcccgcggtctgcagccccaacggctggttcgccggtacaggaacgcccgggaggcggatatcgccggggtggccgagcgggtgttcgacacgtggcggaacacgcttaggacgacgctgctggactttgcccacgggttggtcgcctgctttgcgccgggcggcccgagcggcccgtcaagcttccccaaatatatcgactggctgacgtgcctggggctggtccccatattacgcaagcgacaagaagggggtgtgacgcagggtctgagggcgtttctcaagcagcacccgctgacccgccagctggccacggtcgcggaggccgcggagcgcgccggccccgggttttttgagctggcgctggccttcgactccacgcgcgtggcggactacgaccgcgtgtatatctactacaaccaccgccggggcgactggctcgtgcgagaccccatcagcgggcagcgcggagaatgtctggtgctgtggccccccttgtggaccggggaccgtctggtcttcgattcgcccgtccagcggctgtttcccgagatcgtcgcgtgtcactccctccgggaacacgcgcacgtctgccggctgcgcaataccgcgtccgtcaaggtgctgctggggcgcaagagcgacagcgagcgcggggtggccggtgccgcgcgggtcgttaacaaggtgttgggggaggacgacgagaccaaggccgggtcggccgcctcgcgcctcgtgcggcttatcatcaacatgaagggcatgcgccacgtaggcgacattaacgacaccgtgcgtgcctacctcgacgaggccggggggcacctgatagacgccccggccgtcgacggtaccctccctggattcggcaagggcggaaacagccgcgggtctgcgggccaggaccagggggggcgggcgccgcagcttcgccaggccttccgcacggccgtggttaacaacatcaacggcgtgttggagggctatataaataacctgtttggaaccatcgagcgcctgcgcgagaccaacgcgggcctggcgacccaattgcaggagcgcgaccgcgagctccggcgcgcaacagcgggggccctggagcgccagcagcgcgcggccgacctggcggccgagtccgtgaccggtggatgcggcagccgccctgcgggggcggacctgctccgggccgactatgacattatcgacgtcagcaagtccatggacgacgacacgtacgtcgccaacagctttcagcacccgtacatcccttcgtacgcccaggacctggagcgcctgtcgcgcctctgggagcacgagctggtgcgctgttttaaaattctgtgtcaccgcaacaaccagggccaagagacgtcgatctcgtactccagcggggcgatcgccgcattcgtcgccccctactttgagtcagtgcttcgggccccccgggtaggcgcgcccatcacgggctccgatgtcatcctgggggaggaggagttatgggatgcggtgtttaagaaaacccgcctgcaaacgtacctgacagacatcgcggccctgttcgtcgcggacgtccagcacgcagcgctgcccccgcccccctccccggtcggcgccgatttccggcccggcgcgtccccgcggggccggtccagatcgcggtcgcccggaagaactgcgccaggcgcgccggaccagggcgggggcatcgggcaccgggatggccgccgcgacggccgacgatgaggggtcggccgccaccatcctcaagcaggccatcgccggggaccgcagcctggtcgaggcggccgaggcgattagccagcagacgctgctccgcctggcctgcgaggtgcgccaggtcggcgaccgccagccgcggtttaccgccaccagcatcgcgcgcgtcgacgtcgcgcctgggtgccggttgcggttcgttctggacgggagtcccgaggacgcctatgtgacgtcggaggattactttaagcgctgctgcggccagtccagttatcgcggcttcgcggtggcggtcctgacggccaacgaggaccacgtgcacagcctggccgtgccccccctcgttctgctgcaccggttctccctgttcaaccccagggacctcctggactttgagcttgcctgtctgctgatgtacctggagaactgcccccgaagccacgccaccccgtcgacctttgccaaggttctggcgtggctcggggtcgcgggtcgccgcacgtccccattcgaacgcgttcgctgccttttcctccgcagttgccactgggtcctaaacacactcatgttcatggtgcacgtaaaaccgttcgacgacgagttcgtcctgccccactggtacatggcccggtacctgctggccaacaacccgccccccgttctctcggccctgttctgtgccaccccgacgagctcctcattccggctgccggggccgcccccccgctccgactgcgtggcctataaccccgccgggatcatggggagctgctgggcgtcggaggaggtgcgcgcgcctctggtctattggtggctttcggagaccccaaaacgacagacgtcgtcgctgttttatcagttttgttgaattttaggaaataaacccggttttgtttctgtggcctcccgacggatgcgcgtgtccttcctccgtcttggtgggtgggtgtctgtgtatcgcgtcccatctgtgcggagagggggggcatgtcggcacgtattcggacagactcaagcacacacgggggagcgctcttgtctcagggcaatgtttttattggtcaaactcaggcaaacagaaacgacatcttgtcgtcaaagggatacacaaacttccccccctctccccatactcccgccagcaccccggtaaacaccaactcaatctcgcgcaggatttcgcgcaggtgatgagcgcagtccacgggggggagcacaaggggccgcgggtatagatcgacggggacgccgaccgactccccgcctccgggacagacacgcacgacgcgccgccagtagtgctctgcgtccagcaaggcgccgccgcggaaggcagtggggggcaaggggtcgctagcctcaaagggggacacccgaacgctccagtactccgcgtccaaccgtttattaaacgcgtccacgataaggcggtcgcaggcgtcctccataaggccccgggccgtgagtgcgtcctcctccggcacgcctgccgttgtcaggcccaggacccgtcgcagcgtgtcgcgtacgaccccggccgccgtggtgtacgcgggcccgcggagaggaaatcccccaagatggtcagtgttgtcgcgggagttccagaaccacactcccgcctggttccaggcgactgcgtgggtgtagacgccctcgagggccaggcacagtgggtgccgcagccggaggccgttggccctaagcacggctcccacggccgtctcgatggcccgccgggcgtcctcgatcaccccggaagccgcatccgcgtcttgggggtccacgttaaagacaccccagaacgcacccccatcgcccccgcagaccgcgaacttcaccgagctggccgtctcctcgatctgcaggcagacggcggccattaccccacccaggagctgccgcagcgcagggcaggcgtcgcacgtgtccgggaccaggcgctccaagacggccccggcccagggctctgagggagcggccaccaccagcgcgtccagtcttgctaggcccgtccggccgtgggggtccgccagcccgctccccccgaggtcggccagggccgccaggagctgggcgcgaagtccggggaagcaaaaccgcgccgtccagacgggcccgacggccgcgggcgggtctaacagttggatgattttagtggcgggatgccaccgcgccaccgcctcccgcaccgcgggcaggaggcatccggctgccgccgaggccacgccgggccaggctcgcggggggaggacgaccctggcccccaccgcgggccaggcccccaggagcgcggcgtaagcggccgcggccccgcgcaccaggtcccgtgccgactcggccgtggccggcacggtgaacgtgggccaacccggaaaccccaggacggcaaagtacgggacgggtcccccccggacctcaaactcgggccccagaaaggcaaagacgggggccagggccccgggggcggcgtggaccgtggtatgccactgccggaaaagggcgacgagcgccggcgcggagaacttctcgccggcgcttacaaagtagtcgtaatcgcggggcagcagcacccgtgccgtgactcgttgcgggtgcccgcgtggccgcaggcccacctcgcacacctcgaccaggtccccgaacgcgccctccttcttgatcggcggaaacgcaagagtctggtattcgcgcgcaaatagcgcggttccggtggtgatgttaacggtcagcgaagcggcggacgcgcactggggggtgtcgcgaatggccgccaggcgcgcccacgccagccgcgcgtcgggatgctcggcaacgcgcgccgccagggccatagggtcgatgtcaatgttggcctccgcgaccaggagagcggcgcgaggggcggcgggcgggccccacgacgctctctcaactttcaccaccagtcccgtgcgtgggtccgagccgatacgcagcggggcgaacagggccaccggcccggtctggcgctccagggccgccaggacgcacgcgtacagcgcccgccacagagtcgggttctccaggggctccagcggggaggcggccggcgtcgtcgcggcgcgggcggccgccacgacggcctggacggagacgtccgcggagccgtagaaatcccgcagctccgtcgcggtgacggagacctccgcaaagcgcgcgcgaccctcccctgcggcgttgcgacatacaaaatacaccagggcgtggaagtactcgcgagcgcgggggggcagccataccgcgtaaagggtaatggcgctgacgctctcctccacccacacgatatctgcggtgtccatcgcacggcccctaaggatcacgggcggtctgtgggtcccatgctgccgtgcctggccgggcccggtgggtcgcggaaaccggtgacggggggggggcggtttttggggttggggtgggggtgggaaacggcccgggtccgggggccaacttggcccctcggtgcgttccggcaacagcgccgccggtccgcggacgaccacgtaccgaacgagtgcggtcccgagacttatagggtgctaaagttcaccgccccctgcatcatgggccaggcctcggtggggagctccgacagcgccgcctccaggatgatgtcagcgttggggttggcgctggatgagtgcgtgcgcaaacagcgcccccacgcaggcacgcgtagcttgaagcgcgcgcccgcaaactcccgcttgtgggccataagcagggcgtacagctgcctgtgggtccggcaggcgctgtggtcgatgtggtgggcgtccaacaaccccacgattgtctgtttggtgaggtttttaacgcgccccgccccgggaaacgtctgcgtgcttttggccatctgcacgccaaacagttcgccccagattatcttgaacagcgccaccgcgtggtccgtctcgctaacggacccgcgcgggggacagccgcttagggcgtcggcgacgcgcttgacggcttcctccgagagcagaagtccgtcggttacgttacagtggcccagttcgaacaccagctgcatgtagcggtcgtagtggggggtcagtaggtccagcacgtcatcggggccgaaggtcctcccagatcccccggccgccgagtcccaatgcaggcgcgcggccatggtgctgcacaggcacaacagctcccagacgggggttacgttcagggtggggggcagggccacgagctccagctctccggtgacgttgatcgtggggatgacgcccgtggcgtagtggtcatagatccgccgaaatatggcgctgctgcgggtggccatgggaacgcggagacaggcctccagcaacgccaggtaaataaaccgcgtgcgtcccatcaggctgttgaggttgcgcatgagcgcgacaatttccgccggcgcgacatcggaccggaggtatttttcgacgaaaagacccacctcctccgtctcggcggcctgggccggcagcgacgcctcgggatcccggcaccgcagctcccgtagatcgcgctgggccctgagggcgtcgaaatgtacgccccgcaaaaacagacagaagtcctttggggtcagggtatcgtcgtgtccccagaagcgcacgcgtatgcagtttagggtcagcagcatgtgaaggatgttaaggctgtccgagagacacgccagcgtgcatctctcaaagtagtgtttgtaacggaatttgttgtagatgcgcgacccccgccccagcgacgtgtcgcatgccgacgcgtcacagcgccccttgaaccggcgacacagcaggtttgtgacctgggagaactgcgcgggccactggccgcaggaactgaccacgtgattaaggagcatgggcgtaaagacgggctccgagcgcgccccggagccgtccatgtaaatcagtagctcccccttgcggagggtgcgcacccgtcccagggactggtacacggacaccatgtccggtccgtagttcatgggttttacgtaggcgaacatgccatcaaagtgcaggggatcgaagctgaggcccacggttacgaccgtcgtgtatataaccacgcggtattggccccacgtggtcacgtccccgaggggggtgagcgagtgaagcaacagcacgcggtccgtaaactgacggcagaaccgggccacgatctccgcgaaggagaccgtcgacgaaaaaatgcagatgttatcgcccccgccaaggcgcgcttccagctccccaaagaacgtggccccccgggcgtccggagaggcgtccggagacgggccgctcggcggcccgggcgggcgcagggcagcctgcaggagctcggtccccagacgcgggagaaacaggcaccggcgcgccgaaaacccgggcatggcgtactcgccgaccaccacatgcacgtttttttcgccccggagaccgcacaggaagtccaccaactgcgcgttggcggttgcgtccatggcgatgatccgaggacaggtgcgcagcaggcgtagcattaacgcatccacgcggcccagttgctgcatcgttggcgaatagagctggcccagcgtcgacataacctcgtccagaacgaggacgtcgtagttgttcagaaggttggggcccacgcgatgaaggctttccacctggacgataagtcggtggaaggggcggtcgttcataatgtaattggtggatgagaagtaggtgacaaagtcgaccaggcctgactcagcgaaccgcgtcgccagggtctgggtaaaactccgacgacaggagacgacgagcacactcgtgtccggagagtggatcgcttcccgcagccagcggatcagcgcggtagtttttcccgaccccattggcgcgcggaccacagtcacgcacctggccgtcggggcgctcgcgttggggaaggtgacgggtccgtgctgctgccgctcgatcgttgttttcgggtgaacccggggcacccattcggccaaatcccccccgtacaacatccgcgctagcgatacgctcgacgtgtactgttcgcactcgtcgtccccaatgggacgcccggcccccagaggatctcccgactccgcgccccccacgaaaggcatgaccggggcgcggacggcgtggtgggtctggtgtgtgcaggtggcgacgtttgtggtctctgcggtctgcgtcacggggctcctcgtcctggcctctgtgttccgggcacggtttccctgcttttacgccacggcgagctcttatgccggggtgaactccacggccgaggtgcgcgggggtgtagccgtgcccctcaggttggacacgcagagccttgtgggcacttatgtaatcacggccgtgttgttgttggccgcggccgtgtatgccgtggtcggcgccgtgacctcccgctacgaccgcgccctggacgcgggccgccgtctggctgcggcccgcatggccatgccgcacgccacgctgatcgccggaaacgtctgctcttggttgctgcagatcaccgtcctgttgctggcccatcgcaccagccagctggcccacctggtttacgtcctgcactttgcgtgtctggtgtattttgcggcccatttttgcaccaggggggtcctgagcgggacgtatctgcgtcaggtgcacggcctgatggagccggccccgactcatcatcgcgtcgttggcccggctcgagccgtgctgacaaacgccttgctgttgggcgtcttcctgtgcacggccgacgccgcggtatccctgaataccatcgccgcgttcaactttaatttttcggccccgggcatgctcatatgcctgaccgtgctgttcgcccttctcgtcgtatcgctgttgttggtggtcgagggggtgttgtgtcactacgtgcgcgtgttggtgggcccccacctgggggccgtggccgccacgggcatcgtcggcctggcatgcgagcactattacaccaacggctactacgttgtggagacgcagtggccgggggcccagacgggagtccgcgtcgccctcgccctggtcgccgcctttgccctcggcatggccgtgctccgctgcacccgcgcctatctgtatcacaggcggcaccacaccaaattttttatgcgcatgcgcgacacgcgacaccgcgcacattccgccctcaagcgcgtacgcagttccatgcgcggatcgcgagacggccgccacaggcccgcacccggcagcccgcccgggattcccgaatatgcggaagacccctacgcgatctcatacggcggccagctcgaccggtacggagattccgacggggagccgatttacgacgaggtggcggacgaccaaaccgacgtattgtacgccaagatacaacacccgcggcacctgcccgacgacgagcccatctatgacaccgttggggggtacgaccccgagcccgccgaggaccccgtgtacagcaccgtccgccgttggtagctgtttggttccgttttaataaaccgtttgtgtttaacccgaccgtggtgtatgtctggtgtgtggcgtccgatcccgttactatcaccgttccccccaaaccccggcgattgtgggtttttttaaaaacgacacgcgtgcgaccgtatacagaacattgttgttttttattcgctatcggacatggggggtggaaactgggtggcggggcaggcgcctccgggggttcgccggtgagtgtggcgcgaggggggatccgacgaacgcaggcgctgtctccccggggcccgcgtaaccccgcgcatatccgggggcacgtagaaattaccttcctcttcggactcgatatccacgacgtcaaagtcgtgggcggtcagcgagacgacctccccgtcgtcggtgatgaggacgttgtttcggcagcagcagggccgggtcccggagaacgagaggcccatagctcggcgagcgtgtcgtcgaacgccaggcggctgcttcgctgtatggccttatagatctccggatcgatgcggacgggggtaatgatcagggcgatcggaacggcctggttcgggagaatggacgccttgctgggtcctgcggccccgagagccccggcgccgtcctccaggcggaacgttacgccctcctccgcgctagtgcggtgcctgccgataaacgtcaccagatgcgggtggggggggcagtcggggaagtggctgtcgagcacgtagccctgcaccaagatctgcttaaagttcgggtgacgggggttcgcgaagacgggctcgcggcgtaccagatccccggagctccaggacacgggggagatggtgtggcgtccgaggtcgggggcgccaaacagaagcacctccgagacaacgccgctatttaactccaccaaggcccgatccgcggcggagcaccgccttttttcgcccgaggcgtgggcctctgaccaggcctggtcttgcgtgacgagagcctcctccgggccggggacgcgcccgggcgcgaagtatcgcacgctgggcttcgggatcgaccggataaatgcccggaacgcctccggggaccggtgtgccatcaagtcctcgtacgcggaggccgtggggtcgctggggtccatggggtcgaaagcgtacttggcccggcatttgacctcgtaaaaggccaggggggtcttggggactggggccaagtagccgtgaatgtcccgaggacagacgagaatatccagggacgccccgaccatccccgtgtgaccgtccatgaggaccccacacgtatgcacgttctcttcggcgaggtcgccgggttcgtggaagataaagcgccgcgtgtcggcgccggcctcgccgccgtcgtccgcgcggcccacgcagtagcgaaacagcaggcttcgggccgtcggctcgttcacccgcccgaacatcaccgccgaagactgtacatccggccgcaggctggcgttgtgcttcagccactggggcgagaaacacggaccctgggggccccagcggagggtggatgcggtcgtgaggccccgccggagcagggcccatagctggcagtcggcctggttttgcgtggccgcctcgtaaaaccccatgaggggccggggcgccacggcgtccgcggcggccgggggcccgcggcgcgtcaggcgccataggtgccggccgagtccgcggtccaccatacccgcctcctcgaggaccacggccagggaacacagataatccaggcgggcccagaggggaccgatggccagaggggcgcggacgccgcgcagcaacccgcgcaggtggcgctcgaacgtctcggctagtatatgggagggcagcgcgttggggatcaccgacgccgaccacatagagtcaaggtccggggagtcgggatcggcgtccgggtcgcgggcgtgggtgcccccaggagatagcggaatgtctggggtcggaggccctgaggcgtcagaaagtgccggcgacgcggcccggggcttttcgtctgcggtgtcggtggcgtgctgatcacgtggggggttaacgggcgaatgggagctcgggtccacagctgacgtcgtctggggtggggggggcaggggacggaaggtggttgttagcggaagactgttagggcgggggcgcttgggggggctgtcggggccacgaggggtgtcctcggccagggcccaggaacgcttagtcacggtgcgtcccggcggacatgctgggcctcccgtggactccatttccgagacgacgtggggggagcggtggttgagcgcgccgccgggtgaacgctgattctcacgacagcgcgtgccgcgcgcacgggttggtgtgacacaggcgggacaccagcaccaggagaggcttaagctcgggaggcagcgccaccgacgacagtatcgccttgtgtgtgtgctggtaatttatacaccgatccgtaaacgcgcgccgaatcttgggattgcggaggtggcgccggatgccctctgggacgtcatacgccaggccgtgggtgttggtctcggccgagttgacaaacagggctgggtgcagcacgcggcgataggcgagcagggccagggcgaagtccagcgacagctggttgttgaaatactggtaaccgggaaaccgggtcacgggtacgcccaggctcggggcgacgtacacgctaaccaccaactccagcagcgtctggccaagggcgtacaggtcaaccgctaacccgacgtcgtgcttcaggcggtggttggtaaattcggcccgttcgttgttaaggtatttcaccaacagctccgggggctggttatacccgtgacccaccagggtgtgaaagttggctgtggttagggcggtgggcatgccaaacatccggggggacttgaggtccggctcctggaggcaaaactgcccccgggcgatcgtggagttggagttgagggtgacgaggctaaagtcggcgaggacggcccgccggagcgagacggcgtccgaccgcagcatgacgaggatgttggcgcacttgatatccaggtggctgatcccgcaggtggtgtttaaaaacacaacggcgcgggccagctccgtgaagcactggtggagggccgtcgagaccgaggggtttgttgtgcgcagggacgccagttggccgatatacttaccgaggtccatgtcgtacgcggggaacactatctgtcgttgttgcagcgagaacccgaggggcgcgatgaagccgcggatgttgtgggtgcggccggcgcgtagagcgcactccccgaccaacagggtcgcgatgagctcaacggcaaaccactccttttcctttatggtcttaacggcaagcttatgttcgcgaatcagttggacgtcgccgtatcccccagaccccccgaagcttcgggccccggggatctcgagggtcgtgtagtgtagggcggggttgatggcgaacacggggctgcatagcttgcggatgcgcgtgagggtaaggatgtgcgagggggacgaggggggtgcggttaacgccgcctgggatctgcgcaggggcgggcggttcagtttggccgccgtaccgggcgtctcgggggacgcgcggcgatgagacgagcggctcattcgccatcgggatagtcccgcgcgaagccgctcgcggaggccggatcggtggcgggacccgtgggaggagcgggagccggcggcgtcctggagagaggggccgctggggcgcccggaggccccgtgtgggttggagtgtatgtaggatgcgagccaatccttgaaggactgttggcgtgcaccttgggggctgaggttagctgccacatgaccagcaggtcgctgtctgcgggactcatccatccttcggccaggtcgccgtcttcccacagagaagcgttggtcgctgcttcctcgagttgctcctcctggtccgcaagacgatcgtccacggcgtccaggcgctcaccaagcgccggatcgaggtaccgtcggtgtgcggttagaaagtcacgacgcgccgcttgctcctccacgcgaattttaacacaggtcgcgcgctgtcgcatcatctctaagcgcgcgcgggactttagccgcgcctccaattccaagtgggccgcctttgcagccataaaggcgccaacaaaccgaggatcttgggtgctgacgccctcccggtgcagctgcagggtctggtccttgtaaatctcggctcggaggtgcgtctcggccaggcgtcggcgcagggccgcgtgggcggcatctcggtccattccgccaccctgcgggcgacccggggggtgctctgatagtctcgcgtgcccaaggcccgtgatcggggtacttcgccgccgcgacccgccacccggtgtgcgcgatgtttggtcagcagctggcgtccgacgtccagcagtacctggagcgcctcgagaaacagaggcaacttaaggtgggcgcggacgaggcgtcggcgggcctcacaatgggcggcgatgccctacgagtgccctttttagatttcgcgaccgcgacccccaagcgccaccagaccgtggtcccgggcgtcgggacgctccacgactgctgcgagcactcgccgctcttctcggccgtggcgcggcggctgctgtttaatagcctggtgccggcgcaactaaaggggcgtgatttcgggggcgaccacacggccaagctggaattcctggcccccgagttggtacgggcggtggcgcgactgcggtttaaggagtgcgcgccggcggacgtggtgcctcagcgtaacgcctactatagcgttctgaacacgtttcaggccctccaccgctccgaagcctttcgccagctggtgcactttgtgcgggactttgcccagctgcttaaaacctccttccgggcctccagcctcacggagaccacgggccccccaaaaaaacgggccaaggtggacgtggccacccacggccggacgtacggcacgctggagctgttccaaaaaatgatccttatgcacgccacctactttctggccgccgtgctcctcggggaccacgcggagcaggtcaacacgttcctgcgtctcgtgtttgagatccccctgtttagcgacgcggccgtgcgccacttccgccagcgcgccaccgtgtttctcgtcccccggcgccacggcaagacctggtttctagtgcccctcatcgcgctgtcgctggcctcctttcgggggatcaagatcggctacacggcgcacatccgcaaggcgaccgagccggtgtttgaggagatcgacgcctgcctgcggggctggttcggttcggcccgagtggaccacgttaaaggggaaaccatctccttctcgtttccggacgggtcgcgcagtaccatcgtgtttgcctccagccacaacacaaacgtaagtcctcttttctttcgcatggctctcccaaggggccccgggtcgacccgacccacacccacccacccacccacatacacacacaaccagacgcgggaggaaagtctgccccgtgggcactgatttttattcgggatcgcttgaggaggcccgggcaacggcccgggcaacggtggggcaactcgtagcaaataggcgactgatgtacgaagagaagacacacaggcgccacccggcgctggtcggggggatgttgtccgcgccgcaccgtcccccgacgacctcttgcagacggtccgtgatgcaaggacggcggggggcctgcagcagggtgaccgtatccacgggatggccaaagagaagcggacacaggctagcatccccctggaccgccagggtacactgggccatcttggcccacagacacggggcgacgcagggacaggactccgttacgacggaggagagccacagtgcgttggcggaatcgatgtggggcggcggggcgcaggactcgcagccccccgggtggttggtgatcctggccaggagccatcccagatggcgggccctgcttcccggtggacagagcgaccccaggtcgctgtccatggcccagcagtagatctggccgctggggaggtgccaccaggcccccgggcccaaggcgcaacacgcgcccggctccgggggggtcttcgcggggaccagatacgcgccatccagctcgccgaccactggctcctccgcgagctgttcggtggttgggtcgggggtttcctccgggggggtggccgcccgtatgcgggcgaacgtgagggtgcacaggagcggggtcagggggtgcgtcacgctccggaggtggacgatcgcgcagtagcggcgctcgcggttaaagaaaaagagggcaaagaaggtgttcgggggcaaccgcagcgccttggggcgcgtcagatacagaaaaatctcgcagaagagggcgcgcccggggtctgggttaggaagggccacctgacacagaggctcggtgaggaccgttagacaccgaaagatcttgagccgctcgtccgcccgaacgacgcgccacacaaagacggagttgacaatgcgcgcgatagagtcgacgtccgtccccaggtcgtcgactctgtcgcgcgtgccgcgagctccggcccgggaatccggccggggcaaggtccccgggggaccaggcggcgccaggggccgccggggtcccagctgcgccatgccgggggcggggggagggcaaaccccagaggcgggggccaacggcgcggggaggagtgggtgggcgaggtggccgggggaaggcgcccgctagcgagaacggccgttcccggacgacaccttgcgacaaaacctaaggacagcggcccgcgcgacggggtccgagaggctaaggtaggccgcgatgttaatggtgaacgcaaagccgccgggaaagacaactatgccacagaggcggcgattaaaccccaggcagaggtaggcgtagctttccccgggcaggtattgctcgcagaccctgcgtggggctgtggaggggacggcctccatgaagcgacatttactctgctcgcgtttactgacgtcaccatccatcgccacggcgattggacgattgttaagccgcagcgtgtctccgcttgtgctgtagtagtcaaaaacgtaatggccgtcggagtcggcaaagcgggccgggaggtcgtcgccgagcgggacgacccgccgcccccgaccgccccgtccccccaggtgtgccaggacggccagggcatacgcggtgtgaaaaaaggcgtcgggggcggtcccctcgacggcgcgcatcaggttctcgaggagaatggggaagcgcctggtcacctcccccagccacgcgcgttggtcggggccaaagtcatagcgcaggcgctgtgagattcgagggccgccctgaagcgcggcccggatggcctggcccagggcccggaggcacgccagatgtatgcgcgcagtaaaggcgacctcggcggcgatgtcaaagggcggcaggacggggcgcgggtggcgcaggggcacctcgagcgcgggaaagcggagcagcagctccgcctgcccagcgggagacagctggtgggggcgcacgacgcgttctgcggcgcaggcctcggtcagggccgtggccagcgccgaggacagcagcggagggcgggcgcgtcgcccgccccacgccacggagttctcgtaggagacgacgacgaagcgctgcttggttccgtagtggtggcgcaggaccacggagatagaacgacggctccacagccagtccggccggtcgccgccggccagggcttcccatccgcgatccaaccactcgaccagcgaccgcggctttgcggtaccaggggtcagggttagaacgtcgttcaggatgtcctcgcccccgggcccgtggggcactggggccacaaagcggcccccgcctgggggctccagacccgccaacaccgcatctgcgtcagccgcccccatggcgcccccgctgacggcctggtgaaccagggcgccctggcggagccccgatgcaacgccacaggccgcacgcccggtccgagcgcggaccgggtggcggcgggtgacgtcctgcactgcccgctgaaccaacgcgaggatctcctcgttctcctgcgcgatggacacgtcctgggccgcggtcgtgtcgccgccgggggccgtcagctgctcctccggggagatgggggggtcggacgccccgacgatgggcgggtctgcgggcgcccccgcgtggggccgggccaagggctgcggacgcggggacgcgctttcccccagacccatggacaggtgggccgcagcctccttcgcggccggcggggcggcggcgccaagcagagcgacgtagcggcacaaatgccgacagacgcgcatgatgcgcgtgctgtcggccgcgtagcgcgtgttgggggggacgagctcgtcgtaactaaacagaatcacgcgggcacagctcgcccccgagccccacgcaaggcgcagcgccgccacggcgtacgggtcatagacgccctgtgcgtcacacaccacgggcaaggagacgaacaaccccccggcgctggacgcacgcggaaggaggccagggtgtgccggcacgacgggggccagaagctcccccaccgcatccgcgggcacgtaggcggcaaacgccgtgcaccacggggtacagtcgccggtggcatgagcccgagtctggatttcgacctggaagtttgcggccgtcccgagtccggggcggccgcgcatcagggcggccagagggattcccgcggccgccaggcactcgctggatatgatgacgtgaaccaaagacgagggccgacccgggacgtggccgagatcgtactggacctcgttggccaagtgcgcgttcatggttcgggggtgggtgtgggtgtgtaggcgatgcgggtcccccgagtccgcgggaagggcgcgggtttggcgcgcgtatgcgtattcgccaacggaggcgtgcgtgcttatgcgcggcgcgtttcttctgtctccagggaatccgaggccaggactttaacctgctctttgtcgacgaggccaactttattcgcccggatgcggtccagacgattatgggctttctcaaccaggccaactgcaagattatcttcgtgtcgtccaccaacaccgggaaggccagtacgagctttttgtacaacctccgcggggccgccgacgagcttctcaacgtggtgacctatatatgcgatgatcacatgccgcgggtggtgacgcacacaaacgccacggcctgttcttgttatatcctcaacaagcccgttttcatcacgatggacggggcggttcgccggaccgccgatttgtttctggccgattccttcatgcaggagatcatcgggggccaggccagggagaccggcgacgaccggcccgttctgaccaagtctgcgggggagcggtttctgttgtaccgcccctcgaccaccaccaacagcggcctcatggcccccgatttgtacgtgtacgtggatcccgcgttcacggccaacacccgagcctccgggaccggcgtcgctgtcgtcgggcggtaccgcgacgattatatcatcttcgccctggagcacttttttctccgcgcgctcacgggctcggcccccgccgacatcgcccgctgcgtcgtccacagtctgacgcaggtcctggccctgcatcccggggcgtttcgcggcgtccgggtggcggtcgagggaaatagcagccaggactcggccgtcgccatcgccacgcacgtgcacacagagatgcaccgcctactggcctcggagggggccgacgcgggctcgggccccgagcttctcttctaccactgcgagcctcccgggagcgcggtgctgtacccctttttcctgctcaacaaacagaagacgcccgcctttgaacactttattaaaaagtttaactccgggggcgtcatggcctcccaggagatcgtttccgcgacggtgcgcctgcagaccgacccggtcgagtatctgctcgagcagctgaataacctcaccgaaaccgtctcccccaacacggacgtccgtacgtattccggaaaacggaacggcgcctcggatgaccttatggtcgccgtcattatggccatctaccttgcggcccaggccggacctccgcacacattcgctcccatcacacgcgtttcgtgagcgcccaataaacacacccaggtatgctacgcacgaccacggtgtcgcctgttaagggggggggaagggggtgttggcgggaagcgtgggaacacgggggattctctcacgaccggcaccagtaccacccccctgtgaacacagaaaccccaacccaaatcccataaacatacgacacacaggcatattttggaatttcttaggtttttatttatttaggtatgctggggtttctccctggatgcccacccccacccccccccgtgggtctagccgggccttagggatagcgtataacgggggccatgtctccggaccgcacaacggccgcgccgtcaaaggtgcacacccgaaccacgggagccagggccaaggtgtctcctagttggcccgcgtgggtcagccaggcgacgagcgcctcgtagagcggcagccttcgctctccatcctgcatcagggccggggcttcggggtgaatgagctgggcggcctcccgcgtgacactctgcatctgcaggagagcgttcacgtacccgtcctgggcacttagcgcaaagagccgggggattagcgtaaggatgatggtggttccctccgtgatcgagtaaaccatgttaaggaccagcgatcgcagctcggcgtttacggggccgagttgttggacgtccgccagcagcgagaggcgactcccgttgtagtacagcacgttgaggtctggcagccctccggggtttctggggctggggttcaggtcccggatgcccctggccacgagccgcgccacgatttcgcgcgccaggggcgatggaagcggaacgggaaaccgcaacgtgaggtccagcgaatccaggcgcacgtccgtcgcttggccctcgaacacgggcgggacgaggctgatggggtccccgttacagagatctacgggggaggtgttgcgaaggttaacggtgccggcgtgggtgaggcccacgtccagggggcaggcgacgattcgcgtgggaagcacccgggtgatgaccgcggggaagcgccttcggtacgccagcaacagccccaacgtgtcgggactgacgcctccggagacgaaggattcgtgcgccacgtcggccagcgtcagttgccggcggatggtcggcaggaataccacccgcccttcgcagcgctgcagcgccgccgcatcggggcgcgagatgcccgagggtatcgcgatgtcagtttcaaagccgtccgccagcatggcgccgatccacgcggcagggagtgcagtggtggttcgggtggcgggaggagcgcggtgggggtcagcggcgtagcagagacgggcgaccaacctcgcataggacggggggtgggtcttagggggttgggaggcgacagggaccccagagcatgcgcggggaggtctgtcgggcccagacgcaccgagagcgaatccgtccatggagtcccggcctgggttttatggggcccggccctcggaatcgcggcttgtcggcggggacaaagggggcggggctagggggcttgcggaaacagaagacgtgtgggataaaagaatcgcactaccccaaggaagggcggggcggtttattacagagccagtcccttgagcggggatgcgtcatagacgagatactgcgcgaagtgggtctcccgcgcgtgggcttccccgttgcgggcgctgcggaggagggcggggtcgctggcgcaggtgagcgggtaggcctcctgaaacaggccacacgggtcctccacgagttcgcggcaccccggggggcgcttaaactgtacgtcgctggcggcggtggccgtggacaccgccgaacccgtctccacgatcaggcgctccaggcagcgatgtttggcggcgatgtcggccgacgtaaagaacttaaagcaggggctgagcaccggcgaggccccgttgaggtggtaggccccgttatagagcaggtccccgtacgaaaatcgctgcgacgcccacgggttggccgtggccgcgaaggcccgggacgggtcgctctggccgtggtcgtacatgagggcggtgacatccccctccttgtcccccgcgtaaacgcccccggcggcgcgtccccgggggttgcagggccggcggaagtagttgacgtcggtcgacacgggggtggcgataaactcacacacggcgtcctggccgtggtccatccctgcgcgccgcggcacctgggcgcacccgaacacggggacgggctgggccggccccaggcggtttcccgccacgaccgcgttccgcaggtacacggctgccgcgttgtccagtagagggggagccccgcggcccaggtaaaagttttggggaaggttgcccatgtcggtgacggggttgcggacggttgccgtggccacgacggcggtgtagcccacgcccaggtccacgttcccgcgcggctgggtgagcgtgaagtttacccccccgccagtttcatgccgggccacctggagctggcccaggaagtacgcctccgacgcgcgctccgagaacagcacgttctcagtcacaaagcggtcctgtcggacgacggtgaacccaaacccgggatggaggcccgtcttgagctgatgatgcaaggccacgggactgatcttgaagtaccccgccatgagcgcgtaggtcagcgcgttctccccggccgcgctctcgcggacgtgctgcacgacgggctgtcggatcgacgaaaagtagttggcccccagagccggggggaccagggggacctgccgcgacaggtcgcgcagggccggggggaaattgggcgcgttcgccacgtggtcggccccggcgaacagcgcgtggacggggagggggtaaaaatagtcgccattttggatggtatggtccagatgctggggggccatcagcaggattccggcgtgcaacgccccgtcgaatatgcgcatgttggtggtggacgcggtgttggcgcccgcgtcgggcgccgccgagcagagcagcgccgttgtgcgttcggccatgttgtgggccagcacctgcagcgtgagcatggcgggcccgtccactaccacgcgcccgttgtgaaacatggcgttgaccgtgttggccaccagattggccgggtgcagggggtgcgcggggtccgtcacggggtcgctggggcaatcctcgccgggggtgatctccgggaccaccatgttctgcagggtggcgtatacgcggtcgaagcgaacccccgcggtgcagcagcggccccgcgagaaggcgggcaccatcacgtagtagtaaatcttgtggtgcacggtccagtccgccccccggtgcggccggtcgtccgcggcgtccgcggctcgggcctgggtgttgtgcagcagctggccgtcgttgcggttgaagtccgcggtcgccacgttacacgccgctgcgtacacggggtcgtggccccccgcgctaacccggcagtcgcgatggcggtccagggccgcgcgccgcatcagggcgtcgcagtcccacacgaggggtggcagcagcgccgggtctcgcattaggtgattcagttcggcttgcgcctgcccgcccagttccgggccggtcagggtaaagtcatcaaccagctgggccagggcctcgacgtgcgccaccaggtcccggtacacggccatgcactcctcgggaaggtctcccccgaggtaggtcacgacgtacgagaccagcgagtagtcgttcacgaacgccgcgcaccgcgtgttgttccagtagctggtgatgcactggaccacgagccgggccagggcgcagaagacgtgctcgctgccgtgtatggcggcctgcagcaggtaaaacaccgccgggtagttgcggtcttcgaacgccccgcgaacggcggcgatggtggcgggggccatggcgtggcgtcccacccccagctccaggccccgggcgtcccggaacgccgccggacatagcgccaggggcaagttgccgttcaccacgcgccaggtggcctggatctcccccgggccggccgggggaacgtccccccccggcagctccacgtcggccacccccacgaagaagtcgaacgcggggtgcagctcaagagccaggttggcgttgtcgggctgcataaactgctccggggtcatctggccttccgcgacccatcggacccgcccgtgggccaggcgctgcccccaggcgttcaaaaacagctgctgcatgtctgcggcggggccggccggggccgccacgtacgccccgtacggattggcggcttcgacggggtcgcggttaaggcccccgaccgccgcgtcaacgttcatcagcgaagggtggcacacggtcccgatcgcgtgttccagagacaggcgcagcacctggcggtccttcccccaaaaaaacagctggcggggcgggaaggcgcggggatccgggtggccgggggcggggactaggtccccggcgtgcgcggcaaaccgttccatgaccggattgaacaggcccaggggcaggacgaacgtcaggtccatggcgcccaccagggggtagggaacgttggtggcggcgtagatgcgcttctccagggcctccaaaaagatcagcttctcgccgatggacaccagatccgcgcgcacgcgcgtcgtctggggggcgctctcgagctcgtccagcgtctgccggttcaggtcgagctgctcctcctgcatctccagcaggtggcggcccacgtcgtccagacttcgcacggccttgcccatcacgagcgccgtgaccaggttggccccgttcaggaccatctcgccgtacgtcaccggcacgtcggcttcggtgtcctccactttcaggaaggactgcaggaggcgctgtttgatcggggcggtggtgacgagcaccccgtcgaccggacgcccgcgcgtgtcggcatgcgtcagacggggcacggccacggagggctgcgtggccgtggtgaggtccacgagccaggcctcgacggcctcccggcggtggcccgccttgcccaggaaaaagctcgtctcgcagaagcttcgctttagctcggcgaccagggtcgcccgggccaccctggtggccaggcggccgttgtccaggtatcgttgcatcggcaacaacaaagccaggggcggcgccttttccagcagcacgtgcagcatctggtcggccgtgccgcgctcaaacgccccgaggacggcctggacgttgcgagcgagctgttggatggcgcgcaactggcgatgcgcgctgatacccgtcccgtccagggcctcccccgtgagcagggcgatggcctcggtggccaggctgaaggcggcgttcagggcccggcggtcgataatcttggtcatgtaattgtgtgtgggttgctcgatggggtgcgggccgtcgcgggcaatcagcggctggtggacctcgaactgtacgcgcccctcgttcatgtaggccagctccggaaacttggtacacacgcacgccaccgacaacccgagctccagaaagcgcacgagcgacagggtgttgcaatacgaccccaacagggcgtcgaactcgacgtcatacaggctgtttgcatcggagcgcacgcgggaaaaaaaatcgaacaggcgtcgatgcgacgccacctcgatcgtgctaaggagggacccggtcggcaccatggccgcggcataccggtatcccggagggtcgcggttgggagcggccatggggtcgcgtggagatcggctgtctctagcgatattggcccggggaggctaagatccaccccaacgcccggccacccgtgtacgtgcccgacggcccaaggtccaccgaaagacacgacgggcccggacccaaaaaggcgggggatgctgtgtgagaggccgggtgtcggtcgggggggaaaggcaccgggagaaggctgcggcctcgttccaggagaacccagtgtccccaacagacccggggacgtgggatcccaggccttatataccccccccgccccacccccgttagaacgcgacgggtgcattcaagatggccctggtccaaaagcgtgccaggaagaaattggcagaggcggcaaagctgtccgccgccgccacccacatcgaggccccggccgcgcaggctatccccagggcccgtgtgcgcaggggatcggtgggcggcagcatttggttggtggcgataaagtggaaaagcccgtccggactgaaggtctcgtgggcggcggcgaacaaggcacacagggccgtgcctcccaaaaacacggacatcccccaaaacacgggcgccgacaacggcagacgatccctcttgatgttaacgtacaggaggagcgcccgcaccgcccacgtaacgtagtagccgacgatggcggccaggatacaggccggcgccaccacccttccggtcagcccgtaatacatgcccgctgccaccatctccaacggcttcaggaccaaaaacgaccaaaggaacagaatcacgcgctttgaaaagaccggctgggtatggggcggaagacgcgagtatgccgaactgacaaaaaagtcagaggtgccgtacgaggacaatgaaaactgttcctccagtggcagttctccctcctcccccccaaaggcggcctcgtcgaccagatctcgatccaccagaggaaggtcatcccgcatggtcatggggtgtgcggtggaggtggggagaccgaaaccgcaaagggtcgcttacgtcagcaggatcccgagatcaaagacacccgggttcttgcacaaacaccacccgggttgcatccgcggaggcgagtgttttgataaggccgttccgcgccttgatataacctttgatgttgaccacaaaacccggaatttacgcctacgccccaatgcccacgcaagatgaggtaggtaaccccccccccgtgggtgtgacgttgcgtttagttcattggaggccaaggggaaaatggggtggggaggaaacggaaaacccagtaggccgtgttgggaacacgcccggggttgtcctcaaaaggcagggtccatactacggaagccgtcgttgtattcgagacctgcctgtgcgacgcacgtcggggttgcctgtgtccggttcggccccaccgcgtgcggcacgcacgaggacgagtccgcgtgctttattggcgttccaagcgttgccctccagtttctgttgtcggtgttcccccatacccacgcccacatccaccgtagggggcctctgggccgtgtcacgtcgccgcccgcgatggagcttagctacgccaccaccatgcactaccgggacgttgtgttttacgtcacaacggaccgaaaccgggcctactttgtgtgcggggggtgtgtttattccgtggggcggccgtgtgcctcgcagcccggggagattgccaagtttggtctggtcgttcgagggacaggcccagacgaccgcgtggtcgccaactatgtacgaagcgagctccgacaacgcggcctgcaggacgtgcgtcccattggggaggacgaggtgtttctggacagcgtgtgtcttctaaacccgaacgtgagctccgagctggatgtgattaacacgaacgacgtggaagtgctggacgaatgtctggccgagtactgcacctcgctgcgaaccagcccgggtgtgctaatatccgggctgcgcgtgcgggcgcaggacagaatcatcgagttgtttgaacacccaacgatagtcaacgtttcctcgcactttgtgtataccccgtccccatacgtgttcgccctggcccaggcgcacctcccccggctcccgagctcgctggaggccctggtgagcggcctgtttgacggcatccccgccccacgccagccacttgacgcccacaacccgcgcacggatgtggttatcacgggccgccgcgccccacgacccatcgccgggtcgggggcggggtcggggggcgcgggcgccaagcgggccaccgtcagcgagttcgtgcaagtcaaacacattgaccgcgtgggccccgctggcgtttcgccggcgcctccgccaaacaacaccgactcaagttccctggtgcccggggcccaggattccgccccgcccggccccacgctaagggagctgtggtgggtgttttatgccgcagaccgggcgctggaggagccccgcgccgactctggcctcacccgcgaggaggtacgtgccgtacgtgggttccgggagcaggcgtggaaactgtttggctccgcgggggccccgcgggcgtttatcggggccgcgttgggcctgagccccctccaaaagctagccgtttactactatatcatccaccgagagaggcgcctgtcccccttccccgcgctagtccggctcgtaggccggtacacacagcgccacggcctgtacgtccctcggcccgacgacccagtcttggccgatgccatcaacgggctgtttcgcgacgcgctggcggccggaaccacagccgagcagctcctcatgttcgaccttctccccccaaaggacgtgccggtgggaagcgacgtgcaggccgacagcaccgctctgctgcgctttatagaatcgcaacgtctcgccgtccccgggggggtgatctcccccgagcacgtcgcgtaccttggtgcgttcctgagcgtgctgtacgctggccgcgggcgcatgtccgcagccacgcacaccgcgcggctgacaggggtgacctccctggtgctagcggtgggtgacgtggaccgtctttccgcgtttgaccgcggagcggcgggcgcggccagccgcacgcgggccgccgggtacctggatgtgcttcttaccgttcgtctcgctcgctcccaacacggacagtctgtgtaacagaccccaataaacgtatgtcgctaccacacccttgtgtgtcaatggacgcctctccgggggggaagggaaaacaaagaggggctgggggagcggcaccaccggggcctgaacaaacaaaccacagacacggttacagtttattcggtcgggcggagaaacggccgaagccacgccccctttattcgcgtctccaaaaaaacgggacacttgtccggagaacctttaggatgccagccagggcggcggtaatcataaccacgcccagcgcagaggcggccagaaacccgggcgcaattgcggccacgggctgcgtgtcaaaggctagcaaatgaatgacggttccgtttggaaatagcaacaaggccgtggacggcacgtcgctcgaaaacacgcttggggcgccctccgtcggcccggcggcgatttgctgctgtgtgttgtccgtatccaccagcaacacagacatgacctccccggccggggtgtagcgcataaacacggcccccacgagccccaggtcgcgctggttttgggtgcgcaccagccgcttggactcgatatcccgggtggagccttcgcatgtcgcggtgaggtaggttaggaacagtgggcgtcggacgtcgacgccggtgagcttgtagccgatcccccggggcagaggggagtgggtgacgacgtagctggcgttgtgggtgatgggtaccaggatccgtggctcgacgttggcagactgccccccgcaccgatgtgaggcctcagggacgaaggcgcggatcagggcgttgtagtgtgcccagcgcgtcagggtcgaggcgaggccgtgggtctgctgggccaggacttcgaccggggtctcggatcgggtggcttgagccagcgcgtccaggataaacacgctctcgtctagatcaaagcgcagggaggccgcgcatggcgaaaagtggtccggaagccaaaagagggttttctggtggtcggcccgggccagcgcggtccggaggtcggcgttggtcgctgcggcgacgtcggacgtacacagggccgaggctatcagaaggctccggcgggcgcgttcccgctgcaccgccgaggggacgcccgccaagaacggctgccggaggacagccgaggcgtaaaatagcgcccggtggacgaccggggtggtcagcacgcggccccctagaaactcggcatacagggcgtcgatgagatgggctgcgctgggcgccactgcgtcgtacgccgaggggctatccagcacgaaggccagctgatagcccagcgcgtgtaatgccaagctctgttcgcgctccagaatctcggccaccaggtgctggagccgagcctctagctgcaggcgggccgtgggatccaagactgacacattaaaaaacacagaatccgcggcacagcccgcggccccgcgggcggccaacccggcaagcgcgcgcgagtgggccaaaaagcctagcaggtcggagaggcagaccgcgccgtttgcgtgggcggcgttcacgaaagcaaaacccgacgtcgcgagcagccccgttaggcgccagaagagagggggacgcgggccctgctcggcgcccgcgtcccccgagaaaaactccgcgtatgcccgcgacaggaactgggcgtagttcgtgccctcctccgggtagccgcccacgcggcggagggcgtccagcgcggagccgttgtcggcccgcgtcagggaccctaggacaaagacccgataccgggggccgcccgggggcccgggaagagcccccggggggttttcgtccgcggggtccccgacccgatctagcgtctggcccgcggggaccaccatcacttccaccggagggctgtcgtgcatggatatcacgagccccatgaattcccgcccgtagcgcgcgcgcaccagcgcggcatcgcacccgagcaccagctcccccgtcgtccagatgcccacgggccacgtcgaggccgacggggagaaatacacgtacctacctggggatctcaacaggccccgggtggccaaccaggtcgtggacgcgttgtgcaggtgcgtgatgtccagctccgtcgtcgggtgccgccgggccccaaccggcggtcgggggggcggtgtatcacgcggcccgctcgggtggctcgccgtcgccacgttgtctccccgcgggaacgtcagggcctcggggtcagggacggccgaaaacgttacccaggcccgggaacgcagcaacacggaggcggttggattgtgcaagagacccttaaggggggcgaccgcggggggaggctgggcggtcggctcgaccgtgatgggggcgggcaggctcgcgttcgggggccggccgagcaggtaggtcttcgagatgtaaagcagctggccggggtcccgcggaaactcggccgtggtgaccaatacaaaacaaaagcgctcctcgtaccagcgaagaaggggcagagatgccgtagtcaggtttagttcgtccggcggcgccagaaatccgcgcggtggtttttgggggtcgggggtgtttggcagccacagacgcccggtgttcgtgtcgcgccagtacatgcggtccatgcccaggccatccaaaaaccatgggtctgtctgctcagtccagtcgtggacctgaccccacgcaacgcccaaaagaataacccccacgaaccataaaccattccccatgggggaccccgtccctaacccacggggcccgtggctatggcagggcttgccgccccgacgttggctgcgagccctgggccttcacccgaacttgggggttggggtggggaaaaggaagaaacgcgggcgtattggccccaatggggtctcggtggggtatcgacagagtgccagccctgggaccgaaccccgcgtttatgaacaaacgacccaacacccgtgcgttttattctgtctttttatttccgtcatagcgcgggttccttccggtattgtctccttccgtgtttcagttagcctcccccatctcccgggcaaacgtgcgcgccaggtcgcagatcgtcggtatggagcctggggtggtgacgtgggtctggaccatcccggaggtaagttgcagcagggcgtcccggcagccggcgggcgattggtcgtaatccaggataaagacgtgcatgggacggaggcgtttggccaagacgtccaaggcccaggcaaacacgttatacaggtcgccgttgggggccagcaactcgggggcccgaaacagggtaaataacgtgtccccgatatggggtcgtgggcccgcgttgctctggggctcggcaccctggggcggcacggccgtccccgaaagctgtccccaatcctcccgccacgacccgccgccctgcagataccgcaccgtattggcaagcagcccgtaaacgcggcgaatcgcggccaacatagccaggtcaagccgctcgccggggcgctggcgtttggccaggcggtcgatgtgtctgtcctccggaagggcccccaacacgatgtttgtgccgggcaaggtcggcgggatgagggccacgaacgccagcacggcctggggggtcatgctgcccataaggtatcgcgcggccgggtagcacaggagggcggcgatgggatggcggtcgaagatgagggtgagggccgggggcggggcatgtgagctcccagcctcccccccgatatgaggagccagaacggcgtcggtcacggcataaggcatgcccattgttatctgggcgcttgtcattaccaccgccgcgtccccggccgatatctcaccctggtcgaggcggtgttgtgtggtgtagatgttcgcgattgtctcggaagcccccagcacctgccagtaagtcatcggctcgggtacgtagacgatatcgtcgcgcgaacccagggccaccagcagttgcgtggtggtggttttccccatcccgtgaggaccgtctatataaacccgcagtagcgtgggcattttctgctccaggcggacttccgtggcttcttgctgccggcgagggcgcaacgccgtacgtcggttgctatggccgcgagaacgcgcagcctggtcgaacgcagacgcgtgttgatggcaggggtacgaagccatacgcgcttctacaaggcgcttgccaaagaggtgcgggagtttcacgccaccaagatctgcggcacgctgttgacgctgttaagcgggtcgctgcagggtcgctcggtgttcgaggccacacgcgtcaccttaatatgcgaagtggacctgggaccgcgccgccccgactgcatctgcgtgttcgaattcgccaatgacaagacgctgggcggggtttgtgtcatcatagaactaaagacatgcaaatatatttcttccggggacaccgccagcaaacgcgagcaacgggccacggggatgaagcagctgcgccactccctgaagctcctgcagtccctcgcgcctccgggtgacaagatagtgtacctgtgccccgtcctggtgtttgtcgcccaacggacgctccgcgtcagccgcgtgacccggctcgtcccgcagaaggtctccggtaatatcaccgcagtcgtgcggatgctccagagcctgtccacgtatacggtccccatggagcctaggacccagcgagcccgtcgccgccgcggcggcgctgcccgggggtctgcgagcagaccgaaaaggtcacactctggggcgcgcgacccgcccgagccagcggcccgccaggtaccacccgccgaccaaacccccgcctccacggagggcgggggggtgcttaagaggatcgcggcgctcttctgcgtgcccgtggccaccaagaccaaaccccgagctgcctccgaatgagagtgtttcgttccttccccctccccccgcgtcagacaaaccctaaccaccgcttaagcggcccccgcgaggtccgaagactcatttggatccggcgggagccacctgacaacagcccccgggtttccccacgccagacgccggtccgctgtgccatcgctccccttcatcccacccccatcttgtccccaaataaaacaaggtctggtagttaggacaacgaccgcagttctcgtgtgttattgtcgctctccgcctctcgcagatggacccgtattgcccatttgacgctctggacgtctgggaacacaggcgcttcatagtcgccgattcccgaaacttcatcacccccgagttcccccgggacttttggatgtcgcccgtctttaacctcccccgggagacggcggcggagcaggtggtcgtcctgcaggcccagcgcacagcggctgccgctgccctggagaacgccgccatgcaggcggccgagctccccgtcgatatcgagcgccggttacgcccgatcgaacggaacgtgcacgagatcgcaggcgccctggaggcgctggagacggcggcggccgccgccgaagaggcggatgccgcgcgcggggatgagccggcgggtgggggcgacgggggggcgcccccgggtctggccgtcgcggagatggaggtccagatcgtgcgcaacgacccgccgctacgatacgacaccaacctccccgtggatctgctacatatggtgtacgcgggccgcggggcgaccggctcgtcgggggtggtgttcgggacctggtaccgcactatccaggaccgcaccatcacggactttcccctgaccacccgcagtgccgactttcgggacggccggatgtccaagaccttcatgacggcgctggtcctgtccctgcagtcgtgcggccggctgtatgtgggccagcgccactattccgccttcgagtgcgccgtgttgtgtctctacctgctgtaccgaaacacgcacggggccgccgacgatagcgaccgcgctccggtcacgttcggggatctgctgggccggctgccccgctacctggcgtgcctggccgcggtgatcgggaccgagggcggccggccacagtaccgctaccgcgacgacaagctccccaagacgcagttcgcggccggcgggggccgctacgaacacggagcgctggcgtcgcacatcgtgatcgccacgctgatgcaccacggggtgctcccggcggccccgggggacgtcccccgggacgcgagcacccacgttaaccccgacggcgtggcgcaccacgacgacataaaccgcgccgccgccgcgttcctcagccggggccacaacctattcctgtgggaggaccagactctgctgcgggcaaccgcgaacaccataacggccctgggcgttatccagcggctcctcgcgaacggcaacgtgtacgcggaccgcctcaacaaccgcctgcagctgggcatgctgatccccggagccgtcccttcggaggccatcgcccgtggggcctccgggtccgactcgggggccatcaagagcggagacaacaatctggaggcgctatgtgccaattacgtgcttccgctgtaccgggccgacccggcggtcgagctgacccagctgtttcccggcctggccgccctgtgtcttgacgcccaggcggggcggccggtcgggtcgacgcggcgggtggtggatatgtcatcgggggcccgccaggcggcgctggtgcgcctcaccgccctggaactcatcaaccgcacccgcacaaaccccacccccgtgggggaggttatccacgcccacgacgccctggcgatccaatacgaacaggggcttggcctgctggcgcagcaggcacgcattggcttgggctccaacaccaagcgtttctccgcgttcaacgttagcagcgactacgacatgttgtactttttatgtctggggttcattccacagtacctgtcggcggtttagtgggtggtgggcgaggggggagggggcattagggagaaagaacaagagcctccgttgggttttctttgtgcctgtactcaaaaggtcataccccgtaaacggcgggctccagtcccggcccggcggttggcgtgaacgcaacggcgggagctgggttagcgtttagtttagcattcgctctcgcctttccgcccgcccccgaccgttgagcctttttttttttcgtccaccaaagtctctgtgggtgcgcgcatggcagccgatgccccgggagaccggatggaggagcccctgccagacagggccgtgcccatttacgtggctgggtttttggccctgtatgacagcggggactcgggcgagttggcattggatccggatacggtgcgggcggccctgcctccggataacccactcccgattaacgtggaccaccgcgctggctgcgaggtggggcgggtgctggccgtggtcgacgacccccgcgggccgttttttgtgggactgatcgcctgcgtgcaactggagcgcgtcctcgagacggccgccagcgctgcgattttcgagcgccgcgggccgccgctctcccgggaggagcgcctgttgtacctgatcaccaactacctgccctcggtctccctggccacaaaacgcctggggggcgaggcgcaccccgatcgcacgctgttcgcgcacgtagcgctgtgcgcgatcgggcggcgccttggcactatcgtcacctacgacaccggtctcgacgccgccatcgcgccctttcgccacctgtcgccggcgtctcgcgagggggcgcggcgactggccgccgaggccgagctcgcgctatccggacgcacctgggcgcccggcgtggaggcgctgacccacacgctgctttccaccgccgttaacaacatgatgctgcgggaccgctggagcctggtggccgagcggcggcggcaggccgggatcgccggacacacctacctccaggcgagcgaaaaattcaaaatgtggggggcggagcctgtttccgcgccggcgcgcgggtataagaacggggccccggagtccacggacataccgcccggctcgatcgctgccgcgccgcagggtgaccggtgcccaatcgtccgtcagcgcggggtcgcctcgcccccggtactgccccccatgaaccccgttccaacatcgggcaccccggcccccgcgccgcccggcgacgggagctacctgtggatcccggcctcccattacaaccagctcgtcgccggccacgccgcgccccaaccccagccgcattccgcgtttggtttcccggctgcggcgggggccgtggcctatgggcctcacggcgcgggtctttcccagcattaccctccccacgtcgcccatcagtatcccggggtgctgttctcgggacccagcccactcgaggcgcagatagccgcgttggtgggggccatagccgcggaccgccaggcgggcggtcagccggccgcgggagaccctggggtccgggggtcgggaaagcgtcgccggtacgaggcggggccgtcggagtcctactgcgaccaggacgaaccggacgcggactacccgtactaccccggggaggctcgaggcgggccgcgcggggtcgactctcggcgcgcggcccgccagtctcccgggaccaacgagaccatcacggcgctgatgggggcggtgacgtctctgcagcaggaactggcgcacatgcgggctcggaccagcgccccctatggaatgtacacgccggtggcgcactatcgccctcaggtgggggagccggaaccaacaacgacccacccggccctttgtcccccggaggccgtgtatcgccccccaccacacagcgccccctacggtcctccccagggtccggcgtcccatgcccccactcccccgtatgccccagctgcctgcccgccaggcccgccaccgcccccatgtccttccacccagacgcgcgcccctctaccgacggagcccgcgttcccccccgccgccaccggatcccaaccggaggcatccaacgcggaggccggggcccttgtcaacgccagcagcgcagcacacgtggacgttgacacggcccgcgccgccgatttgttcgtctctcagatgatgggggcccgctgattcgccccggtctttggtaccatgggatgtcttactgtatatctttttaaataaaccaggtaataccaaataagacccattggtgtatgttctttttttattgggaggggcgggtaggcgggtagctttacaatgcaaaagcctttgacgtggaggaaggcgtgggggggaggaaatcggcactgaccaagggggtccgttttgtcacgggaaaggaaagaggaaacaggccgcggacacccgggggagtttatgtgttcctttttctttcttcccacacacacacaaaaggcgtaccaaacaaaaaaaccaaaagatgcgcatgcggtttaacacccgtggtttttatttacaacaaaccccccgtcacaggtcgtcctcgtcggcgtcaccgtctttgttgggaacttgggtgtagttggtgttgcggcgcttgcgcatgaccatgtcggtgaccttggcgctgagcagcgcgctcgtgcccttcttcttggccttgtgttccgtgcgctccatggccgacaccagggccatgtaccgtatcatctccctggcctcggctagcttggcctcgtcaaagtcgccgccctcctcgccctccccggacgcgtccgggttggtggggttcttgagctccttggtggttagagggtacagggccttcatggggttgctctgcagccgcatgacgtaacgaaaggcgaagaaggccgccgccaggccggccaggaccaacagacccacggccagcgccccaaaggggttggacatgaaggaggacacgcccgacacggccgataccacgccgcccacgatgcccatcaccaccttgccgaccgcgcgccccaggtcgcccatcccctcgaagaacgcgcccaggcccgcgaacatggcggcgttggcgtcggcgtggatgaccgtgtcgatgtcggcgaagcgcaggtcgtgcagctggttgcggcgctggacctccgtgtagtccagcaggccgctgtccttgatctcgtggcgggtgtacacctccagggggacaaactcgtgatcctccagcatggtgatgttgaggtcgatgaaggtgctgacggtggtgatgtcggcgcggctcagctggtgggagtacgcgtactcctcgaagtacacgtagcccccaccgaaggtgaagtagcgccggtgtcccacggtgcacggctcgatcgcatcgcgcgtcagccgcagctcgttgttctcccccagctgcccctcgaccaacgggccctggtcttcgtaccgaaagctgaccagggggcggctgtagcaggccccgggccgcgagctgatgcgcatcgagttttggacgatcacgttgtccgcggcgaccggcacgcacgtggagacggccatcacgtcgccgagcatccgcgcgctcacccgccggcccacggtgaccgaggcgatggcgttggggttcagcttgcgggcctcgttccacagggtcagctcgtgattctgtagctcgcaccacgcgatggcaacgcggcccaacatatcgttgacatggcgctgtatgtggttgtacgtaaactgcagccgggcgaactcgatggaggaggtggtcttgatgcgctccacggacgcgttggcgctggccccgggcggcgggggcgtggggtttgggggcttgcggctctgctctcggaggtgttcccgcacgtacagctccgcgagcgtgttgctgagaaggggctggtacgcgatcagaaagcccccattggccaggtagtactgcggctggcccaccttgatgtgcgtcgcgttgtacctgcgggcgaagatgcggtccatggcgtcgcgggcgtccttgccgatgcagtcccccaggtccacgcgcgagagcgggtactcggtcaggttggtggtgaaggtggtggatatggcgtcggaggagaatcggaaggagccgccgtactcggagcgcagcatctcgtccacttcctgccacttggtcatggtgcagaccgacgggcgctttggcacccagtcccaggccacggtgaacttgggggtcgtgagcaggttccgggtggtcggcgccgtggcccgggccttggtggtgaggtcgcgcgcgtagaagccgtcgacctgcttgaagcggtcggcggcgtagctggtgtgttcggtgtgcgacccctcccggtagccgtaaaacggggacatgtacacaaagtcgccagtcgccagcacaaactcgtcgtacgggtacaccgagcgcgcgtccacctcctcgacgatgcagtttaccgtcgtcccgtaccggtggaacgcctccacccgcgaggggttgtacttgaggtcggtggtgtgccagccccggctcgtgcgggtcgcggcgttggccggtttcagctccatgtcggtctcgtggtcgtcccggtgaaacgcggtggtctccaggttgttgcgcacgtacttggccgtggaccgacagacccccttggcgttgatcttgtcgatcacctcctcgaaggggacgggggcgcggtcctcaaagatccccataaactgggagtagcggtggccgaaccacacctgcgaaacggtgacgtctttgtagtacatggtggccttgaacttgtacggggcgatgttctccttgaagaccaccgcgatgccctccgtgtagttctgaccctcgggccgggtcgggcagcggcgcggctgctcgaactgcaccaccgtggcgcccgtggggggtgggcacacgtaaaagtttgcatcggtgttctccgccttgatgtcccgcaggtgctcgcgcagggtggcgtggcccgcggcgacggtcgcgttgtcgccggcggggcgtggtggcgttgggtttttcggttttttgttcttcttcggtttcgggtcccccgttggggcggcgccaagggcgggcggcgccggagtggcagggcccccgttcgccgcctgggtcgcggccgcgaccccaggcgtgccgggggaactcggagccgccgacgccaccaggacccccagcgtcaaccccaagagcgcccatacgacgaaccaccggcgcccccacgagggggcgccctggtgcatggcgggactacgggggcccgtcgtgccccccgtcaggtagcctgggggcgaggtgctggaggaccgagtagaggatcgagaaaacgtcgcggtcgtagaccacgaccgaccgggggccgatacagccgtcgggggcgctctcgacgatggccaccagcggacagtcggagtcgtacgtgagatatacgccgggcgggtaacggtaacgaccttcggaggtcgggcggctgcagtccgggcggcgcaactcgagctccccgcaccggtagaccgaggcaaagagtgtggtggcgataatcagctcgcgaatatatcgccaggcggcgcgctgagtgggcgttattccggaaatgccgtcaaaacagtaaaacctctgaaattcgctgacggcccaatcagcacccgagccccccgcccccatgatgaaccgggcgagctcctccttcaggtgcggcaggagccccacgttctcgacgctgtaatacagcgcggtgttggggggctgggcgaagctgtgggtggagtgatcaaagaggggcccgttgacgagctcgaagaagcgatgggtgatgctggggagcagggccgggtccacctggtgtcgcaggagagacgctcgcatgaaccggtgcgcgtcgaacacgcccggcgccgagcggttgtcgatgaccgtgcccgcgcccgccgtcagggcgcagaagcgcgcgcgcgccgcaaagccgttggcgaccgcggcgaacgtcgcgggcagcacctcgccgtggacgctgacccgcagcatcttctcgagctccccgcgctgctcgcggacgcagcgccccaggctggccaacgaccgcttcgtcaggcggtccgcgtacagccgccgtcgctcccgtacgtccgcggccgcttgcgtggcgatgtccccccacgtctcgggcccctgccccccgggcccgcggcgacggtcttcgtcctcgcccccgcccccgggagctcccaacccccgtgccccttcctctacggcgacacggtccccgtcgtcgtcggggcccgcgccgcccttgggcgcgtccgccgcgccccccgcccccatgcgcgccagcacgcgacgcagcgcctcctcgtcgcactgttcggggctgacgaggcgccgcaagagcggcgtcgtcaggtggtggtcgtagcacgcgcggatgagcgcctcgatctgatcgtcgggtgacgtggcctgaccgccgattattagggcgtccaccatatccagcgccgccaggtggctcccgaacgcgcgatcgaaatgctccgcccgccgcccgaacagcgccagttccacggccaccgcggcggtctcctgctgcaactcgcgccgcgccagcgcggtcaggttgctggcaaacgcgtccatggtggtctggccggcgcggtcgccggacgcgagccagaatcgcaattcgctgatggcgtacaggccgggcgtggtggcctgaaacacgtcgtgcgcctccagcagggcgtcggcctccttgcggaccgagtcgttctcgggcgacgggtggggctgcccgtcgccccccgcggtccgggccagcgcatggtccaacacggagagcgcccgcgcgcggtcggcgtccgacagcccggcggcgtggggcaggtaccgccgcagctcgttggcgtccagccgcacctgcgcctgctgggtgacgtggttacagatacggtccgccaggcggcgggcgatcgtcgccccctggttcgccgtcacacacagttcctcgaaacagaccgcgcaggggtgggacgggtcgctaagctccggggggacgataaggcccgaccccaccgcccccaccataaactcccgaacgcgctccagcgcggcggtggcgccgcgcgagggggtgatgaggtggcagtagtttagctgctttagaaagttctcgacgtcgtgcaggaaacacagctccatatggacggtcccgccatacgtatccagcctgacccgttggtgatacggacagggtcgggccaggcccatggtctcggtgaaaaacgccgcgacgtctcccgcggtcgcgaacgtctccaggctgcccaggagccgctcgccctcgcgccacgcgtactctagcagcaactccagggtgaccgacagcggggtgagaaaggccccggcctgggcctccaggcccggcctcagacgacgccgcagcgcccgcacctgaagcgcgttcagcttcagttgggggagcttcccccgtccgatgtgggggtcgcaccgccggagcagctctatctgaaacacataggtctgcacctgcccgagcagggctaacaacttttgacgggccacggtgggctcggacaccggggcggccatctcgcggcgccgatctgtaccgcggccggagtatgcggtggaccgaggcggtccgtacgctacccggtgtctggctgagccccggggtccccctcttcggggcggcctcccgcgggcccgccgaccggcaagccgggagtcggcggcgcgtgcgtttctgttctattcccagacaccgcggagaggaatcacggcccgcccagagatatagacacggaacacaaacaagcacggatgtcgtagcaataatttattttacacacattccccgccccgccctaggttcccccaccccccaacccctcacagcatatccaacgtcaggtctccctttttgtcggggggcccctccccaaacgggtcatccccgtggaacgcccgtttgcggccggcaaatgccggtcccggggcccccgggccgccgaacggcgtcgcgttgtcgtcctcgcagccaaaatccccaaagttaaacacctccccggcgttgccgagttggctgactagggcctcggcctcgtgcgccacctccagggccgcgtccgtcgaccactcgccgttgccgcgctccagggcacgcgcggtcagctccatcatctcctcgcttaggtactcgtcctccaggagcgccagccagtcctcgatctgcagctgctgggtgcggggccccaggcttttcacggtcgccacgaacacgctactggcgacggccgccccgccctcggagataatgccccggagctgctcgcacagcgagctttcgtgcgctccgccgccgaggttcgaggccgcgcacacaaacccggcccggggacaggccaggacgaacttgcgggtgcggtcaaaaataaggagcgggcacgcgtttttgccgcccatcaggctggcccagttcccggcctgaaacacacggtcgttgccggccatgccgtagtatttgctgatgctcaaccccaacacgaccatggggcgcgccgccatgacgggccgcagcaggttgcagctggcgaacatggacgtccacgcgcccggatgcgcgtccacggcgtccatcagcgcgcgggccccggcctccaggcccgccccgccctgcgcggaccacgcggccgccgcctgcacgctggggggacggcgggaccccgcgatgatggccgtgagggtgttgatgaagtatgtcgagtgatcgcagtaccgcagaatctggtttgccatgtagtacatcgccagctcgctcacgttgttgggggccaggttaataaagtttatcgcgccgtagtccagggaaaactttttaatgaacgcgatggtctcgatgtcctcgcgcgacaggagccgggcgggaagctggttgcgttggagggccgtccagaaccactgcgggttcggctggttggaccccgggggcttgccgttggggaagatggccgcgtggaactgcttcagcagaaagcccagcggtccgaggaggatgtccacgcgcttgtcgggcttctggtaggcgctctggaggctggcgacccgcgccttggcggcctcggacgcgttggcgctcgcgcccgcgaacaacacgcggctcttgacgcgcagctccttgggaaaccccagggtcacgcgggcaacgtcgccctcgaagctgctctcggcgggggccgtctggccggccgttaggctgggggcgcagatagccgccccctccgagagcgcgaccgtcagcgttttggccgacagaaacccgttgttaaacatgtccatcacgcgccgccgcagcaccggttggaattgattgcgaaagttgcgcccctcgaccgactgcccggcgaacaccccgtggcactggctcagggccaggtcctgatacacggcgaggttggatcgccgcccgagaagctgaagcagggggcatggcccgcacgcgtacgggtccagcgtcagggacatggcgtggttggcctcgcccagaccgtcgcgaaacttgaagttcctcccctccaccaggttgcgcatcagctgctccacctcgcggtccacgacctgcctgacgttgttcaccaccgtatgcagggcctcgcggttggtgatgatggtctccagccgccccatggccgtggggaccgcctggtccacgtactgcagggtctcgagttcggccatgacgcgctcggtcgccgcgcggtacgtctcctgcatgatggtccgggcggtctcggatccgtccgcgcgcttcagggccgagaaggcggcgtagtttcccagcacgtcgcagtcgctgtacatgctgttcatggtcccgaagacgccgatggctccgcgggcggcgctggcgaacttgggatggcgcgcccggaggcgcatgagcgtcgtgtgtacgcaggcgtggcgcgtgtcgaaggtgcacaggttgcagggcacgtcggtctggttggagtccgcgacgtatcgaaacacgtccatctcctggcgcccgacgatcacgccgccgtcgcagcgctccaggtaaaacagcatcttggccagcagcgccggggaaaacccacacagcatggccaggtgctcgccggcaaattcctgggttccgccgacgaggggcgcggtgggccgaccctcgaacccgggcaccacgtgtccctcgcggtccacctgtgggttggccgccacgtgggtcccgggcacgaggaagaagcggtaaaaggagggtttgctgtggtcctttgggtccgccggaccggcgtcgtccacctcggtgagatggagggccgagttggtgctaaataccatggcccccacgagtcccgcggcgcgcgccaggtacgccccgacggcgttggcgcgggccgcggccgtgtcctggccctcgcacagcggccacgcggagatgtcggtgggcggctcgtcgaagacggccatcgacacgatagactcgagggccagggcggcgtctccggccatgacggaggccaggcgctgttcgaacccgcccgccgggcccttgccgccgccgtcgcgcccaccccgcggggtcttaccctggctggcttcgaaggccgtgaacgtaatgtcggcggggagggcggcgccctcgtggttttcgtcaaacgccaggtgggcggccgcgcgggccacggcgtccacgtttcggcatcgcagtgccacggcggcgggtcccacgaccgcctcgaacaggaggcggttgagggggcggttaaaaaacggaagcgggtaggtaaaattctccccgatcgatcggtggttggcgttgaacggctcggcgatgacccggctaaaatccggcatgaacagctgcaacggatacacgggtatgcggtgcacctccgccccgcctatggttaccttgtccgagcctcccaggtgcagaaaggtgttgttgatgcacacggcctccttgaagccctcggtaacgaccagatacaggagggcgcggtccgggtccaggccgaggcgctcacacagcgcctcccccgtcgtctcgtgtttgaggtcgccgggccggggggtgtagtccgaaaagccaaaatggcggcgtgcccgctcgcagagtcgcgtcaggtttggggcctgggtgctggggtccaggtgccggccgccgtgaaagacgtacacggacgagctgtagtgcgatggcgtcagtttcagggacaccgcggtacccccgagccccgtcgtgcgagaacccacgaccacggctacgttggcctcaaagccgctctccacggtcaggcccacgaccaggggcgccacggcgacgtcggcatcgccgctgcgcgccgacagtaacgccagaagctcgatgccttcggacggacacgcgcgagcgtacacgtatcccaggggcccgggggggaccttgatggtggttgccgtcttgggctttgtctccatgtcctcctggcaatcggtccgcaaacggaggtaatcccggcacgacgacggacgcccgacgaggtatgtctcccgagcgtcaaaatccgggggggggggcggcgacggtcaaggggagggtgggagaccggggttggggaatgaatccctacccttcacagacaacccccgggtaaccacggggtgccgatgaaccccggcggctggcaacgcggggtccctgcgagaggcacagatgcttacggtcaggtgctccgggccgggtgcgtctgatatgcggttggtatatgtacactttacctgggggcgtgccggaccgccccagcccctcccacaccccgcgcgtcatcagccggtgggcgtggccgctattataaaaaaagtgagaacgcgaagcgttcgcactttgtcctaataatatatatattattaggacaaagtgcgaacgcttcgcgttctcactttttttataatagcggccacgcccaccggctacgtcacgctcctgtcggccgccggcggtccataagcccggccggccgggccgacgcgaataaaccgggccgccggccggggcgccgcgcagcagctcgccgcccggatccgccagacaaacaaggcccttgcacatgccggcccgggcgagcctgggggtccggtaattttgccatcccacccaagcggcttttggggtttttcctcttcccccctccccacatcccccctctttaggggttcgggtgggaacaaccgcgatgttttccggtggcggcggcccgctgtcccccggaggaaagtcggcggccagggcggcgtccgggttttttgcgcccgccggccctcgcggagccggccggggacccccgccttgtttgaggcaaaacttttacaacccctacctcgccccagtcgggacgcaacagaagccgaccgggccaacccagcgccatacgtactatagcgaatgcgatgaatttcgattcatcgccccgcgggtgctggacgaggatgcccccccggagaagcgcgccggggtgcacgacggtcacctcaagcgcgcccccaaggtgtactgcgggggggacgagcgcgacgtcctccgcgtcgggtcgggcggcttctggccgcggcgctcgcgcctgtggggcggcgtggaccacgccccggcggggttcaaccccaccgtcaccgtctttcacgtgtacgacatcctggagaacgtggagcacgcgtacggcatgcgcgcggcccagttccacgcgcggtttatggacgccatcacaccgacggggaccgtcatcacgctcctgggcctgactccggaaggccaccgggtggccgttcacgtttacggcacgcggcagtacttttacatgaacaaggaggaggttgacaggcacctacaatgccgcgccccacgagatctctgcgagcgcatggccgcggccctgcgcgagtccccgggcgcgtcgttccgcggcatctccgcggaccacttcgaggcggaggtggtggagcgcaccgacgtgtactactacgagacgcgccccgctctgttttaccgcgtctacgtccgaagcgggcgcgtgctgtcgtacctgtgcgacaacttctgcccggccatcaagaagtacgagggtggggtcgacgccaccacccggttcatcctggacaaccccgggttcgtcaccttcggctggtaccgtctcaaaccgggccggaacaacacgctagcccagccgcgggccccgatggccttcgggacatccagcgacgtcgagtttaactgtacggcggacaacctggccatcgaggggggcatgagcgacctaccggcatacaagctcatgtgcttcgatatcgaatgcaaggcggggggggaggacgagctggcctttccggtggccgggcacccggaggacctggttattcagatatcctgtctgctctacgacctgtccaccaccgccctggagcacgtcctcctgttttcgctcggttcctgcgacctccccgaatcccacctgaacgagctggcggccaggggcctgcccacgcccgtggttctggaattcgacagcgaattcgagatgctgttggccttcatgacccttgtgaaacagtacggccccgagttcgtgaccgggtacaacatcatcaacttcgactggcccttcttgctggccaagctgacggacatttacaaggtccccctggacgggtacggccgcatgaacggccggggcgtgtttcgcgtgtgggacataggccagagccacttccagaagcgcagcaagataaaggtgaacggcatggtgaacatcgacatgtacgggatcataaccgacaagatcaagctctcgagctacaagctcaacgccgtggccgaagccgtcctgaaggacaagaagaaggacctgagctatcgcgacatccccgcctactacgccaccgggcccgcgcaacgcggggtgatcggcgagtactgcatacaggattccctgctggtgggccagctgttttttaagtttttgccccatctggagctctcggccgtcgcgcgcttggcgggtattaacatcacccgcaccatctacgacggccagcagatccgcgtctttacgtgcctgctgcgcctggccgaccagaagggctttattctgccggacacccaggggcgatttaggggcgccgggggggaggcgcccaagcgtccggccgcagcccgggaggacgaggagcggccagaggaggagggggaggacgaggacgaacgcgaggagggcgggggcgagcgggagccggagggcgcgcgggagaccgccggccggcacgtggggtaccagggggccagggtccttgaccccacttccgggtttcacgtgaaccccgtggtggtgttcgactttgccagcctgtaccccagcatcatccaggcccacaacctgtgcttcagcacgctctccctgagggccgacgcagtggcgcacctggaggcgggcaaggactacctggagatcgaggtgggggggcgacggctgttcttcgtcaaggctcacgtgcgagagagcctcctcagcatcctcctgcgggactggctcgccatgcgaaagcagatccgctcgcggattccccagagcagccccgaggaggccgtgctcctggacaagcagcaggccgccatcaaggtcgtgtgtaactcggtgtacgggttcacgggagtgcagcacggactcctgccgtgcctgcacgttgccgcgacggtgacgaccatcggccgcgagatgctgctcgcgacccgcgagtacgtccacgcgcgctgggcggccttcgaacagctcctggccgatttcccggaggcggccgacatgcgcgcccccgggccctattccatgcgcatcatctacggggacacggactccatatttgtgctgtgccgcggcctcacggccgccgggctgacggccatgggcgacaagatggcgagccacatctcgcgcgcgctgtttctgccccccatcaaactcgagtgcgaaaagacgttcaccaagctgctgctgatcgccaagaaaaagtacatcggcgtcatctacgggggtaagatgctcatcaagggcgtggatctggtgcgcaaaaacaactgcgcgtttatcaaccgcacctccagggccctggtcgacctgctgttttacgacgataccgtatccggagcggccgccgcgttagccgagcgccccgcagaggagtggctggcgcgacccctgcccgagggactgcaggcgttcggggccgtcctcgtagacgcccatcggcgcatcaccgacccggagagggacatccaggactttgtcctcaccgccgaactgagcagacacccgcgcgcgtacaccaacaagcgcctggcccacctgacggtgtattacaagctcatggcccgccgcgcgcaggtcccgtccatcaaggaccggatcccgtacgtgatcgtggcccagacccgcgaggtagaggagacggtcgcgcggctggccgccctccgcgagctagacgccgccgccccaggggacgagcccgccccccccgcggccctgccctccccggccaagcgcccccgggagacgccgtcgcatgccgaccccccgggaggcgcgtccaagccccgcaagctgctggtgtccgagctggccgaggatcccgcatacgccattgcccacggcgtcgccctgaacacggactattacttctcccacctgttgggggcggcgtgcgtgacattcaaggccctgtttgggaataacgccaagatcaccgagagtctgttaaaaaggtttattcccgaagtgtggcaccccccggacgacgtggccgcgcggctccgggccgcagggttcggggcggtgggtgccggcgctacggcggaggaaactcgtcgaatgttgcatagagcctttgatactctagcatgagccccccgtcgaagctgatgtccctcattttacaataaatgtctgcggccgacacggtcggaatctccgcgtccgtgggtttctctgcgttgcgccggaccacgagcacaaacgtgctctgccacacgtgggcgacgaaccggtaccccgggcacgcggtgagcatccggtctatgagccggtagtgcaggtgggcggacgtgccgggaaagatgacgtacagcatgtggcccccgtaagtggggtccgggtaaaacaacagccgcgggtcgcacgccccgcctccgcgcaggatcgtgtggacgaaaaaaagctcgggttggccaagaatcccggccaagaggtcctggaggggggcgttgtggcggtcggccaacacgaccaaggaggccaggaaggcgcgatgctcgaatatcgtgttgatctgctgcacgaaggccaggattagggcctcgcggctggtggcggcgaaccgcccgtctcccgcgttgcacgcgggacagcaacccccgatgcctaggtagtagcccatcccggagagggtcaggcagttgtcggccacggtctggtccagacagaagggcagcgacacgggagtggtcttcaccaggggcaccgagaacgagcgcacgatggcgatctcctcggagggcgtctgggcgagggcggcgaaaaggccccgatagcgctggcgctcgtgtaaacacagctcctgtttgcgggcgtgaggcggcaggctcttccgggaggcccgacgcaccacgcccagagtcccgccggccgcagaggagcacgaccgccggcgctccttgccgtgatagggcccgggccgggagccgcggcgatgggggtcggtatcatacataggtacacagggtgtgctccagggacaggagcgagatcgagtggcgtctaagcagcgcgcccgcctcacggacaaatgtggcgagcgcggtgggctttggtacaaatacctgatacgtcttgaaggtgtagatgagggcacgcaacgctatgcagacacgcccctcgaactcgttcccgcaggccagcttggccttgtggagcagcagctcgtcgggatgggtggcggggggatggccgaacagaacccaggggtcaacctccatctccgtgatggcgcacatggggtcacagaacatgtgcttaaagatggcctcgggccccgcggcccgcagcaggctcacaaaccggcccccgtccccgggctgcgtctcggggtccgcctcgagctggtcgacgacgggtacgatacagtcgaagaggctcgtgttgttttccgagtagcggaccacggaggcccggagtctgcgcagggccagccagtaagcccgcaccagtaacaggttacacagcaggcattctccgccggtgcgcccgcgcccccggccgtgtttcagcacggtggccatcagagggcccaggtcgaggtcgggctgggcatcgggttcggtaaactgcgcaaagcgcggagccacgtcgcgcgtgcgtgccccgcgatgcgcttcccaggactggcggaccgtggcgcgacgggcctccgcggcagcgcgcagctggggccccgactcccagacggcgggggtgccggcgaggagcagcaggaccagatccgcgtacgcccacgtatccggcgactcctccggctcgcggtccccggcgaccgtctcgaattccccgttgcgagcggcggcgcgcgtacagcagctgtccccgcccccgcgccgaccctccgtgcagtccaggagacgggcgcaatccttccagttcatcagcgcggtggtgagcgacggctgcgtgccggatcccgccgccgaccccgccccctcctcgcccccggaggccaaggttccgatgagggcccgggtggcagactgcgccaggaacgagtagttggagtactgcaccttggcggctcccggggagggcgagggcttgggttgcttctgggcatgccgcccgggcaccccgccgtcggtacggaagcagcagtggagaaaaaagtgccggtggatgtcgtttatggtgagggcaaagcgtgcgaaggagccgaccagggtcgccttcttggtgcgcagaaagtggcggtccatgacgtacacaaactcgaacgcggccacgaagatgctagcggcgcagtggggcgcccccaggcatttggcacagagaaacgcgtaatcggccacccactggggcgagaggcggtaggtttgcttgtacagctcgatggtgcggcagaccagacagggccggtccagcgcgaaggtgtcgatggccgccgcggaaaagggcccggtgtccaaaagcccctccccacagggatccgggggcgggttgcggggtcctccgcgcccgcccgaaccccctccgtcgcccgcccccccgcgggcccttgagggggcggtgaccacgtcggcggcgacgtcctcgtcgagcgtaccgacgggcggcacacctatcacgtgactggccgccaggagctcggcgcagagagcctcgttaagagccaggaggctgggatcgaaggccacatacgcgcgctcgaacgcccccgccttccagctgctgccgggggactcttcgcacaccgcgacgctcgccaggaccccggggggcgaagttgccatggctgggcgggaggggcgcacgcgccagcgaactttacgggacacaatccccgactgcgcgctgcggtcccagaccctggagagtctagacgcgcgctacgtctcgcgagacggcgcgcatgacgcggccgtctggttcgaggatatgacccccgccgagctggaggttgtcttcccgactacggacgccaagctgaactacctgtcgcggacgcagcggctggcctccctcctgacgtacgccgggcctataaaagcgcccgacgacgccgccgccccgcagaccccggacaccgcgtgtgtgcacggcgagctgctcgcccgcaagcgggaaagattcgcggcggtcattaaccggttcctggacctgcaccagattctgcggggctgacgcgcgcgctgttgggcgggacggttcgcgaaccctttggtgggtttacgcgggcacgcacgctcccatcgcgggcgccatggcgggactgggcaagccctaccccggccacccaggtgacgccttcgagggtctcgttcagcgaattcggcttatcgtcccatctacgttgcggggcggggacggggaggcgggcccctactctccctccagcctcccctccaggtgcgcctttcagtttcatggccatgacgggtccgacgagtcgtttcccatcgagtatgtactgcggcttatgaacgactgggccgaggtcccgtgcaacccttacctgcgcatacagaacaccggcgtgtcggtgctgtttcaggggttttttcatcgcccacacaacgcccccgggggcgcgattacgccagagcggaccaatgtgatcctgggctccaccgagacgacggggctgtccctcggcgacctggacaccatcaaggggcggctcggcctggatgcccggccgatgatggccagcatgtggatcagctgctttgtgcgcatgccccgcgtgcagctcgcgtttcggttcatgggccccgaagatgccggacggacgagacggatcctgtgccgcgccgccgagcaggctattacccgtcgccgccgaacccggcggtcccgggaggcgtacggggccgaggccgggctgggggtggctggaacgggtttccgggccaggggggacggttttggcccgctccccttgttaacccaagggccctcccgcccgtggcaccaggccctgcggggtcttaagcacctacggattggcccccccgcgctcgttttggcggcgggactcgtcctgggggccgctatttggtgggtggttggtgctggcgcgcgcctataaaaaaggacgcaccgccgccctaatcgccagtgcgttccggacgccttcgccccacacagccctcccgtccgacacccccatatcgcttcccgacctccggtcccgatggccgtcccgcaatttcaccgccccagcaccgttaccaccgatagcgtccgggcgcttggcatgcgcgggctcgtcttggccaccaataactctcagtttatcatggataacaaccacccgcacccccagggcacccaaggggccgtgcgggagtttctccgcggtcaggcggcggcgctgacggaccttggtctggcccacgcaaacaacacgtttaccccgcagcctatgttcgcgggcgacgccccggccgcctggttgcggcccgcgtttggcctgcggcgcacctattcaccgtttgtcgttcgagaaccttcgacgcccgggaccccgtgaggcccggggagttccttctggggtgttttaatcaataaaagaccacaccaacgcacgagccttgcgtttaatgtcgtgtttattcaagggagtgggatagggttcgacggttcgaaacttaacacacaaaataatcgagcgcgtctagcccagtaacatgcgcacgtgatgtaggctggtcagcacggcgtcgctgtgatgaagcagcgcccggcgggtccgctgtaactgctgttgtaggcggtaacaggcgcggatcagcaccgccagggcgctacgaccggtgcgttgcacgtagcgtcgcgacagaactgcgtttgccgatacgggcggggggccgaattgtaagcgcgtcacctcttgggagtcatcggcggataacgcactgaatggttcgttggttatgggggagtgtggttcccgagggagtgggtcgagcgcctcggcctcggaatccgagaggaacaacgaggtggtgtcggagtcttcgtcgtcagagacatacagggtctgaagcagcgacacgggcgggggggtagcgtcaatgtgtagcgcgagggaggatgcccacgaagacaccccagacaaggagctgcccgtgcgtggatttgtggacgacgcggaagccgggacggatgggcggttttgcggtgcccggaaccgaaccgccggatactccccgggtgctacatgcccgttttggggctggggttggggctggggctggggttggggttggggctggggttggggctggggttggggctggggttggggttggggttggggctggggttggggttggggctggggctggggctggggctggggctggggctggggctggggctggggctggggctggggctggggctggggctggggctggggttggggctggggttggggctggggcgcggacaggcggttgacggtcaaatgcccccgggggcgcgcagatgtggtgggcgtggccaccggctgccgtgtagtggggcggcgggaaaccgggcctccgggcgtaacaccgccctccagcgtcaagtatgtggggggcgggcctgacgtcgggggcggggtgacgggttggaccgcgggaggcgggggagagggacctgcgggagaggatgaggtcggctcggccgggttgcggcctaaaacaggggccgtggggtcggcggggtcccagggtgaagggagggattcccgcgattcggacagcgacgcgacagcggggcgcgtaaggcgccgctgcggcccgcctacgggaaccctggggggggttggcgcgggacccgaggttagcggggggcggcggttttcgcccccgggcaaaaccgtgccggttgcgaccgggggcggaacgggatcgatagggagagcgggagaagcctggccggcgaactggggaccgagcgggaggggcacaccagacaccaaagcgtggagcgctggctctgggggtttgggaggggccggggggcgcgcgaaatcggtaaccggggcgaccgtgtcggggagggcaggcggccgccaaccctgggtggtcgcggaagcctgggtggcgcgcgccagggagcgtgcccggcggtgtcggcgcgcgcgcgacccggacgaagaagcggcagaagcgcgggaggaggcgggggggcggggggcggtggcatcggggggcgccggggaactttggggggacggcaagcgccggaagtcgtcgcgggggcccacgggcgccggccgcgtgctttcggccgggacgcccggtcgtgcttcgcgagccgtgactgccggcccagggggccgcggtgcacactgggacgtggggacggactgatcggcggtgggcgaaagggggtccggggcaaggaggggcgcggggccgccggagtcgtcagacgcgagctcctccaggccgtgaatccatgcccacatgcgaggggggacgggctcgccgggggtggcgtcggtgaatagcgtgggggccaggcttccgggccccaacgagccctccgtcccaacaaggtccgccgggccgggggtcgggttcgggaccgaggggctctggtcgtcgggggcgcgctggtacaccggatgccccgggaatagctcccccgacaggagggaggcgtcgaacggccgcccgaggatagctcgcgcgaggaaggggtcctcgtcggtggcgctggcggcgaggacgtcctcgccgcccgccacaaacgggagctcctcggtggcctcgctgccaacaaaccgcacgtcgggggggccgggggggtccgggttttcccacaacaccgcgaccggggtcatggagatgtccacgagcaccagacacggcgggccccgggcgaggggccgctcggcgatgagcgcggacaggcgcgggagctgtgccgccagacacgcgttttcaatcgggttcaggtcggcgtgcaggaggcggacggcccacgtctcgatgtcggacgacacggcatcgcgcaaggcggcgtccggcccgcgagcgcgtgagtcaaacagcgtgagacacagctccagctccgactcgcgggaaaaggccgtggtgttgcggagcgccacgacgacgggcgcgcccaggagcactgccgccagcaccaggtccatggccgtaacgcgcgccgcgggggtgcggtgggtggcggcggccggcacggcgacgtgctggcccgtgggccggtagagggcgttggggggagcggggggtgacgcctcgcgcccccccgaggggctcagcgtctgcccagattccagacgcgcggtcagaagggcgtcgaaactgtcatactctgtgtagtcgtccggaaacatgcaggtccaaagagcggccagagcggtgcttgggagacacatgcgcccgaggacgctcaccgccgccagcgcctgggcgggactcagctttcccagcgcggcgccgcgctcggttcccagctcggggaccgagcgccagggcgccagggggtcggtttcggacaacttgccgcggcgccagtctgccagccgcgtgccgaacatgaggccccgggtcggagggcctccggtcgaaaacactggcagcacgcggatgcgggcgtctggatgcggggtcaggcgctgcacgaatagcatggaatctgctgcgttctgaaacgcacgggggagggtgagatgcatgtactcgtgttggcggaccagatccaggcgccaaaaggtgtaaatgtgttccggggagctggccaccagcgccaccagcacgtcgttctcgttaaaggaaacgcggtgcctagtggagctgtggggcccgagcggcggtcccggggccgccgcgtcacccccccattccagctgggcccagcgacacccaaactcgcgcgtgagagtggtcgcgacgagggcgacgtagagctcggccgccgcatccatcgaggccccccatctcgcctggcggtggcgcacaaagcgtccgaagagctgaaagttggcggcctgggcgtcgctgagggccagctgaagccggttgatgacggtgatgacgtacatggccgtgacggtcgaggccgactccagggtgtccgtcggaagcggggggcgaatgcatgccgcctcgggacacatcagcagcgcgccgagcttgtcggtcacggccgggaagcagagcgcgtactgcagtggcgttccatccgggaccaaaaagctgggggcgaacggccgatccagcgtactggtggcctcgcgcagcaccaggggccccgggcctccgctcactcgcaggtacgcctcgccccggcggcgcagcatctgcgggtcggcctcttggccgggtggggcggacgcccgggcgcgggcgtctagggcgcgaagatccacgagcaggggcgcgggcgcggcggccgcgcccgcgcccgtctggcctgtggccttggcgtacgcgctatataagcccatgcggcgttggatgagctcccgcgcgccccggaactcctccaccgcccatggggccaggtccccggccaccgcgtcgaattccgccaacaggccccccagggtgtcaaagttcatctcccaggccacccttggcaccacctcgtcccgcagccgggcgctcaggtcggcgtgttgggccacgcgccccccgagctcctccacggccccggcccgctcggcgctcttggcgcccaggacgccctggtacttggcgggaaggcgctcgtagtcccgctgggctcgcagccccgacacagtgttggtggtgtcctgcagggcgcgaagctgctcgcatgccgcgcgaaatccctcgggcgatttccaggcccccccgcgaacgcggccgaagcgaccccatacctcgtcccactccgcctcggcctcctcgagagacctccgcagggcctcgacgcggcgacgggtgtcgaagagcgcctgcaggcgcgcgccctgtcgcgtcaggaggcccgggccgtcgccgctggccgcgtttagcgggtgcgtctcaaaggtacgctgggcatgttccaaccaggcgaccgcctgcacgtcgagctcgcgcgccttctccgtctggtccaacagaatttcgacctgatccgcgatctcctccgccgagcgcgcctggtccagcgtcttggccacggtcgccgggacggcgaccaccttcagcagggtcttcagattggccagaccctcggcctcgagctgggcccggcgctcgcgcgcggccagcacctcccgcagccccgccgtgacccgctcggtggcttcggcgcgctgctgtttggcgcgcaccacggcgtccttggtatcggccaggtcctgtcgggtcacgaatgcgacgtagtcggcgtacgccgtgtccttcacggggctctggtccacgcgctccagcgccgccacgcacgccaccagcgcgtcctcgctcgggcagggcagggtgacccctgcccggacaagctcggcggccgccgccgggtcgttgcgcaccgcggatatctcctccgcggcggcggccaggtccagcgccacgcttccgatcgcgcgccgcgcgtcggcccggagggcgtccaggcgatcgcggatatccacgtactcggcgtagcccttttgaaaaaacggcacgtactggcgcagggccggcacgccccccaagtcttccgacaggtgtaggacggcctcgtggtagtcgataaacccgtcgttcgcctgggcccgctccagcagcccccccgccagccgcagaagccgcgccaggggctcggtgtccacccgaaacatgtcggcgtacgtgtcggccgcggccccgaaggccgcgctccagtcgatgcggtgaatggctgcgagcggggggagcatggggtggcgctggttctcgggggtgtatgggttaaacgcaagggccgtctccagggcaagggtcaccgccttggcgttggttcccagcgcctgttcggcccgctttcggaagtcccgggggttgtagccgtgcgtgcccgccagcgcctgcaggcgacggagctcgaccacgtcaaactcggcaccgctttccacgcggtccagcacggcctccacgtcggcggcccagcgctcgtggctactgcgggcgcgctgggccgccatcttctctctcaggtcggcgatggcggcctcaagttcgtcggcgcggcgtcgcgtggcgccgatgacctttcccagctcctgcagggcgcgcccgctgggggagtggtccccggccgtcccttcggcgtgcaacaggcccccgaacctgccctcgtggcccgcgaggctttcccgcgcgccggtggtcgcgcgcgtcgcggcctggatcagggaggcatgctctccctccggttggttggcggcccggcgcacctggacgacaaggtcggctgccgccgaccctaaggtcgtgagctgggcgatggccccccgcgcgtccagggccaaccgagtcgccttgacgtatcccgcggcgctgtcggccatggccgctaggaaggccaggggggaggccgggtcgctggcggccgcgcccagggccgtcaccgcgtcgaccaggacgcggtgcgcccgcacggccgcatccaccgtcgacgcggggtctgccgtcgcgacggcggcgctgccggcgttgatggcgttcgagacggcgtgggctatgatcggggcgtgatcggcgaagaactgcaagagaaacggagtctctggggcgtcggcgaacaggttcttcagcaccaccacgaagctgggatgcaagccagacagagccgtcgccgtgtccggagtcgggtgctccagggcatctcggtactgccccagcagcccccacatgtccgcccgcagcgccgccgtaacctcagggggcgccccccgaacggcctcggggaggtccgaccagcccgccggcagggaggcccgcagggtcgccaggacggccggacaggcctttagccccacaaagtcagggagggggcgcaggaccccctggagtttgtgcaagaacttctcccgggcgtcgcgggccaccttcgcccgctcccgcgctccctcgagcattgcctccagggagcgcgcgcgctcccgcaaacgggcacgcgcatcgggggcgagctctgccgtcagcttggcggcatccatggcccgcgcctgccgcagcgcttcctcggccatgcgcgtggcctctggcgacagcccgccgtcgtcggggtagggcgacgcgccgggcgcaggaacaaaggccgcgtcgctgtccagctgctggcccagggccgcatctagggcgtcgaagcgccgcagctcggccagacccgagctgcggcgcgcctgctggtcgttaatgtcgcggatgctgcgcgccagctcgtccagcggcttgcgttctatcagcccttggttggcggcgtccgtcaggacggagagccaggccgccaggtcctcgggggcgtccagcgtctggccccgctggatcagatcccgcaacaggatggccgtggggctggtcgcgatcgggggcggggcgggaatggcggcgcgctgcgcgatgtcccgcgtgtgctggtcgaagacaggcagggactcgagcagctggaccacgggcacgacggcggccgaagccacgtgaaaccggcggtcgttgttgtcgctggcctgtagagccttggcgctgtatacggccccccggtaaaagtactccttaaccgcgccctcgatcgcccgacgggcctgggtccgcacctcctccagccgaacctgaacggcctcggggcccagggggggtgggcgcggagccccctgcggggccgccccggccggggcgggcattacgccgaggggcccggcgtgctgtgagaccgcgtcgaccccgcgagcgagggcgtcgagggcctcgcgcatctggcgatcctccgcctccaccctaatctcttcgccacgggcaaatttggccagagcctggactctatacagaagcggttctgggtgcgtcggggtggcgggggcaaaaagggtgtccgggtgggcctgcgagcgctccagaagccactcgccgaggcgtgtatacagattggccggcggggccgcgcgaagctgcagctccaggtccgcgagttccccgtaaaaggcgtccgtctcccgaatgacatccctagccacaaggatcagcttcgccagcgccaggcgaccgatcagagagttttcgtccagcacgtgctggacgaggggcagatgggcggccacgtcggccaggctcaggcgcgtggaggccagaaagtcccccacggccgttttccggggcagcatgctcagggtaaactccagcagggcggcggccgggccggccaccccggcctgggtgtgcgtccgggccccgttctcgatgagaaaggcgaggacgcgttcaaagaaaaaaataacacagagctccagcagccccggagaagccggatacggcgaccgtaaggcgctgatggtgagccgcgaacacgcggcgacctcgcgggccagggtggcggagcacgcggtgaacttaaccgccgtggcggccacgtttgggtgggcctcgaacagctgggcgaggtctgcgcccgggggctcgggtgagcggcgagtcttcagcgcctcgagggcctgtgaggacgccggaaccatgggcccgtcgtcctcgcccgcctcggcgaccggcggcccggccgggtcggggggtgccgaggcgaggacaggctccggaacggaggcggggaccgcggccccgacgggggttttgcctttgggggtggatttcttcttggttttggcagggggggccgagcgtttcgttttctcccccgaagtcaggtcttcgacgctggaaggcggagtccaggtgggtcggcggcgcttgggaaggccggccgagtagcgtgcccggtgccgaccaaccgggacgacgcccatctccaggacccgcatgtcgtcgtcatcttcttcggccgcctctgcggcgggggtcttgggggcggagggaggcggtggtgggatcgcggagggtgggtcggcggaggggggatccgtgggtggggtaccctttagggccaccgcccatacatcgtcgggcgcccgattcgggcgcttggcctctggttttgccgacggaccggccgtcccccgggatgtctcggaggccctgtcgtcgcgacgggcccgggtcggtggcggcgactgggcggctgtgggcgggtgtggccccggcccccctcccccctcccgggggcccacgccgacgcagggctcccccaggcccgcgatctcgccccgcagggggtgcgtgatggccacgcgccgttcgctgaacgcttcgtcctgcatgtaagtctcgctggccccgtaaagatgcagagccgcggccgtcaagtccgcaggagccgcgggttccgggcccgacggcacgaaaaacaccatggctcccgcccaccgtacgtccgggcgatcgcgggtgtaatacgtcaggtatggatacatgtcccccgcccgcactttggcgatgaacgcgggggtgccctccggaaggccatgcgggtcaaaaaggtatgcggtgtcgccgtccctgaacagccccatccctagggggccaatggttaggagcgtgtacgacagggggcgcagggcccacgggccggcgaagaacgtgtgtgcggggcattgtgtctccagcaggcctgccgcgggctccccgaagaagcccacctcgccgtatacgcgcgagaagacacagcgcagtccgccgcgcgcccctgggtactcgaggaagttggggagctcgacgatcgaacacatgcgcggcggcccagggcccgcagtcgcgcgcgtccactcgcccccctcgaccaaacatccctcgatggcctccgcggacagaacgtcgcgagggcccacatcaaatatgaggctgagaaaggacagcgacgagcgcatgcacgataccgacccccccggctccaggtcgggcgcgaactggttccgagcaccggtgaccacgatgtcgcgatcccccccgcgttccatcgtggagtgcggtggggtgcccgcgatcatatgtgccctgcgggccagagacccggcctgtttatggaccggacccccggggttagtgttgtttccgccacccacgcccccgtaccatggccccggttcccctgattaggctacgagtcgcggtgatcgcttcccaaaaaccgagctgcgtttgtctgtcttggtcttccccccccccagcccgcacaccataacaccgagaacaacacacgggggtgggcggaacataataaagctttattggtaactagttaacggcaagtccgtgggtggcgcgacggtgtcctccgggatcatctcgtcgtcctcgacgggggtgttggaatgaggcgcctcctcgcggtccacctggcgtgggccgtgcccataggcctccggcttctgtgcgtccatgggcgtaggcgcggggagactgtttccggcgtcgcggacctccaggtccctgggagcctccggtccggctaacggacgaaacgcggaagcgcgaaacacgccgtcggtgacccgcaggagctcgttcatcagtaaccaatccatactcagcgtaacggccagcccctggcgagacagatccacggagtccggaaccgcggtcgtctggcccagggggccgaggctgtagtccccccaggcccctaggtcgcgacggctcgtaagcacgacgcggtcggccgcggggctttgcgggggggcgtcctcgggcgcatgcgccattacctctcggatggccgcggcgcgctggtcggccgagctgaccaagggcgccacgaccacggcgcgctccgtctgcaggcccttccacgtgtcgtggagttcctggacaaactcggccacgggctcgggtcccgcggccgcgcgcgcggcttgatagcaggccgacagacgccgccagcgcgctagaaactgacccatgaaacaaaacccggggacctggtctcccgacagcagcttcgacgcccgggcgtgaatgccggacacgacggacagaaacccgtgaatttcgcgccggaccacggccagcacgttgtcctcgtgcgacacctgggccgccagctcgtcgcacacccccaggtgcgccgtggtttcggtgatgacggaacgcaggctcgcgagggacgcgaccagcgcgcgcttggcgtcgtgatacatgctgcagtactgactcaccgcgtcccccatggcctcggggggccagggccccaggcggtcgggcgtgtccccgaccaccgcatacaggcggcgcccgtcgctctcgaaccgacactcgaaaaaggcggagagcgtgcgcatgtgcagccgcagcagcacgatggcgtcctccagttggcgaatcagggggtcggcgcgctcggcgaggtcctgcagcaccccccgggcagccagggcgtacatgctaatcaacaggaggctggtgcccacctcggggggcggggggggctgcagttggaccaggggccgcagctgctcgacggcacccctggagatcacgtacagctcccggagcagctgctctatgttgtcggccatctgcatagtggggccgaggccgccccgggcggccggttcgaggagagtgatcagcgcgcccagtttggtgcgatggccctcgaccgtggggagatagcccagcccaaagtcccgggcccaggccaacacacgcagggcgaactcgaccgggcggggaaggtaggccgcgctacacgtggccctcagcgcgtccccaaccaccagggccagaacgtaggggacgaagcccgggtcggcgaggacgttggggtgaatgccctcgagggcggggaagcggatctgggtcgccgcggccaggtggacagagggggcatggctgggctgcccgacggggagaagcgcggacagcggcgtggccggggtggtgggggtgatgtcccagtgggtctgaccatacacgtcgatccagatgagcgccgtctcgcggagaaggctgggttgaccggaactaaagcggcgctcggccgtctcaaactcccccacgagcgcccgccgcaggctcgccagatgttccgtcggcacggccggccccatgatacgcgccagcgtctggctcagaacgccccccgacaggccgaccgcctcacagagccgcccgtgcgtgtgctcgctggcgccctggacccgcctgaaagtttttacgtagttggcatagtacccgtattcccgcgccagaccaaacacgttcgaccccgcgagggcaatgcacccaaagagctgctggacttcgccgagtccgtggccggcgggcgtccgcgcggggacgcccgccgccagaaacccctccagggccgaaaggtagtgcgtgcagtgcgagggcgtgaacccagcgtcgatcagggtgttgatcaccacggagggcgaattggtattctggatcaacgtccacgtctgctgcagcagagccagcagccgctgctgggcgccggcggagggctgctccccgagctgcagcaggctggagacggcaggctggaagactgccagtgccgacgaactcaggaacggcacgtcgggatcaaacacggccacgtccgtccgcacgcgcgccattagcgtccccgggggcgcacaggccgagcgcgggctgacgcggctgagggccgtcgacacgcgcacctcctcgcggctgcgaaccatcttgttggcctccagtggcggaatcattatggccgggtcgatctcccgcacggtgtgctgaaactgcgccaacaggggcggcgggaccacagccccccgctcgggggtcgtcaggtactcgtccaccagggccaacgtaaagagggcccgtgtgaggggagtgagggtcgcgtcgtctatgcgctggaggtgcgccgagaacagcgtcacccgattactcaccagggccaagaaccggaggccctcttgcacgaacggggcggggaagagcaggctgtacgccggggtggtaaggttcgcgctgggctgccccaacgggaccggcgccagcttgagcgacgtctccccaagggcctcgatggaggtccgcgggctcatggccaagcagctcttggtgacggtttgccagcggtctatccactccacggcgcactggcggacgcggaccggccccagggccgccgcggtgcgcaggccggcggactccagcgcatgggacgtgtcggagccggtgaccgcgaggatggtgtccttgatgacctccatctcccggaaggcctggtcgggggcctcggggagagccaccaccaagcggtgtacgagcaacccggggaggttctcggccaagagcgccgtctccggaagcccgtgggcccggtggagcgcgcacaggtgttccagcagcggccgccagcatgcccgcgcgtctgccggggcgatggccgttcccgacaacagaaacgccgccatggcggcgcgcagcttggccgtggccagaaacgccgggtcgtccgccccgtttgccgtctcggccgtgggggttggcggttggcgaaggccggctaggctcgccaataggcgctgcataggtccgtccgagggcggaccggcgggtgaggtcgtgacgacgggggcctcggacgggagaccgcggtctgccatgacgcccggctcgcgtgggtgggggacagcgtagaccaacgacgagaccgggcgggaatgactgtcgtgcgctgtagggagcggcgaattatcgatcccccgcggccctccaggaaccccgcaggcgttgcgagtaccccgcgtcttcgcggggtgttatacggccacttaagtcccggcatcccgttcgcggacccaggcccgggggattgtccggatgtgcgggcagcccggacggcgtgggttgcggactttcggcggggcggcccaaatggccctttaaacgtgtgtatacggacgcgccgggccagtcggccaacacaacccaccggaggcggtagccgcgtttggctgtggggtgggtggttccgccttgcgtgagtgtcctttcgaccccccccctcccccgggtcttgctaggtcgcgatctgtggtcgcaatgaagaccaatccgctacccgcaaccccttccgtgtggggcgggagtaccgtggaactcccccccaccacacgcgataccgcggggcagggcctgcttcggcgcgtcctgcgccccccgatctctcgccgcgacggcccagtgctccccagggggtcgggaccccggagggcggccagcacgctgtggttgcttggcctggacggcacagacgcgccccctggggcgctgacccccaacgacgataccgaacaggccctggacaagatcctgcggggcaccatgcgcgggggggcggccctgatcggctccccgcgccatcatctaacccgccaagtgatcctgacggatctgtgccaacccaacgcggatcgtgccgggacgctgcttctggcgctgcggcaccccgccgacctgcctcacctggcccaccagcgcgccccgccaggccggcagaccgagcggctgggcgaggcctggggccagctgatggaggcgaccgccctggggtcggggcgagccgagagcgggtgcacgcgcgcgggcctcgtgtcgtttaacttcctggtggcggcgtgtgccgcctcgtacgacgcgcgcgacgccgccgatgcggtacgggcccacgtcacggccaactaccgcgggacgcgggtgggggcgcgcctggatcgtttttccgagtgtctgcgcgccatggttcacacgcacgtcttcccccacgaggtcatgcggtttttcggggggctggtgtcgtgggtcacccaggacgagctagcgagcgtcaccgccgtgtgcgccgggccccaggaggcggcgcacaccggccacccgggccggccccgctcggccgtgatcctcccggcgtgtgcgttcgtggacctggacgccgagctggggctggggggcccgggcgcggcgtttctgtacctggtattcacttaccgccagcgccgggaccaggagctgtgttgtgtgtacgtgatcaagagccagctccccccgcgcgggttggagccggccctggagcggctgtttgggcgcctccggatcaccaacacgattcacggcaccgaggacatgacgcccccggccccaaaccgaaaccccgacttccccctcgcgggcctggccgccaatccccaaaccccgcgttgctctgctggccaggtcacgaacccccagttcgccgacaggctgtaccgctggcagccggacctgcgggggcgccccaccgcacgcacctgtacgtacgccgcctttgcagagctcggcatgatgcccgaggatagtccccgctgcctgcaccgcaccgagcgctttggggcggtcagcgtccccgttgtcatcctggaaggcgtggtgtggcgccccggcgagtggcgggcctgcgcgtgagcgtagcaaacgccccgcccacacaacgctccgcccccaaccccttccccgctgtcactcgttgttcgttgacccggacgtccgccaaataaagccactgaaacccgaaacgcgagtgttgtaacgtcctttgggcgggaggaagccacaaaatgcaaatgggatacatggaaggaacacacccccgtgactcaggacatcggcgtgtccttttgggtttcactgaaactggcccgcgccccacccctgcgcgatgtggataaaaagccagcgcgggtggtttagggtaccacaggtgggtgctttggaaacttgtcggtcgccgtgctcctgtgagcttgcgtccctccccggtttcctttgcgctcccgccttccggacctgctctcgcctatcttctttggctctcggtgcgattcgtcaggcagtggccttgtcgaatctcgaccccaccactcgccggacccgccgacgtcccctctcgagcccgccgaaacccgccgcgtctgttgaaatggccagccgccccgccgcatcctctcccgtcgaagcgcgggccccggttgggggacaggaggccggcggccccagcgcagccacccagggggaggccgccggggcccctctcgcccgcggccaccacgtgtactgccagcgagtcaatggcgtgatggtgctttccgacaagacgcccgggtccgcgtcctaccgcatcagcgatagcaactttgtccaatgtggttccaactgcaccatgatcatagacggagacgtggtgcgcgggcgcccccaggacccgggggccgcggcatcccccgctcccttcgttgcggtgacaaacatcggagccggcagcgacggcgggaccgccgtcgtggcattcgggggaaccccacgtcgctcggcggggacgtctaccggtacccagacgaccgacgtccccaccgaggcccttgggggcccccctcctcctccccgcttcaccctgggtggcggctgttgttcctgtcgcgacacacggcgccgctctgcggtattcgggggggagggggatcccgtcggccccgcggagttcgtctcggacgaccggtcgtccgattccgactcggatgactcggaggacaccgactcggagacgctgtcacacgcctcctcggacgtgtccggcggggccacgtacgacgacgcccttgactccgattcgtcatcggatgactccctgcagatagatggccccgtgtgtcgcccgtggagcaatgacaccgcgcccctggatgtttgccccgggacccccggcccgggcgccgacgccggtggtccctcagcggtagacccacacgcaccgacgccaggggccggcgctggtcttgcggccgatcccgccgtggcccgggacgacgcggaggggctttcggacccccggccacgtctgggaacgggcacggcctaccccgtccccctggaactcacgcccgagaacgcggaggccgtggcgcgctttctgggagatgccgtgaaccgcgaacccgcgctcatgctggagtacttttgccggtgcgcccgcgaggaaaccaagcgtgtcccccccaggacattctgcagcccccctcgcctcacggaggacgactttgggcttctcaactacgcgctcgtggagatgcagcgcctgtgtctggacgttcctccggtcctgccgaacgcatacatgccctattatctcagggagtatgtgacgcggctggtcaacgggttcaagccgctggtgagccggtccgctcgcctttaccgcatcctgggggttctggtgcacctgcggatccggacccgggaggcctcctttgaggagtggctgcgatccaaggaagtggccctggactttggcctgacggaaaggcttcgcgagcacgaagcccagctggtgatcctggcccaggctctggaccattacgactgtctgatccacagcacaccgcacacgctggtcgagcgggggctgcaatcggccctgaagtatgaggagttttacctaaagcgctttggcgggcactacatggagtccgtcttccagatgtacacccgcatcgccggctttttggcctgccgggccacgcgcggcatgcgccacatcgccctggggcgagaggggtcgtggtgggaaatgttcaagttctttttccaccgcctctacgaccaccagatcgtaccgtcgacccccgccatgctgaacctggggacccgcaactactacacctccagctgctacctggtaaacccccaggccaccacaaacaaggcgaccctgcgggccatcaccagcaacgtcagcgccatcctcgcccgcaacgggggcatcgggctatgcgtgcaggcgtttaacgactccggccccgggaccgctagcgtcatacccgccctcaaggtcctcgactcgctggtggcggcgcacaacaaagagagcgcgcgtccaaccggcgcgtgcgtgtacctggagccgtggcacaccgacgtgcgggccgtgctccggatgaagggggtcctcgccggcgaagaggcccagcgctgcgacaatatcttcagcgccctctggatgccagacctgtttttcaagcgcctgattcgccacctggacggcgagaagaacgtcacatggaccctgttcgaccgggacaccagcatgtcgctcgccgactttcacggggaggagttcgagaagctctaccagcacctcgaggtcatggggttcggcgagcagatacccatccaggagctggcctatggcattgtgcgcagtgcggccacgaccgggagccccttcgtcatgttcaaagacgcggtgaaccgccactacatctacgacacccagggggcggccatcgccggctccaacctctgcaccgagatcgtccatccggcctccaagcgatccagtggggtctgcaatctgggaagcgtgaatctggcccgatgcgtctccaggcagacgtttgactttgggcggctccgcgacgccgtgcaggcgtgcgtgctgatggtgaacatcatgatcgacagcacgctacaacccacgccccagtgcacccgcggcaacgacaacctgcggtccatgggaatcggcatgcagggcctgcacacggcctgcctgaagctggggctggatctggagtctgtcgaatttcaggacctgaacaaacacatcgccgaggtgatgctgctgtcggcgatgaagaccagcaacgcgctgtgcgttcgcggggcccgtcccttcaaccactttaagcgcagcatgtatcgcgccggccgctttcactgggagcgctttccggacgcccggccgcggtacgagggcgagtgggagatgctacgccagagcatgatgaaacacggcctgcgcaacagccagtttgtcgcgctgatgcccaccgccgcctcggcgcagatctcggacgtcagcgagggctttgcccccctgttcaccaacctgttcagcaaggtgacccgggacggcgagacgctgcgccccaacacgctcctgctaaaggaactggaacgcacgtttagcgggaagcgcctcctggaggtgatggacagtctcgacgccaagcagtggtccgtggcgcaggcgctcccgtgcctggagcccacccaccccctccggcgattcaagaccgcgtttgactacgaccagaagttgctgatcgacctgtgtgcggaccgcgccccctacgtcgaccatagccaatccatgaccctgtatgtcacggagaaggcggacgggaccctcccagcctccaccctggtccgccttctggtccacgcatataagcgcggactaaaaacagggatgtactactgcaaggttcgcaaggcgaccaacagcggggtctttggcggcgacgacaacattgtctgcacgagctgcgcgctgtgaccgacaaaccccctccgcgccaggcccgccgccactgtcgtcgccgtcccacgcgctcccccgctgccatggattccgcggccccagccctctcccccgctctgacggcccatacgggccagagcgcgccggcggacctggcgatccagattccaaagtgccccgaccccgagaggtacttctacacctcccagtgtcccgacattaaccacctgcgctccctcagcatccttaaccgctggctggaaaccgagcttgttttcgtgggggacgaggaggacgtctccaagctttccgagggcgagctcagcttttaccgcttcctcttcgctttcctgtcggccgccgacgacctggttacggaaaacctgggcggcctctccggcctgtttgagcagaaggacattctccactactacgtggagcaggaatgcatcgaagtcgtacactcgcgcgtgtacaacatcatccagctggtgctttttcacaacaacgaccaggcgcgccgcgagtacgtggccggcaccatcaaccacccggccatccgcgccaaggtggactggctggaagcgcgggtgcgggaatgcgcctccgttccggaaaagttcatcctcatgatcctcatcgagggcatcttttttgccgcctcgtttgccgccatcgcctaccttcgcaccaacaaccttctgcgggtcacctgccagtcaaacgacctcatcagccgggacgaggccgtgcacacgacggcctcgtgttacatctacaacaactacctcggcgggcacgccaagcccccgcccgaccgcgtgtacgggctgttccgccaggcggtcgagatcgagatcggatttatccgatcccaggcgccgacggacagccatatcctgagcccggcggcgctggcggccatcgaaaactacgtgcgattcagcgcggatcgcctgttgggccttatccacatgaagccactgttttccgccccaccccccgacgccagctttccgctgagcctcatgtccaccgacaaacacaccaattttttcgagtgtcgcagcacctcctacgccggggcggtcgtcaacgatctgtgagggtcgcggcgcgcttctacccgtgtttgcccataataaacctctgaaccaaactttgggtctcattgtgattcttgtcagggacgcgggggtgggagaggataaaaggcggcgcaaaaagcagtaaccaggtccgtccagattctgagggcataggataccataattttattggtgggtcgtttgttcggggacaagcgcgctcgtctgacgtttgggctactcgtcccagaatttggccaggacgtccttgtagaacgcgggtgggggggcctgggtccgcagctgctccagaaacctgtcggcgatatcaggggccgtgatatgccgggtcacaatagatcgcgccaggttttcgtcgcggatgtcctggtagataggcaggcgtttcagaagagtccacggcccccgctccttggggccgataagcgatatgacgtacttaatgtagcggtgttccaccagctcggtgatggtcatgggatcggggagccagtccagggactctggggcgtcgtggatgacgtggcgtcgccggctggccacataactgcggtgctcttccagcagctgcgcgttcgggacctggacgagctcgggcggggtgagtatctccgaggaggacgacctggggccggggtggcccccggtaacgtcccggggatccagggggaggtcctcgtcgtcttcgtatccgccggcgatctgttgggttagaatttcggtccacgagacgcgcatctcggtgccgccggcggccggcggcaaagggggcctggtttccgtggagcgcgagctggtgtgttcccggcggatggcccgccgggtctgagagcgactcgggggggtccagtgacattcgcgcagcacatcctccacggaggcgtaggtgttattgggatggaggtcggtgtggcagcggacaaagagggccaggaactgggggtagctcatcttaaagtactttagtatatcgcgacagttgatcgtgggaatgtagcaggcgctaatatccaacacaatatcacagcccatcaacaggaggtcagtgtctgtggtgtacacgtacgcgaccgtgttggtgtgatagaggttggcgcaggcatcgtccgcctccagctgacccgagttaatgtaggcgtaccccagggcccggagaacgcgaatacagaacagatgcgccagacgcagggccggcttcgagggcgcggcggacggcagcgcggctccggacccggccgtcccccgggtccccgaggccagagaggtgccgcgccggcgcatgttggaaaaggcagagctgggtctggagtcggtgatgggggaaggcggtggagaggcgtccacgtcactggcctcctcgtccgtccggcattgggccgtcgtgcgggccaggatggccttggctccaaacacaaccggctccatacaattgaccccgcgatcggtaacgaagatggggaaaagggacttttgggtaaacacctttaataagcgacagaggcagtgtagcgtaatggcctcgcggtcgtaactggggtatcggcgctgatatttgaccaccaacgtgtacatgacgttccacaggtccacggcgatgggggtgaagtacccggccggggccccaaggccctggcgcttgaccagatggtgtgtgtgggcaaacttcatcatcccgaacaaacccatgtcaggtcgattgtaactgcggatcggcctaactaaggcgtggttggtgcgacggtccgggacacccgagcctgtctctctgtgtatggtgacccagacaacaacaccgacacaagaggacaataatccgttaggggacgctctttataatttcgatggcccaactccacgcggattggtgcagcaccctgcatgcgccggtgtgggccaaacttccccccgctcattgcctcttccaaaagggtgtggcctaacgagctgggggcgtatttaatcaggctagcgcggcgggcctgccgtagtttctggctcggtgagcgacggtccggttgcttgggtcccctggctgccagcaaaaccccaccctcgcagcggcatacgccccctccgcgtcccgcacccgagaccccggcccggctgccctcaccaccgaagcccacctcgtcactgtggggtgttcccagcccgcattgggatgacggattcccctggcggtgtggcccccgcctcccccgtggaggacgcgtcggacgcgtccctcgggcagccggaggagggggcgccctgccaggtggtcctgcagggcgccgaacttaatggaatcctacaggcgtttgccccgctgcgcacgagccttctggactcgcttctggttatgggcgaccggggcatccttatccataacacgatctttggggagcaggtgttcctgcccctggaacactcgcaattcagtcggtatcgctggcgcggacccacggcggcgttcctgtctctcgtggaccagaagcgctccctcctgagcgtgtttcgcgccaaccagtacccggacctacgtcgggtggagttggcgatcacgggccaggccccgtttcgcacgctggttcagcgcatatggacgacgacgtccgacggcgaggccgttgagctagccagcgagacgctgatgaagcgcgaactgacgagctttgtggtgctggttccccagggaacccccgacgttcagttgcgcctgacgaggccgcagctcaccaaggtccttaacgcgaccggggccgatagtgccacgcccaccacgttcgagctcggggttaacggcaaattttccgtgttcaccacgagtacctgcgtcacatttgctgcccgcgaggagggcgtgtcgtccagcaccagcacccaggtccagatcctgtccaacgcgctcaccaaggcgggccaggcggccgccaacgccaagacggtgtacggggaaaatacccatcgcaccttctctgtggtcgtcgacgattgcagcatgcgggcggtgctccggcgactgcaggtcgccgggggcaccctcaagttcttcctcacgacccccgtccccagtctgtgcgtcaccgccaccggtcccaacgcggtatcggcggtatttctcctgaaaccccagaagatttgcctggactggctgggtcatagccaggggtctccttcagccgggagctcggcctcccgggcctctgggagcgagccaacagacagccaggactccgcgtcggacgcggtcagccacggcgatccggaagacctcgatggcgctgcccgggcgggagaggcgggggcctcgcacgcctgtccgatgccgtcgtcgaccacgcgggtcactcccacgaccaagcgggggcgctcggggggcgaggatgcgcgcgcggacacggccctaaagaaacctaagacggggtcgcccaccgcacccccgcccacagatccagtccccctggacacggaggacgactccgatgcggcggacgggacggcggcccgtcccgccgctccagacgcccggagcggaagccgttacgcgtgttactttcgcgacctcccgaccggagaagcaagccccggcgccttctccgccttccgggggggcccccaaaccccgtatggttttggattcccctgacggggcggggccttggcggccgcccaactctcgcaccatcccgggttaatgtaaataaacttggtattgcccaacactctcccgcgtgtcgcgtgtggttcatgtgtgtgcctggcgtcccccaccctcgggttcgtgtatttcctttccctgtccttataaaagccgtatgtggggcgctgacggaaccaccccgcgtgccatcacggccaaggcgcgggatgctccgcaacgacagccaccgggccgcgtccccggaggacggccagggacgggtcgacgacggacggccacacctcgcgtgcgtgggggccctggcgcgggggttcatgcatatctggcttcaggccgccacgctgggttttgcgggatcggtcgttatgtcgcgcgggccgtacgcgaatgccgcgtctggggcgttcgccgtcgggtgcgccgtgctgggctttatgcgcgcaccccctcccctcgcgcggcccaccgcgcggatatacgcctggctcaaactggcggccggtggagcggcccttgttctgtggagtctcggggagcccggaacgcagccgggggccccgggcccggccacccagtgcctggcgctgggcgccgcctatgcggcgctcctggtgctcgccgatgacgtctatccgctctttctcctcgccccggggcccctgttcgtcggcaccctggggatggtcgtcggcgggctgacgatcggaggcagcgcgcgctactggtggatcggtgggcccgccgcggccgccttggccgcggcggtgttggcgggcccgggggcgaccaccgccagggactgcttctccagggcgtgccccgaccaccgccgcgtctgcgtcatcgtcgcaggcgagtctgtttcccgccgccccccggaggacccagagcgacccggggaccccgggccaccgtcccccccgacaccccaacgatcccaggggccgccggccgatgaggtcgcaccggccggggtagcgcggcccgaaaacgtctgggtgcccgtggtcacctttctgggggcgggcgcgctcgccgtcaagacggtgcgagaacatgcccgggaaacgccgggcccgggcctgccgctgtggccccaggtgtttctcggaggccatgtggcggtggccctgacggagctgtgtcaggcgcttatgccctgggaccttacggacccgctgctgtttgttcacgccggactgcaggtcatcaacctcgggttggtgtttcggttttccgaggttgtcgtgtatgcggcgctagggggtgccgtgtggatttcgttggcgcaggtgctggggctccggcgtcgcctgcacaggaaggaccccggggacggggcccggttggcggcgacgcttcggggcctcttcttctccgtgtacgcgctggggtttggggtgggggcgctgctgtgccctccggggtcaacgggcgggtggtcgggcgattgatatatttttcaataaaaggcattagtcccgaagaccgccggtgtgtgatgatttcgccataacacccaaaccccggatggggcccgggtataaattccggaaggggacacgggctaccctcactaccgagggcgcttggtcgggaggccgcatcgaacgcacacccccatccggtggtccgtgtggaggtcgtttttcagtgcccggtctcgctttgccgggaacgctagccgatccctcgcgagggggaggcgtcgggcatggccccggggcgggtgggccttgccgtggtcctgtggagcctgttgtggctcggggcgggggtggccgggggctcggaaactgcctccaccgggcccacgatcaccgcgggagcggtgacgaacgcgagcgaggcccccacatcggggtcccccgggtcagccgccagcccggaagtcacccccacatcgaccccaaaccccaacaatgtcacacaaaacaaaaccacccccaccgagccggccagccccccaacaacccccaagcccacctccacgcccaaaagcccccccacgtccacccccgaccccaaacccaagaacaacaccacccccgccaagtcgggccgccccactaaaccccccgggcccgtgtggtgcgaccgccgcgacccattggcccggtacggctcgcgggtgcagatccgatgccggtttcggaattccacccgcatggagttccgcctccagatatggcgttactccatgggtccgtcccccccaatcgctccggctcccgacctagaggaggtcctgacgaacatcaccgccccacccgggggactcctggtgtacgacagcgcccccaacctgacggacccccacgtgctctgggcggagggggccggcccgggcgccgaccctccgttgtattctgtcaccgggccgctgccgacccagcggctgattatcggcgaggtgacgcccgcgacccagggaatgtattacttggcctggggccggatggacagcccgcacgagtacgggacgtgggtgcgcgtccgcatgttccgccccccgtctctgaccctccagccccacgcggtgatggagggtcagccgttcaaggcgacgtgcacggccgccgcctactacccgcgtaaccccgtggagtttgtctggttcgaggacgaccgccaggtgtttaacccgggccagatcgacacgcagacgcacgagcaccccgacgggttcaccacagtctctaccgtgacctccgaggctgtcggcggccaggtccccccgcggaccttcacctgccagatgacgtggcaccgcgactccgtgatgttctcgcgacgcaatgccaccgggctggccctggtgctgccgcggccaaccatcaccatggaatttggggtccggcatgtggtctgcacggccggctgcgtccccgagggcgtgacgtttgcctggttcctgggggacgacccctcaccggcggctaagtcggccgttacggcccaggagtcgtgcgaccaccccgggctggctacggtccggtccaccctgcccatttcgtacgactacagcgagtacatctgtcggttgaccggatatccggccgggattcccgttctagagcaccacggcagtcaccagcccccacccagggaccccaccgagcggcaggtgatcgaggcgatcgagtgggtggggattggaatcggggttctcgcggcgggggtcctggtcgtaacggcaatcgtgtacgtcgtccgcacatcacagtcgcggcagcgtcatcggcggtaacgcgagacccccccgttacctttttaatatctatatagtttggtccccctctatcccgcccaccgctgggcgctataaagccgccaccctctcttccctcaggtcatccttggtcgatcccgaacgacacacggcgtggagcaaaacgcctccccctgagccgctttcctaccaacacaacggcatgcctctgcgggcatcggaacacgcctaccggcccctgggccccgggacaccccccatgcgggctcggctccccgccgcggcctgggttggcgtcgggaccatcatcgggggagttgtgatcattgccgcgttggtcctcgtgccctcgcgggcctcgtgggcactttccccatgcgacagcggatggcacgagttcaacctcgggtgcatatcctgggatccgacccccatggagcacgagcaggcggtcggcggctgtagcgccccggcgaccctgatcccccgcgcggctgccaaacagctggccgccgtcgcacgcgtccagtcggcaagatcctcgggctactggtgggtgagcggagacggcattcgggcctgcctgcggctcgtcgacggcgtcggcggtattgaccagttttgcgaggagcccgcccttcgcatatgctactatccccgcagtcccgggggctttgttcagtttgtaacttcgacccgcaacgcgctggggctgccgtgaggcgcgtgtactgcggtctgtctcgtctcctcttctccccttccctccccctccgcatcccaggatcacaccggccaacgagggttgggggggtccggcacggacccaaaataataaacacacaatcacgtgcgataaaaagaacacgcggtcccctgtggtgtttttggttatttttattaaatctcgtcgacaaacagggggaaaggggcgtggtctagcgacggcagcacgggcggaggcgttcaccggctccggcgtccttcgcgtttaagcttggtcaggagggcgctcagggcggcgacgttggtcgggccgtcgttggtcagggcgttggctcgatggcgggcgaggacgggcgaggggctcaacggcgggggcgggggtccggtgcggcccgggggggaaaatagggcggatcccccccagtcgtacaggggattttccgcctcaatgtacggggaggccggcgctgcattcgccgtgttcacgcagacgttttcgtagacccgcatccatggtatttcctcgtagacacgccccccgtcctcgctcacggtctcgtatattgactcgtcgtcctcgtagggggcgtgccgttcgcgggccgaggcggcgtgggtggctttgcggcgggcgtcgtcgtcgtcgtcgtcggccgtcagatacgtggcttccatctggtcgggttctccctccggggcgggtccccacacccgtggccgatcgaggctccccagagacgcgcgccggacaagaagggggcacgtcgccgccggcggtcgcctgtcgggtcccgcgacgttacgggccgggaggcgcgggggcacctcccccatgtgcgtgtaatacgtggccggctgtgcggccgcagcggggggctcggcgaccgggtcgtccgcatccggaagcgggggccccgcgccgtccgcacggcgcctccggaaccgccgggtggacggcgcgggggtcgagtgtaggcgaggtcgggggaggggcgggggctcgttgtcgcgccgcgcccgctgaatcttttcccgacaggtcccaccccccgcgcgatgcccccccgggccgcgggccatgtcgtccgggggaggccccgcggaccacgtcgtccggcgagacgccacgagccgcaggatggactcgtagtggagcgacggcgccccgctgcggagcagatccgcggccagggcggccccgaaccaagccttgatgctcaactccatccgggcccagctgggggcggtcatcgtggggaacaggggggcggtggtccgacagaaacgctcctggctgtccaccgcggcccgcagatactcgttgttcaggctgtcggtggcccagacgccgtacccggtgagggtcgcgttgatgatatactgggcgtggtgatggacgatcgacagaacctccaccgtggataccacggtatccacggtcccgtacgtaccgccgctccgcttgccggtctgccacaggttggctaggcacgtcaggtggcccaggacgtcgctgaccgccgccctgagcgccatgcactgcatggagccggtcgtgccgctgggaccccggtccagatggcgcgcgaacgtttccgcgggcgcctccgggctgccgccgagcgggaggaaccggcgattggagggactcagccggtgacatacgtgcttgtccgtcgtccacagcatccaggacgcccaccggtacagcacggagacgtaggccaggagctcgttgagccgcagtgcggtgtcggtgctggggcggcttgggtccgccgggcgcataaagaacatgtactgctgaatccgatggagggcgtcgcgcaggccggccacggtggcggcgtacttggccgccgcggccccgctcttgaacggggtgcgcgccagcagctttggcgccagggtgggccgcagcagcacgtgaaggctggggtcgcagtcgcccacggggtcctcggggacgtccaggccgctgggcaccaccgtctgcaggtacttccagtactgcgtgaggatggcgcggctcaactggccgccgggcagctccacctcgcccagcgcctgggtggcggccgaagcgtagtgccggatgtactcgtagtgcgggtcgctggcgagcccgtccacgatcaaactctcgggaaccgtgttgtgttgccgcgcggccaaccggacgctgcgatcggtgcaggtcagaaacgccggctgcgcgtcgtcggagcgctgccgcaaggcgcccacggccgcgctaaggagcccctccggggtggggagcagacacccgccgaagatgcgccgctcgggaacgcccgcgttgtcgccgcggatcaggttggcaggcgtcaggcaccgcgccagccgcagggagctcgcgccgcgcgtccggcgctgcatggtgacgcccgttcggtcgggacccgccggtcggagttatgccgcgtccagggccatcggggcgctttttatcgggaggagcttatgggcgtggcgggcctcccagcccggtcgcgcgcctccccgacacgtgcgcccgcagggcggcggccccctcgtctcccatcagcagtttcctaaactgggacatgatgtccaccacgcggacccgcgggcccaacacggacccgccgcttacgggggcgggggggaagggctccaggtccttgagcagaaaggcggggtctgccgtcccggacacgggggcccggggcgcggaggaggcggggcgcagatccacgtgctccgcggccgcgcggacgtccgcccagaacttggcgggggtggtgcgcgcgtacaggggctgggtcgctcggaggacacacgcgtagcgcaggggggtgtacgtgcccacctcgggggccgtgaatcccccgtcaaacgcggccagtgtcacgcacgccaccacggtgtcggcaaagcccagcagccgctgcaggacgagcccggcggccagaatggcgcgcgtggtcgcagcgtcgtcccggcgccggtgcgcgtccccgcacgcccgggcgtactttaaggtcactgtcgccagggccgtgtgcagcgcgtacaccgcagcgcccagcacggcgttgagcccgctgttggcgagcagccggcgcgctgcggtgtcgcccagcgcctcgtgctcggcccccacgaccgcggggcttcccaggggcagggcgcgaaacagctcctcccgcgccacgtccgcaaaggcggggtggtgcacgtgcgggtgcaggcgcgcccccacgaccaccgagagccactggaccgtctgctccgccatcaccgccaacacatccagcacgcgccccaggaaggcggcctcccgcgtcaaaacgcaccggacggcgtcgggattgaagcgggcgagcagggccccggtggccaggtacgtcatgcggccggcatagcgggcggccacgcgacagtcgcggtccagcagcgcgcgcaccccgggccagtacagcagggaccccagcgagctgcgaaacaccgcggcgtcggggccggattggggggacactaacccccccgcgctcagtaacggcacggccgcggccccgacgggacgcaacgccgtgaggctcgcgaactgccgcctcagctcggcagccctgtcgtccaggtccgacccgcgcgcctctgcgtgaaggcgcgtcccgcacacccacccgttgatggccagccgcacgacggcatccgccaaaaagctcatcgcctgggcggggctggtttttgttcgacgatccgtcaggtcaagaatcccatcgcccgtgatataccaggccaacgcctcgccctgctgcagggtttggcggaaaaacaccgcggggttgtcgggggaggcgaagtgcatgacccccacgcgcgataacccgaacgcgctatccggacacgggtaaaacccggccggatgccccagggctagggcggagcgcacggactcgtcccacacggcaacctgaggggccagtcgatccaacgggaatgccgcccggagctccgggcccggcacgcgtccctccagaacctccaccttgggcggggaacgggccccgccgccgtcctccggcccgacgtcttccgggtagtcgtcctcctcgtactgcagttcctctaggaacagcggcgacggcgccacccgcgaaccgccgacccgccccaaaatagcccgcgcgtcgacgggacccaggtatcccccctgccgggcctgcggaggaccgcggggaacctcatcatcatcgtccaggcgaccgcgcaccgactggctacgggccgcatcgggcccggggcgctgccgggacgctcggcgatgggatgagggcggggcttccgacgcgcgccgtcgtcgggctcgcgggccttcccgtcgacggcgcacgggcggctcgtcgcccgccatctcctccagagcctctagctcgctgtcgtcatccccgcggaacaccgcacgcaggtaccccatgaaccccaccccatcgcccgctggctcgtccgccacgggcgaggcgcgggggcgggtggatgcgcgcctcctgcgccccgcgggttcgcgagccgacatggtggcgatagacgcgggttatcggatgtccgctaccccccaaaaaagaaaaagaccccacagcgcggatggaggtcggggtaggtgccgccggaccccctcgcgatgggaatggacgggagcgacggggccggcgcaaaaaacgcagtatctcccgcgaaggctacccgccgccccagcccccggccaaatgcggaaacggtcccgcgctctcgcctttatacgcgggccgccctgcgacacaatcacccgtccgtggtttcgaatctacacgacaggcccgcagacgcggctaacacacacgccggcaacccagaccccagtgggttggttgcgcggtcccgtctcctggctagttctttcccccaccaccaaataatcagacgacaaccgcaggtttttgtaatgtatgtgctcgtgtttattgtggatacgaaccggggacgggaggggaaaacccagacgggggatgcgggtccggtcgcgccccctacccaccgtactcgtcaattccaagggcatcggtaaacatctgctcaaactcgaagtcggccatatccagagcgccgtagggggcggagtcgtggggggtaaatcccggacccggggaatccccgtcccccaacatgtccagatcgaaatcgtctagcgcgtcggcatgcgccatcgccacgtcctcgccgtctaagtggagctcgtcccccaggctgacatcggtcgggggggccgtcgacagtctgcgcgtgtgtcccgcggggagaaaggacaggcgcggagccgccagccccgcctcttcgggggcgtcgtcgtccgggagatcgagcaggccctcgatggtagacccgtaattgtttttcgtacgcgcgcggctgtacgcgtgttcccgcatgaccgcctcggagggcgaggtcgtgaagctggaatacgagtccaacttcgcccgaatcaacaccataaagtacccagaggcgcgggcctggttgccatgcagggtgggaggggtcgtcaacggcgcccctggctcctccgtagccgcgctgcgcaccagcgggaggttaaggtgctcgcgaatgtggtttagctcccgcagccggcgggcctcgattggcactccccggacggtgagcgctccgttgacgaacatgaagggctggaacagacccgccaactgacgccagctctccaggtcgcaacagaggcagtcaaacaggtcgggccgcatcatctgctcggcgtacgcggcccataggatctcgcgggtcaaaaatagatacaaatgcaaaaacagaacacgcgccagacgagcggtctctcggtagtacctgtccgcgatcgtggcgcgcagcatttctcccaggtcgcgatcgcgtccgcgcatgtgcgcctggcggtgcagctgccggacgctggcgcgcaggtaccggtacagggccgagcagaagttggccaacacggttcgatagctctcctcccgcgcccgtagctcggcgtggaagaaacgagagagcgcttcgtagtagagcccgaggccgtcgcgggtggccggaagcgtcgggaaggccacgtcgccgtgggcgcgaatgtcgatttgggcgcgttcggggacgtacgcgtccccccattccaccacatcgctgggcagcgttgataggaatttacactcccggtacaggtcggcgttggtcggtaacgccgaaaacaaatcctcgttccaggtatcgagcatggtacatagcgcggggcccgcgctaaagcccaagtcgtcgaggagacggttaaagagggcggcgggggggacgggcatgggcggggagggcatgagctgggcctggctcaggcgccccgttgcgtacagcggaggggccgccggggtgtttttgggacccccggccgggcgggggggtggtggcgaagcgccgtccgcgtccatgtcggcaaacagctcgtcgaccaagaggtccattgggtggggttgatacgggaaagacgatatcgggcttttgatgcgatcgtccccgcccgcccagagagtgtgggacgcccgacggcgcgggaagagaaaaacccccaaacgcgttagaggaccggacggaccttatggggggaagtgggcagcgggaaccccgtccgttcccgaggaatgacagcccgtggtcgccaccccgcatttaagcaacccgcacgggccgccccgtacctcgtgacttccccccacattggctcctgtcacgtgaaggcaaaccgagggcggctgtccaacccaccccccgccacccagtcacggtccccgtcggattgggaaacaaaggcacgcaacgccaacaccgaatgaacccctgttggtgctttattgtctgggtacggaagtttttcactcgacgggccgtctggggcgagaagcggagcgggctggggctcgaggtcgctcggtggggcgcgacgccgcagaacgccctcgagtcgccgtggccgcgtcgacgtcctgcaccacgtctggattcaccaactcgttggcgcgctgaatcaggtttttgccctcgcagaccgtcacgcggatggtggtgatgccaaggagttcgttgaggtcttcgtctgtgcgcggacgcgacatgtcccagagctggaccgccgccatccgggcatgcatggccgccaggcgcccaaccgcggcgcagaagacgcgcttgttaaagccggccacccggggggtccatggcgcgtcggggtttgggggggcggtgctaaagtgcagctttctggccagcccctgcgcgggtgtcttggatcgggttggcgccgtcgacgcgggggcgtctgggagtgcggcggattctggctgggccgatttcctgccgcgggtggtctccgccgccggggccgcgggggccttagtcgccacccgctgggttcggggggcccggggggcggtggtgggtgtgcgtccggcccctccggacccagcgggcggcggaggcgcccgcgcaggccccggggcggacaaaaccgccccggaaacgggacgccgcgtccgggggacctccgggtgttcgtcgtcttcggatgacgagcccccgtagagggcataatccgactcgtcgtactggacgaaacggacctcgccccttgggcgcgcgcgtgtctgtagggcgccacggcgggaggtgtcaggcggactatcgggactcgccatacatgaagacggggtgtagtacagatcctcgtactcatcgcgcggaacctcccgcggacccgacttcacggagcggcgagaggtcatggttccacgaacacgctagggtcggatgcgcggacaattaggcctgggttcggacggcgggggtggtgcaggtgtggagaggtcgagcgataggggcggcccgggagagaagagagggtccgcaaaacccactggggatgcgtgagtggccctctgtgggcggtgggggagagtcttataggaagtgcatataaccacaacccatgggtctaaccaatccccaggggccaagaaacagacacgccccaaacggtctcggtttccgcgaggaaggggaagtcctgggacaccctccacccccacccctcaccccacacagggcgggttcaggcgtgcccggcagccagtagcctctggcagatctgacagacgtgtgcgataatacacacgcccatcgaggccatgcctacataaaagggcaccagggcccccggggcagacatttggccagcgttttgggtctcgcaccgcgcgcccccgatcccatcgcgcccgccctcctcgccgggcggctccccgtgcgggcccgcgtctcccgccgctaaggcgacgagcaagacaaacaacaggcccgcccgacagacccttctgggggggcccatcgtccctaacaggaagatgagtcagtggggatccggggcgatccttgtccagccggacagcttgggtcgggggtacgatggcgactggcacacggccgtcgctactcgcgggggcggagtcgtgcaactgaacctggtcaacaggcgcgcggtggcttttatgccgaaggtcagcggggactccggatgggccgtcgggcgcgtctctctggacctgcgaatggctatgccggctgacttttgtgcgattattcacgcccccgcgctatccagcccagggcaccacgtaatactgggtcttatcgactcggggtaccgcggaaccgttatggccgtggtcgtagcgcctaaaaggacgcgggaatttgcccccgggaccctgcgggtcgacgtgacgttcctggacatcctggcgacccccccggccctcaccgagccgatttccctgcggcagttcccgcaactggcgcccccccctccaaccggggccgggatacgcgcagatccttggttggagggggcgctcggggacccaagcgtgactcctgccctaccggcgcgacgccgagggcggtccctcgtctatgccggcgagctgacgccggttcagacggaacacggggacggcgtacgagaagccatcgccttccttccaaaacgcgaggaggatgccggtttcgacattgtcgtccgtcgcccggtcaccgtcccggcaaacggcaccacggtcgtgcagccatccctccgcatgctccacgcggacgccgggcccgcggcctgctatgtgctggggcggtcgtcgctcaacgcccgcggcctcctggtcgttcctacgcgctggctccccgggcacgtatgtgcgtttgttgtttacaaccttacgggggttcctgtgaccctcgaggccggcgccaaggtcgcccagctcctggttgcgggggcggacgctcttccttggatccccccggacaactttcacgggaccaaagcgcttcgaaactaccccaggggtgttccggactcaaccgccgaacccaggaacccgccgctcctggtgtttacgaacgagtttgacgcggaggcccccccgagcgagcgcgggaccgggggttttggctctaccggtatttagcccatagcttggggttcgttccgggcaataaaaaacgtttgtatctcatctttcctgtgtgtagttgtttctgttggatgcctgtgggtctatcacacccgcccctccatcccacaaacacagaacacacgggttggatgaaaacacgcatttattgacccaaaacacacggagctgctcgagatgggccagggcgaggtgcggttggggaggctgtaggtctgggaacggacacgcggggacacgattccggtttggggtccgggagggcgtcgccgtttcgggcggcaggcgccagcgtaacctccgggggcggcgtgtgggggtgccccaaggagggcgcctcggtcaccccaagcccccccgagcgggttcccccggcaaccccgaaggcggagaggccaagggcccgttcggcgatggccacatcctccatgaccacgtcgctctcggccatgctccgaatagcctgggagacgagcacatccgcggacttgtcagccgcccccacggacatgtacatctgcaggatggtggccatacacgtgtccgccaggcgccgcatcttgtcctgatgggccgccacggccccgtcgatcgtgggggcctcgagcccggggtggtggcgcgccagtcgttctaggttcaccatgcaggcgtggtacgtgcgggccaaggcgcgggccttcacgaggcgtcgggtgtcgtccagggaccccagggcgtcatcgagcgtgatgggggcgggaagtagcgcgttaacgaccaccagggcctcctgcagccgcggctccgcctccgagggcggaacggccgcgcggatcatctcatattgttcctcggggcgcgctccccagccacatatagccccgagaagagaagccatcgcgggcgggtactggcccttgggcgcgcggacgcaatggggcaggaagacgggaaccgcggggagaggcgggcggccgggactcccgtggaggtgaccgcgctttatgcgaccgacgggtgcgttattacctcttcgatcgccctcctcacaaactctctactgggggccgagccggtttatatattcagctacgacgcatacacgcacgatggccgtgccgacgggcccacggagcaagacaggttcgaagagagtcgggcgctctaccaagcgtcgggcgggctaaatggcgactccttccgagtaaccttttgtttattggggacggaagtgggtgggacccaccaggcccgcgggcgaacccgacccatgttcgtctgtcgcttcgagcgagcggacgacgtcgccgcgctacaggacgccctggcgcacgggaccccgctacaaccggaccacatcgccgccaccctggacgcggaggccacgttcgcgctgcatgcgaacatgatcctggctctcaccgtggccgtcaacaacgccagcccccgcaccggacgcgacgccgccgcggcgcagtatgatcagggcgcgtccctacgctcgctcgtggggcgcacgtccctgggacaacgcggccttaccacgctatacgtccaccacgaggcgcgcgtgctggccgcgtaccgcagggcgtattatggaagcgcgcagagtcccttctggtttcttagcaaattcgggcctgacgaaaaaagcctggtgctcaccactcggtactacctgcttcaggcccagcgtctggggggcgcgggggccacgtacgacctgcaggccatcaaggacatctgcgccacctacgcgattccccacgccccccgccccgacaccgtcagcgccgcgtccctgacctcgtttgccgccatcacgcggttctgttgcacgagccagtacgcccgcggggccgcggcggccgggtttccgctttacgtggagcgccgtattgcggccgacgtccgcgagaccagtgcgctggagaagttcataacccacgatcgcagttgcctgcgcgtgtccgaccgtgaattcattacgtacatttacctggcccattttgagtgtttcagccccccgcgcctagccacgcatcttcgggccgtgacgacccaggaccccaaccccgcggccaacacggagcagccctcgcccctgggcagggaggccgtggaacaatttttttgccacgtgcgcgcccaactgaatatcggggagtacgtcaaacacaacgtgaccccccgggagaccgtcctggatggcgatacggccaaggcctacctgcgcgctcgcacgtacgcgcccggggccctgacgcccgcccccgcgtattgcggggccgtggactccgccaccaaaatgatggggcgtttggcggacgccgaaaagctcctggtcccccgcgggtggcccgcgtttgcgcccgccagtcccggggaggatacggcgggcggcacgccgcccccacagacctgcggaatcgtcaagcgcctcctgagactggccgccacggaacaacaggacaccacgcccccggcgatcgcggcgcttatccgtaatgcggcggtgcagactcccctgcccgtctaccggatatccatggtccccacgggacaggcatttgccgcgctggcctgggacgactgggcccgcataacgcgggacgctcgcctggccgaagcggtcgtgtccgccgaagcggcggcgcaccccgaccacggcgcgctgggcaggcggctcacggatcgcatccgcgcccagggccccgtgatgccccctggcggcctggatgccggggggcagatgtacgtgaatcgcaacgagatatttaacggcgcgctggcaatcacaaacatcatcctggatctcgacatcgccctgaaggagcccgtcccctttcgccggctccacgaggccctgggccactttaggcgcggggctctggcggcggttcagctcctgtttcccgcggcccgcgtggaccccgacgcatatccctgttattttttcaaaagcgcatgtcggcccggcccggcgtccgtgggttccggcagcggactcggcaacgacgacgacggggactggtttccctgctacgacgacgccggtgatgaggagtgggcggaggacccgggcgccatggacacatcccacgatcccccggacgacgaggttgcctactttgacctgtgccacgaagtcggccccacggcggaacctcgcgaaacggattcgcccgtgtgttcctgcaccgacaagatcggactgcgggtgtgcatgcccgtccccgccccgtacgtcgtccacggttctctaacgatgcggggggtggcacgggtcatccagcaggcggtgctgttggaccgagattttgtggaggccatcgggagctacgtaaaaaacttcctgttgatcgatacgggggtgtacgcccacggccacagcctgcgtttgccgtattttgccaaaatcgcccccgacgggcctgcgtgcggaaggctgctgccagtgtttgtgatcccccccgcctgcaaagacgttccggcgtttgtcgccgcgcacgccgacccgcggcgcttccattttcacgccccgcccacctatctcgcttccccccgggagatccgtgtcctgcacagcctgggtggggactatgtgagcttctttgaaaggaaggcgtcccgcaacgcgctggaacactttgggcgacgcgagaccctgacggaggtcctgggtcggtacaacgtacagccggatgcgggggggaccgtcgaggggttcgcatcggaactgctggggcggatagtcgcgtgcatcgaaacccactttcccgaacacgccggcgaatatcaggccgtatccgtccggcgggccgtcagtaaggacgactgggtcctcctacagctagtccccgttcgcggtaccctgcagcaaagcctgtcgtgtctgcgctttaagcacggccgggcgagtcgcgccacggcgcggacattcgtcgcgctgagcgtcggggccaacaaccgcctgtgcgtgtccttgtgtcagcagtgctttgccgccaaatgcgacagcaaccgcctgcacacgctgtttaccattgacgccggcacgccatgctcgccgtccgttccctgcagcacctctcaaccgtcgtcttgataacggcgtacggcctcgtgctcgtgtggtacaccgtcttcggtgccagtccgctgcaccgatgtatttacgcggtacgccccaccggcaccaacaacgacaccgccctcgtgtggatgaaaatgaaccagaccctattgtttctgggggccccgacgcacccccccaacgggggctggcgcaaccacgcccatatctgctacgccaatcttatcgcgggtagggtcgtgcccttccaggtcccacccgacgccacgaatcgtcggatcatgaacgtccacgaggcagttaactgtctggagaccctatggtacacacgggtgcgtctggtggtcgtagggtggttcctgtatctggcgttcgtcgccctccaccaacgccgatgtatgtttggtgtcgtgagtcccgcccacaagatggtggccccggccacctacctcttgaactacgcaggccgcatcgtatcgagcgtgttcctgcagtacccctacacgaaaattacccgcctgctctgcgagctgtcggtccagcggcaaaacctggttcagttgtttgagacggacccggtcaccttcttgtaccaccgccccgccatcggggtcatcgtaggctgcgagttgatgctacgctttgtggccgtgggtctcatcgtcggcaccgctttcatatcccggggggcatgtgcgatcacataccccctgtttctgaccatcaccacctggtgttttgtctccaccatcggcctgacagagctgtattgtattctgcggcggggcccggcccccaagaacgcagacaaggccgccgccccggggcgatccaaggggctgtcgggcgtctgcgggcgctgttgttccatcatcctgtcgggcatcgcaatgcgattgtgttatatcgccgtggtggccggggtggtgctcgtggcgcttcactacgagcaggagatccagaggcgcctgtttgatgtatgacgtcacatccaggccggcggaaaccggaacggcatatgcaaactggaaactgtcctgtcttggggcccacccacccgacgcgtcatatgtaaatgaaaatcgttcccccgaggccatgtgtagcctggatcccaacgaccccgcccatgggtcccaattggccgtcccgttaccaagaccaacccagccagcgtatccacccccgcccgggtccccgcggaagcggaacggtgtatgtgatatgctaattaaatacatgccacgtacttatggtgtctgattggtccttgtctgtgccggaggtggggcgggggccccgcccggggggcggaactaggaggggtttgggagagccggccccggcaccacgggtataaggacatccaccacccggccggtggtggtgtgcagccgtgttccaaccacggtcacgcttcggtgcctctccccgattcgggcccggtcgcttgctaccggtgcgccaccaccagaggccatatccgacaccccagccccgacggcagccgacagcccggtcatggcgactgacattgatatgctaattgacctcggcctggacctctccgacagcgatctggacgaggacccccccgagccggcggagagccgccgcgacgacctggaatcggacagcaacggggagtgttcctcgtcggacgaggacatggaagacccccacggagaggacggaccggagccgatactcgacgccgctcgcccggcggtccgcccgtctcgtccagaagaccccggcgtacccagcacccagacgcctcgtccgacggagcggcagggccccaacgatcctcaaccagcgccccacagtgtgtggtcgcgcctcggggcccggcgaccgtcttgctcccccgagcggcacgggggcaaggtggcccgcctccaacccccaccgaccaaagcccagcctgcccgcggcggacgccgtgggcgtcgcaggggtcggggtcgcggtggtcccggggccgccgatggtttgtcggacccccgccggcgtgcccccagaaccaatcgcaacccggggggaccccgccccggggcggggtggacggacggccccggcgccccccatggcgaggcgtggcgcggaagtgagcagcccgacccacccggaggcccgcggacacggagcgtgcgccaagcaccccccccgctaatgacgctggcgattgcccccccgcccgcggacccccgcgccccggccccggagcgaaaggcgcccgccgccgacaccatcgacgccaccacgcggttggtcctgcgctccatctccgagcgcgcggcggtcgaccgcatcagcgagagcttcggccgcagcgcacaggtcatgcacgacccctttggggggcagccgtttcccgccgcgaatagcccctgggccccggtgctggcgggccaaggagggccctttgacgccgagaccagacgggtctcctgggaaaccttggtcgcccacggcccgagcctctatcgcacttttgccggcaatcctcgggccgcatcgaccgccaaggccatgcgcgactgcgtgctgcgccaagaaaatttcatcgaggcgctggcctccgccgacgagacgctggcgtggtgcaagatgtgcatccaccacaacctgccgctgcgcccccaggaccccattatcgggacggccgcggcggtgctggataacctcgccacgcgcctgcggccctttctccagtgctacctgaaggcgcgaggcctgtgcggcctggacgaactgtgttcgcggcggcgtctggcggacattaaggacattgcatccttcgtgtttgtcattctggccaggctcgccaaccgcgtcgagcgtggcgtcgcggagatcgactacgcgacccttggtgtcggggtcggagagaagatgcatttctacctccccggggcctgcatggcgggcctgatcgaaatcctagacacgcaccgccaggagtgttcgagtcgtgtctgcgagttgacggccagtcacatcgtcgcccccccgtacgtgcacggcaaatatttttattgcaactccctgttttaggtacaataaaaacaaaacatttcaaacaaatcgccccacgtgttgtccttctttgctcatggccggcggggcgtgggtcacggcagatggcgggggtgggcccggcgtacggcctgggtgggcggagggaactaacccaacgtataaatccgtccccgctccaaggccggtgtcatagtgcccttaggagcttcccgcccgggcgcatccccccttttgcactatgacagcgacccccctcaccaacctgttcttacgggccccggacataacccacgtggcccccccttactgcctcaacgccacctggcaggccgaaacggccatgcacaccagcaaaacggactccgcttgcgtggccgtgcggagttacctggtccgcgcctcctgtgagaccagcggcacaatccactgctttttctttgcggtatacaaggacacccaccatacccctccgctgattaccgagctccgcaactttgcggacctggttaaccacccgccggtcctacgcgaactggaggataagcgcggggtgcggctgcggtgtgcgcggccgtttagcgtcgggacgattaaggacgtctctgggtccggcgcgtcctcggcgggagagtacacgataaacgggatcgtgtaccactgccactgtcggtatccgttctcaaaaacatgctggatgggggcctccgcggccctacagcacctgcgctccatcagctccagcggcatggccgcccgcgcggcagagcatcgacgcgtcaagattaaaattaaggcgtgatctccaaccccccatgaatgtgtgtaaccccccccaaaaaaataaagagccgtaacccaaccaaaccaggcgtggtgtgagtttgtggacccaaagccctcagagacaatgcgacaggccagtatggaccgtgatacttttatttattaactcacaggggcgcttaccgccacaggaataccagaataatgaccaccacaatcgcgaccaccccaaatacagcatggcgccacaccacgccacaacagccctgtcgccggtatggggcatgatcagacgagccgcgcgccgcgcgttgggccctgtacagctcgcgcgaattgaccctaggaggccgccacgcgcccgagttttgcgttcgtcgctggtcgtcgggcgccaaagccccggacggctgttcggtcgaacgaacggccacgacagtggcataggttggggggtggtccgacatagcctcggcgtacgtcgggaggcccgacaagaggtcccttgtgatgtcgggtggggccacaagcctggtttccggaagaaacaggggggttgccaataacccgccagggccaaaactccggcgctgcgcacgtcgttcggcgcggcgccgggcgcgccgagcggctcgctgggcggcttggcgtgagcggccccgctccgacgcctcgccctctccggaggaggttggcggaattggcacggacgacaggggcccagcagagtacggtggaggtgggtccgtgggggtgtccagatcaataacgacaaacggcccctcgttcctaccagacaagctatcgtaggggggcgggggatcagcaaacgcgttccccgcgctccatagacccgcgtcgggttgcgccgcctccgaagccatggatgcgccccaaagccacgactcccgcgcgctaggtccttggggtaagggaaaaggccctactccccatccaagccagccaagttaacgggctacgccttcggggatgggactggcaccccggcggattttgttgggctggtacgcgtcgcccaaccgagggccgcgtccacgggacgcgccttttataaccccggggtcattcccaacgatcacatgcaatctaactggctcccctctccccccctctcccctctccccccctctcccctctccccccctctcccctctccccccctctcccctctccccccctctcccctctccccccctctcccctctccccccctctcccctctccccccctctcccctctccccccctctcccctctccccccctctcccctgctctttccccgtgacacccgacgctggggggcgtggctgccgggaggggccgcgtatgggcgggcctactcggtctcccgcccccccgaaccgccccgccggctttgcccccctttgatcccctgctacccccaccccgtgctcgtggtgcggggtggggggatgtgggcgggggtgcgcgggaggtgtcggtggtgggggtggtggtggtggtggtagtaggaatggtggtgggggggagggcgctggttggtcaaaaaagggagggacgggggccggcagaccgacggcgacaacgctccccggcggccgggtcgcggctcttacgagcggcccggcccgcgctcccaccccccgggccgtgtccttgctttccccccgtctccccccccgccttctcctcctcctcctcgtttttccaaaccccgcccacccggcccggcccggcccggcccggccaccgccgcccacccacccacctcgggatacccagccccggtcccccgttccccgggggccgttatctccagcgccccgtccggcgcgccgccccccgccgctaaaccccatcccgcccccgggaccccacatataagcccccagccacacgcaagaacagacacgcagaacggctgtgtttattttaaataaaccgatgtcggaataaacaaacacaaacacccgcgacggggggacggaggggacggagggaggggggtgacgggggacggaaacagacacaaaaaacaaccacaaaaaacaaccacccaccgacacccccaccccagtctcctcgccttctcccacccaccccacgcccccactgagcccggtcgatcgacgagcacccccgcccacgcccccgcccctgccccggcgacccccggcccgcacgatcccgacaacaataacaaccccaacggaaagcggcggggtgttgggggaggcgaggaacaaccgaggggaacgggggatggaaggacgggaagtggaagtcctgatacccatcctacacccccctgccttccaccctccggccccccgcgagtccacccgccggccggctaccgagaccgaacacggcggccaccgccgccgccgccgccgacaccgcagagccggcgcgcgcacacacaagcggcagaggcagaaaggccccgagtcattgtttatgtggccgcgggccagcagacggcccgcgacacccccccccgcccgtgtgggtatccggccccccgccccgcgccggtccattaagggcgcgcgtgcccgcgagatatcaatccgttaagtgctctgcagacaggggcaccgcgcccggaaatccattaggccgcagacgaggaaaataaaattacatcacctacccatgtggtgctgtggcctgtttttgctgcgtcatctgagcctttataaaagcgggggcgcggccgtgccgatcgccggtggtgcgaaagactttccgggcgcgtccgggtgccgcggctctccgggcccccctgcagccggggcggccaaggggcgtcggcgacatcctccccctaagcgccggccggccgctggtctgttttttcgttttccccgtttcgggggtggtgggggttgcggtttctgtttctttaacccgtctggggtgtttttcgttccgtcgccggaatgtttcgttcgtctgtcccctcacggggcgaaggccgcgtacggcccgggacgaggggcccccgaccgcggcggtccgggccccgtccggacccgctcgccggcacgcgacgcgaaaaaggccccccggaggcttttccgggttcccggcccggggcctgagatgaacactcggggttaccgccaacggccggcccccgtggcggcccggcccggggccccggcggacccaaggggccccggcccggggccccacaacggcccggcgcatgcgctgtggtttttttttcctcggtgttctgccgggctccgtcgcctttcctgttctcgcttctcccccccccccttcacccccagtaccctcctccctcccttcctcccccgttatcccactcgtcgagggcgccccggtgtcgttcaacaaagacgccgcgtttccaggtaggttagacacctgcttctccccaatagagggggggggacccaaacgacagggggcgccccagaggctaaggtcggccacgccactcgcgggtgggctcgtgttacagcacaccagcccgttattttccccccctcccacccttagttagactctgttacttacccgtccgaccaccaactgcccccttatctaagggccggctggaagaccgccagggggtcggccggtgtcgctgtaaccccccacgccaatgacccacgtactccaagaaggcatgtgtcccaccccgcctgtgtttttgtgcctggctctctatgcttgggtcttactgcctggggggggggagtgcgggggagggggggggtgtggaaggaaatgcacggcgcgtgtgtacccccccctaaagttgttcctaaagcgaggatatggaggagtggcgggtgccgggggaccggggtgatctctggcacgcgggggtgggaagggtcgggggagggggggatggggtaccggcccacctggccggcgcgggtgcgcgtgcctttgcacaccaaccccacgtcccccggcggtctctaagaaacaccgccccccctccttcataccaccgagcatgcctgggtgtgggttggtaaccaacacgcccatcccctcgtctcctgtgattctctggctgcaccgcattcttgttttctaactatgttcctgtttctgtctccccccccacccctccgccccaccccccaacacccacgtctgtggtgtggccgacccccttttgggcgccccgtcccgccccgctacccctcccatcctttgttgccctatagtgtagttaacccccccccccgccctttgtggcggccagaggccaggtcagtccgggcgggcaggcgctcgcggaaacttaacacccacacccaacccactgtggttctggctccatgccagtggcaggatgctttcggggatcggtggtcaggcagcccgggccgcggctctgtggttaacaccagagcctgcccaacatggcacccccactcccacgcacccccactcccacgcacccccactcccacgcacccccactcccacgcacccccactcccacgcacccccactcccacgcacccccactcccacgcacccccactcccacgcacccccactcccacgcacccccgcgatacatccaacacagacagggaaaagatacaaaagtaaacctttatttcccaacagacagcaaaaatcccctgagttttttttattagggccaacacaaaagacccgctggtgtgtggtgcccgtgtctttcactttccacctccccgacacggattggctggtgtagtgggcgcggccagagaccacccagcgcccgacccccccctccccacaaacacgggggcgtcccttattgttttccctcgtcccgggtcgacgccccctgctccccggaccacgggtgccgagaccgcaggctgcggaagtccagggcgcccactagggtgccctggtcgaacagcatgttccccacgggggtcatccagaggctgttccactccgacgcgggggccgtcgggtactcggggggcgtcacgtggttacccgcggtctcggggagcagggtgcggcggctccagccggggaccgcggcccgcagccgggtcgccatgtttcccgtctggtccaccaggaccacgtacgccccgatgttccccgtctccatgtccaggatgggcaggcagtcccccgtgatcgtcttgttcacgtaaggcgacagggcgaccacgctagagacccccgagatgggcaggtagcgcgtgaggccgcccgcggggacggccccggaagtctccgcgtggcgcgtcttccgggcacacttcctcggcccccgcggcccagaagcagcgcgggggccgagggaggtttcctcttgtctccctcccagggcaccgacggccccgcccgaggaggcggaagcggaggaggacgcggccccggtggcggaagaggtggcccccgcgggagtcggggccgaggaggaagaggcggaggaggaagaggcggaggccgccgaggacgtcaggggggtcccgggccctccctggccgcgcccccccggccctgagtcggagggggggtgcgtcgccgccctcttggcccctgccggcgcgagggggggacgcgtggactggggggaggggttttcctggcccgacccgcgcctcttcctcggacgcaccgccgcctcctgctcgacagaggcggcggaggggagcgggggggcgccggagggggcggcgccggagggggcggcgccgcgggagggcccgtgtccaccctccacgcccggcccccccgagccgcgcgccaccgtcgcacgcgcccggcacagactctgttcttggttcgcggcctgagccagggacgagtgcgactggggcacacggcgcgcgtccgcggggcgggcggccggctccgccccgggggccggggcgcgggggccgggccccggaggcggcgcccgcacacacggggccacggccgcgcgggggcgcgcggggcccgacgcggccgcggacgcggggggaccggggcggggggcggagcctggcatgggcgccgcggggggcctgtggggagaggccgggggggagtcgctgatcactatggggtctctgttgtttgcaaggggggcgggtctgttgacaagggggcccgtccggcccctcggccgccccgcctccgcttcaacaaccccaacccccccggaggggccagacgccccccgcggcaccgcggctcgcgactggcgggagccgccgccgccgctgctgttggtggtggtgttagtgttactgctgccgtgtggcccgatgggcgccgaggggggcgctgtccgagccgcggccggctggggggctgcgtgagacgccccgcccgtcacggggggcgcggcggcgcctctgcgtgggggggcgcggggcgtccggcggggggcgggcggtacgtagtctgctgcaagagacaacggggggcgcgatcaggttacgccccctccccggcccgccctttcctcgcccgcccgcccgcctattcctccctcccccccccctcctcctcctcccccagggtcctcgccgcccccccgcctcaccgtcgtccaggtcgtcgtcatcctcgtccgtggtgggctcagggtgggtgggcgacagggccctcaccgtgtgcccccccagggtcaggtaccgcggggcgaaccgctgattgcccgtccagataaagtccacggccgtgcccgccctgacggcctcctcggcctccatgcgggtctgggggtcgttcacgatcgggatggtgctgaacgacccgctgggcgtcacgcccactatcaggtacaccagcttggcgttgcacagcgggcaggtgttgcgcaattgcatccaggttttcatgcacgggatgcagaagcggtgcatgcacgggaaggtgtcgcagcgcaggtggggcgcgatctcatccgtgcacacggcgcacacgtcgccctcgtcgctccccccgtcctctcgagggggggcgcccccgcaactgccggggtcttcctcgcggggggggctcccccccgagaccgcccccccatccacgccctgcggccccagcagccccgtctcgaacagttccgtgtccgtgctgtccgcctcggaggcggagtcgtcgtcatggtggtcggcgtccccccgcccccccacttcggtctccgcctccgagtcgctgctgtccggcaggtctcggtcgcagggaaacacccagacatccggggcgggctgaggggaaaaaagggggggcgggtaagaatggggggatttcccgcgtcaatcagcgcccacgagttccccctccccccccgcctcacaaagtcctgcccccctgctggcctcggaagaggggggagaaaggggtctgcaaccaaaggtggtctgggtccgtcctttggatcccgacccctcttcttccctcttctcccgccctccagacgcaccggagtcgggggtcccacggcgtcccccaaatatggcgggcggctcctccccacccccctagatgcgtgtgagtaagggggccctgcgtatgagtcagtggggaccacgccccctaacacggcgaccccggtccctgtgtgtttgttgtgggggcgtgtctctgtgtatgagtcaggggggtcccacggcgaccccgggccctgcgtctgagtcaaaggggccatgtgtaggtgttgggggtctgtatatataaagtcagggggtcacatggcgacccctaacagggcgaccccggtccctgtatatatagggtcagggggttccgcgccccctaacatggcgcccccggtccctgtatatatagtgtcacggggttccacgccccctaacatggcgccccaacatggcgcccggctcccgtgtatgagtgggggtcccccaacatggcggccggttccagtgtaagggtcgggggtcccccaacatggcgccccccaacatggcgccccccaacatggcgccccagacatggcgcccggcccctcacctcgcgctgggggcggccctcaggccggcgggtactcgctccggggcggggctccatgggggtcgtatgcggctggagggtcgctgacggagggtccctgggggtcgcaacgtaggcggggcttctgtggtgatgcggagagggggcggcccgagtctgcctggctgctgcgtctcgctccgagtgccgaggtgcaaatgcgaccagaccgtcgggccagggctaacttataccccacgcctttcccctccccaaaggggcggcagtgacgattcccccaatggccgcgcgtcccaggggaggcaggcccaccgcggggcggccccgtccccggggaccaacccggcgcccccaaagaatatcattagcatgcacggcccggcccccgatttgggggaccaacccggtgtcccccaaagaaccccattagcatgcccctcccgccgacgcaacaggggcttggcctgcgtcggtgccccggggcttcccgccttcccgaagaaactcattaccatacccggaaccccaggggaccaatgcgggttcattgagcgacccgcgggccaatgcgcgaggggccgtgtgttccgccaaaaaagcaattaacataacccggaaccccaggggagtggttacgcgcggcgcgggaggcggggaataccggggttgcccattaagggccgcgggaattgccggaagcgggaagggcggccggggccgcccattaatgagtttctaattaccataccgggaagcggaacaaggcctctgcaagtttttaattaccataccgggaagtgggcggcccggcccactgggcgggagttaccgcccagtgggccgggccccgacgactcggcggacgctggttggccgggccccgccgcgctggcggccgccgattggccagtcccgccctccgagggcgggcccgcctcgggggcgggccggctccaagcgtatatatgcgcggctcctgccatcgtctctccggagagcggcttggtgcggagctcccgggagctccgcggaagacccaggccgcctcgggtgtaacgttagaccgagttcgccgggccggctccgcgggccagggcccgggcacgggcctcgggccccaggcacggcccgatgaccgcctcggcctccgccacccggcgccggaaccgagcccggtcggcccgctcgcgggcccacgagccgcggcgcgccaggcgggcggccgaggcccagaccaccaggtggcgcacccggacgtggggcgagaagcgcacccgcgtgggggtcgcgggggtcgcgggggtcgcggggggcttcggcgccccctccccgcccgcgcgtcgcaggcgcaggcgcgccaggtgctctgcggtgacgcgcaggcggagggcgaggcgcggcggaaggcggaaggggcgtgagggggggtgggaggggttagccccgccccccgggcccgcgccgggcggtggggaccgggggcggggggcggcggcggtgggccgggcctctggcgccggctcgggcggggggctgtccggccagtcgtcgtcgtcgtcgtcggacgcggactcgggaacgtggagccactggcgcagcagcagcgaacaagaaggcgggggcccactggcggggggcggcggcggggcggccgcgggcgcgctcctgaccacgggttccgagttgggcgtggaggttacctgggactgtgcggttgggaccgcgcccgtgggcccgggcggccgggggcggcgggggccgcgatggcggcggcgggccatggagacagagagcgtgccggggtggtagagtttgacaggcaagcatgtgcgtgcagaggcgagtagtgcttgcctgtctaactcgctagtctcggccgcggggggcccgggctgcccgccgcccgcctttaaagggccgcgcgcgacccccggggggtgtgttttggggggggcccgtttccggggtctggccgctcctcccccgctcctccccccgctcctccccccgctcctccccccgctcctccccccgctcctccccccgctcctccccccgctcctccccccgctcctccccccgctcctccccccgctcctccccccgctcctccccccgctcctccccccgctcctccccccgctcctccccccgctcctccccccgctcctcccccgctcctcccccgctcccgcggccccgccccccacgcccgccgcgcgcgcgcacgccgcccggaccgccgcccgccttttttgcgcgcgcgcgcgcccgcggggggcccgggctgccacaggtaaaacaacaccaacaaagcacggcgcaatccgcacgtcacacgtcacgtcatccaccacacctgcccaacaacacaactcacagcgacaactcaccgcgcaacaactcctgttcctcatccacacgtcaccgcgcacctcccgctcctccagacgtaccccggcgcaacacaccgctcctgctacacaccaccgcccctccccagccccagccctccccagccccagccctccccggccccagccctccccggccccagccctccccggccccagccctccccggccccagccctccccggccccagccctccccagccccagccctccccagccgcgtcccgcgctccctcgggggggttcgggcatctctacctcagtgccgccaatctcaggtcagagatccaaaccctccgggggcgcccgcgcaccaccaccgcccctcgccccctcccgcccctcgccccctcccgcccctcgccccctcccgcccctcgccccctcccgcccctcgccccctcccgcccctcgccccctcccgcccctcgccccctcccgcccctcgccccctcccgcccctcgccccctcccgcccctcgccccctcccgcccctcgccccctcccgcccctcgccccctcccgcccctcgccccctcccgcccctcgccccctcccgcccctcgccccctcccgcccctcgccccctcccgcccctcgccccctcccgcccctcgccccctcccgcccctcgccccctcccgcccctcgaataaacaacgctactgcaaaacttaatcaggtcgttgccgtttattgcgtcttcgggtttcacaagcgccccgccccgtcccggcccgttacagcaccccgtccccctcgaacgcgccgccgtcgtcttcgtcccaggcgccttcccagtccacaacgtcccgtcgcgggggcgtggccaagcccgcctccgcccccagcacctccacggcccccgccgccgccagcacggtgccgctgcggcccgtggccgaggcccagcgaatcccgggcggcgccggcggcagggcccccgggccgtcgtcgtcgtcgccgcgcagcaccagcgggggggcgtcgtcgtcgggctccagcagggcgcgggcgcaaaagtccctccgcggcccgcgccaccgggccgggccggcgcgcaccgcctcgcgccccagcgccacgtacacgggccgcagcggcgcgcccaggccccagcgcgcgcaggcgcggtgcgagtgggcctcctcctcgcagaagtccggcgcgccgggcgccatggcgtcggtggtccccgaggccgccgcccggccgtccagcgccggcagcacggcccggcggtactcgcgcggggacatgggcaccggcgtgtccgggccgaagcgcgtgcgcacgcggtagcgcacgttgccgccgcggcacaggcgcagcggcggcgcgtcggggtacaggcgcgcgtgcgcggcctccacgcgcgcgaagacccccgggccgaacacgcggcccgaggccagcaccgtgcggcgcaggtcccgcgccgccggccagcgcacggcgcactgcacggcgggcagcaggtcgcacgccaggtaggcgtgctgccgcgacaccgcgggcccgtcggcgggccagtcgcaggcgcgcacggtgttgaccacgatgagccgccggtcgccggcgctggcgagcagccccagaaactccacggccccggcgaaggccaggtcccgcgtggacagcagcagcacgccctgcgcgcccagcgccgacacgtcgggggcgccggtccagttgcccgcccaggcggccgtgtccggcccgcacagccggttggccagggccgccagcaggcaggacagcccgccgcgctcggcggaccactccggcggcccccccgaggccccgccgccggccaggtcctcgcccggcagcggcgagtacagcaccaccacgcgcacgtcctcggggtcggggatctggcgcatccaggccgccatgcggcgcagcgggcccgaggcgcgcagggggccaaagaggcggcccccggcggccccgtgggggtgggggttctcgtcgtcgtcgccgccgcacgcggcctgggcggcgggggcgggcccggcgcaccgcgcggcgatcgaggccagggcccgcgggtcaaacatgagggccggtcgccaggggacggggaacagcgggtggtccgtgagctcggccacggcgcgcggggagcagtaggcctccagggcggcggccgcgggcgccgccgtgtggctgggcccccggggctgccgccgccagccgcccagggggtcggggccctcggcgggccggcgcgacagcgccacggggcgcgggcgggcctgcgccgcggcgccccgggccgccgcgggctgggcgggggtgggctcgggccccgggggcgtggaggggggcgcggggaggggggcgcgggcgtccgagccgggggcgtccgcgccgctcttcttcgtcttcgggggtcgcgggccgccgcctccgggcggccgggccgggccgggactcttgcgcttgcgcccctcccgcggcgcggcggaggcggcggcggccgccagcgcgtcggcggcgtccggtgcgctggccgccgccgccagcagggggcggaggctctggttctcaaacagcaggtccgcggcggcggcggccgcggagctcggcaggcgcgggtcccgcggcagcgcggggcccagggccccggcgaccaggctcacggcgcgcacggcggccacggcggcctcgctgccgccggccacgcgcaggtccccgcgcaggcgcatgagcaccagcgcgtcgcgcacgaaccgcagctcgcgcagccacgcgcgcaggcggggcgcgtcggcgtgcggcggcggcggggaagcggggcccgcgggtccctccggccgcggggggctggcgggccgggccccggccagccccgggacggccgccaggtcgccgtcgaagccctcggccagcgcctccaggatcccgcggcaggcggccaggcactcgacggccacgcggccggcctgggcgcggcgcccggcgtcggcgtcggcgtggcgggcggcgtcggggtcgtcgccccccacgggggaggcgggcgcggcggacagccgccccagggcggcgaggatccccgcggcgccgtacccggcgggcaccgcgcgctcgcccggtgcggcggcggcgacggcggcgaccccctcgtcatctgcgccggcgccggggctccccgcggcccccgtcagcgccgcgttctcgcgcgccaacaggggcgcgtaggcgcggcgcaggctggtcagcaggaagcccttctgcgcgcggtcgtatcggcggctcatggccacggcggccgccgcgtgcgccaggccccagccgaagcggccggccgccatggcgtagcccaggtggggcacggcccgcgccacgctgccggtgatgaaggagctgctgttgcgcgcggcgcccgagatccggaagcaggcctggtccagcgccacgtccccggggaccacgcgcgggttctggagccaccccatggcctccgcgtccggggtgtacagcagccgcgtgatcagggcgtactgctgcgcggcgtcgcccagctcgggcgcccacacggccgccggggcgcccgaggcctcgaaccggcgtcgcgcctcctccgcctcgggcgccccccagaggcccgggcggctgtcgcccaggccgccgtacagcacccgccccgggggcgggggcccggcgccgggccacggctccccgctgacgtacccgtcgcgatagcgcgcgtagaaggcgccggaggccgcgtcggcgtccagctcgacccgccggggctgcccggccgtgaagcggcccgtggcgtcgcggccggccaccgccgcgcgggcccggcggcgctcgatgcggcccgcggaggccgcgggggtcctcgccgccgcccggggcttgggcgcggcctcggagagggggggtggcccgggcgggggcggcgtccgcccgggggcttccggcgccgcgctcgacggaccccgcccgacggcccgcgcctcgcgtgcgtggtcggccgcgtcgttgccgtcgtcgtcctcgtcctcgtcggacgacgaggacgaagaggatgcggacgacgaggacgaggacccggagtccgacgaggtcgatgacgccgatggccgccgccggccgtgacgacgtctccgcggcggctgggccggcgggcgcggcgacaggcggtccgtggggtccggatacgcgccgcgtagcggggcctcccgttcgcggccccgggccggggcccggtcgccggcggcgtcggctgcgtcgtcgtactcgtccccgtcatcgtcgtcggctagaaaggcgggggtccggggcggcgaggccgcggggtcgggcgtcgggatcgtccggacggcctcctctaccatggaggccagcagagccagctgtcgcgacgagacggcgtccccggcgtcctcgccggcgtcggtgcccgccgcgggggccctcccgtcccgccgggcgtcgtcgaggtcgtgggggtggtcggggtcgtggtcggggtcgtccccgccctcctccgtctccgcgccccacccgagggccccccgctcgtcgcggtctgggctcggggtgggcggcggcccgtcggtggggcccggggagccggggcgctgcttgttctccgacgccatcgccgatgcggggcgatcctccggggatacggctgcgacggcggacgtagcacggtaggtcacctacggactctcgatggggggagggggcgagacccacggaccccgacgacccccgccgtcgacgcggaactagcgcggaccggtcgatgcttgggtggggaaaaaggacagggacggccgatccccctcccgcgcttcgtccgcgtatcggcgtcccggcgcggcgagcgtctgacggtctgtctctggcggtcccgcgtcgggtcgtggatccgtgtcggcagccgcgctccgtgtggacgatcggggcgtcctcgggctcatatagtcccaggggccggcgggaaggaggagcagcggaggccgccggccccccgccccccggcgggcccaccccgaacggaattccattatgcacgaccccgccccgacgccggcacgccgggggcccgtggccgcggcccgttggtcgaacccccggccccgcccatccgcgccatctgccatggacggggcgcgagggcgggtgggtccgcgccccgccccgcatggcatctcattaccgcccgatccggcggtttccgcttccgttccgcatgctaacgaggaacgggcagggggcggggcccgggccccgacttcccggttcggcggtaatgagatacgagccccgcgcgcccgttggccgtccccgggcccccggtcccgcccgccggacgccgggaccaacgggacggcgggcggcccttgggccgcccgccttgccgcccccccattggccggcgggcgggaccgccccaagggggcggggccgccgggtaaaagaagtgagaacgcgaagcgttcgcacttcgtcccaatatatatatattattagggcgaagtgcgagcactggcgccgtgcccgactccgcgccggccccgggggcggacccgggcggcggggggcgggtctctccggcgcacataaaggcccggcgcgaccgacgcccgcagacggcgccagccacgaacgacgggagcggctgcggagcacgcggaccgggagcgggagtcgcagagggccgtcggagcggacggcgtcggcatcgcgacgccccggctcgggatcgggatcgcatcggaaagggacacgcggacgcgggggggaaagacccgcccaccccacccacgaaacacaggggacgcaccccgggggcctccgacgacagaaacccaccggtccgccttttttgcacgggtaagcaccttgggtgggcagaggaggggggacgcgggggcggaggaggggggacgcgggggcggaggaggggggacgcgggggcggaggaggggggacgcgggggcggaggaggggggacgcgggggcggaggagggggctcacccgcgttcgtgccttcccgcaggaggaacgccctcgtcgaggcgaccggcggcgaccgttgcgtggaccgcttcctgctcgtcgggggggggggagccactgtggtcctccgggacgttttctggatggccgacatttccccaggcgcttttgtgccttgtgtaaaagcgcggcgtcccgctctccgatccccgcccctgggcacgcgcaagcgcaagcgccctgcccgccccctctcatcggagtctgaggtcgaatccgagacagccttggagtctgaggtcgaatccgagacagcatcggattcgaccgagtctggggaccaggaggaagccccccgcatcggtggccgtagggccccccggaggcttggggggcggttttttctggacatgtcggcggaatccaccacggggacggaaacggatgcgtcggtgtcggacgaccccgacgacacgtccgactggtcttgtgacgacattcccccacgacccaagcgggcccgggtaaacctgcggctcactagctctcccgatcggcgggatggggttatttttcctaagatggggcgggtccggtctacccgggaaacgcagccccgggcccccaccccgtcggccccaagcccaaatgcaatgctccggcgctcggtgcgccaggcccagaggcggagcagcgcacgatggacccccgacctgggctacatgcgccagtgtatcaatcagctgtttcgggtcctgcgggtcgcccgggacccccacggcagtgccaaccgcctgcgccacctgatacgcgactgttacctgatgggatactgccgagcccgtctggccccgcgcacgtggtgccgcttgctgcaggtgtccggcggaacctggggcatgcacctgcgcaacaccatacgggaggtggaggctcgattcgacgccaccgcagaacccgtgtgcaagcttccttgtttggaggccagacggtacggcccggagtgtgatcttagtaatctcgagattcatctcagcgcgacaagcgatgatgaaatctccgatgccaccgatctggaggccgccggttcggaccacacgctcgcgtcccagtccgacacggaggatgccccctcccccgttacgctggaaaccccagaaccccgcgggtccctcgctgtgcgtctggaggatgagtttggggagtttgactggaccccccaggagggctcccagccctggctgtctgcggtcgtggccgataccagctccgtggaacgcccgggcccatccgattctggggcgggtcgcgcagcagaagaccgcaagtgtctggacggctgccggaaaatgcgcttctccaccgcctgcccctatccgtgcagcgacacgtttctccggccgtgagtccggtcgccccgacccccttgtatgtccccaaaataaaagaccaaaatcaaagcgtttgtcccagcgtcttaatggcgggaagggcggagagaaacagaccacgcgtacatggggggtgtttgggggtttattgacatcggggctacagggtggtaaccggatagcagatgtgaggaagtctgggccgttcgccgcgaacggcgatcagagggtccgtttcttgcggaccacggcccggtgatgtgggttgctcgtctaaaatctcgggcatacccatacacgcacaacacggacgccgcaccgaatgggacgtcgtaagggggtgggaggtagctgggtggggtttgtgcagagcaatcagggaccgcagccagcgcatacaatcgcgctcccgtccgttggtcccgggcaggaccacgccgtactggtattcgtaccggctgagcagggtctccagggggtggttgggtgccgcggggaacggggtccacgccacggtccactcgggcaaaaaccgagtcggcacggcccacggttctcccacccacgcgtctggggtcttgatggcgataaatcttaccccgagccggattttttgggcgtattcgagaaacggcacacacagatccgccgcgcctaccacccacaagtggtagaggcgaggggggctgggttggtctcggtgcaacagtcggaagcacgccacggcgtccacgacctcggtgctctccaaggggctgtcctccgcaaacaggcccgtggtggtgtttggggggcagcgacaggacctagtgcgcacgatcgggcgggtgggtttgggtaagtccatcagcggctcggccaaccgtcgaaggttggccgggcgaacgacgaccggggtacccaggggttctgatgccaaaatgcggcactgcctaagcaggaagctccacagggccgggcttgcgtcgacggaagtccggggcagggcgttgttctggtcaaggagggtcattacgttgacgacaacaacgcccatgttggtatattacaggcccgtgtccggtttggggcacttgcagatttgtaaggccacgcacggcggggagacaggccgacgcgggggctgctctaaaaatttaagggccctacggtccacagacccgccttcccgggggggcccttggagcgaccggcagcggaggcgtccgggggaggggagggttatttacgggggggtaggtcagggggtgggtcgtcaaactgccgctccttaaaaccccggggcccgtcgttcggggtgctcgttggttggcactcacggtgcggcgaatggcctgtcgtaagttttgtcgcgtttacgggggacagggcaggaggaaggaggaggccgtcccgccggagacaaagccgtcccgggtgtttcctcatggccccttttataccccagccgaggacgcgtgcctggactccccgcccccggagacccccaaaccttcccacaccacaccacccggcgatgccgagcgcctgtgtcatctgcaggagatcctggcccagatgtacggaaaccaggactaccccatagaggacgaccccagcgcggatgccgcggacgatgtcgacgaggacgccccggacgacgtggcctatccggaggaatacgcagaggagctttttctgcccggggacgcgaccggtccccttatcggggccaacgaccacatccctcccccgcgtggcgcatctccccccggtatacgacgacgcagccgggatgagattggggccacgggatttaccgcagaagagctggacgccatggacaggcaggcggctcgagccatcagccgcggcggcaagcccccctcgaccatggccaagctggtgactggcatgggctttacgatccacggagcgctcaccccaggatcggaggggtgtgtctttgacagcagccacccagattacccccaacgggtaatcgtgaaggcggggtggtacacgagcacgagccacgaggcgcgactgctgaggcgactggaccacccggcgatcctgcccctcctggacctgcatgtcgtctccggggtcacgtgtctggtcctccccaagtaccaggccgacctgtatacctatctgagtaggcgcctgaacccactgggacgcccgcagatcgcagcggtctcccggcagctcctaagcgccgttgactacattcaccgccagggcattatccaccgcgacattaagaccgaaaatatttttattaacacccccgaggacatttgcctgggggactttggtgccgcgtgcttcgtgcagggttcccgatcaagccccttcccctacggaatcgccggaaccatcgacaccaacgcccccgaggtcctggccggggatccgtataccacgaccgtcgacatttggagcgccggtctggtgatcttcgagactgccgtccacaacgcgtccttgttctcggccccccgcggccccaaaaggggcccgtgcgacagtcagatcacccgcatcatccgacaggcccaggtccacgttgacgagttttccccgcatccagaatcgcgcctcacctcgcgctaccgctcccgcgcggccgggaacaatcgcccgccttacacccgaccggcctggacccgctactacaagatggacatagacgtcgaatatctggtttgcaaagccctcaccttcgacggcgcgcttcgccccagcgccgcagagctgctttgtttgccgctgtttcaacagaaatgaccgcccccggggggcggtgctgtttgcgggttggcacaaaaagaccccgacccgcgtctgtggtgtttttggcatcatgtcgccgggcgccatgcgtgccgttgttcccattatcccattccttttggttcttgtcggtgtatcgggggttcccaccaacgtctcctccaccacccaaccccaactccagaccaccggtcgtccctcgcatgaagcccccaacatgacccagaccggcaccaccgactctcccaccgccatcagccttaccacgcccgaccacacaccccccatgccaagtatcggactggaggaggaggaggaagaggaggagggggccggggatggcgaacatcttaaggggggagatgggacccgtgacaccctaccccagtccccgggtccagccgtcccgttggccggggatgacgagaaggacaaacccaaccgtcccgtagtcccaccccccggtcccaacaactcccccgcgcgccccgagaccagtcgaccgaagacaccccccaccagtatcgggccgctggcaactcgacccacgacccaactcccctcaaaggggcgacccttggttccgacgcctcaacataccccgctgttctcgttcctcactgcctcccccgccctggacaccctcttcgtcgtcagcaccgtcatccacaccttatcgtttgtgtgtattgttgctatggcgacacacctgtgtggtggttggtccagacgcgggcgacgcacacaccctagcgtgcgttacgtgtgcctgccgcccgaacgcgggtagggtatggggcggggatggggagagcccacacgcggaaagcaagaacaataaaggcggcgggatctagttgatatgcgtctctgggtgtttttggggtgtggtgggcgcggggcggtcattggacgggggtgcagttaaatacatgcccgggacccatgaagcatgcgcgacttccgggcctcggaacccacccgaaacggccaacggacgtctgagccaggcctggctatccggagaaacagcacacgacttggcgttctgtgtgtcgcgatgtctctgcgcgcagtctggcatctggggcttttgggaagcctcgtgggggctgttcttgccgccacccatctgggacctgcggccaacacaacggaccccttaacgcacgccccagtgtcccctcaccccagccccctggggggctttgccgtccccctcgtagtcggtgggctgtgtgccgtagtcctgggggcggcgtgtctgcttgagctcctgcgtcgtacgtgccgcgggtgggggcgttaccatccctacatggacccagttgtcgtataattttttcccccccccccttctccgcatgggtgatgtcgggtccaaactcccgacaccaccagctggcatggtataaatcaccggtgcgccccccaaaccatgtccggcagggggatggggggcgaatgcggagggcacccaacaacaccgggctaaccaggaaatccgtggccccggcccccaacaaagatcgcggtagcccggccgtgtgacattatcgtccataccgaccacaccgacgaatcccctaagggggaggggccattttacgaggaggaggggtataacaaagtctgtctttaaaaagcaggggttagggagttgttcggtcataagcttcagtgcgaacgaccaactaccccgatcatcagttatccttaaggtctcttttgtgtggtgcgttccggtatggggggggctgccgccaggttgggggccgtgattttgtttgtcgtcatagtgggcctccatggggtccgcggcaaatatgccttggcggatgcctctctcaagatggccgaccccaatcgctttcgcggcaaagaccttccggtcctggaccagctgaccgaccctccgggggtccggcgcgtgtaccacatccaggcgggcctaccggacccgttccagccccccagcctcccgatcacggtttactacgccgtgttggagcgcgcctgccgcagcgtgctcctaaacgcaccgtcggaggccccccagattgtccgcggggcctccgaagacgtccggaaacaaccctacaacctgaccatcgcttggtttcggatgggaggcaactgtgctatccccatcacggtcatggagtacaccgaatgctcctacaacaagtctctgggggcctgtcccatccgaacgcagccccgctggaactactatgacagcttcagcgccgtcagcgaggataacctggggttcctgatgcacgcccccgcgtttgagaccgccggcacgtacctgcggctcgtgaagataaacgactggacggagattacacagtttatcctggagcaccgagccaagggctcctgtaagtacgccctcccgctgcgcatccccccgtcagcctgcctctccccccaggcctaccagcagggggtgacggtggacagcatcgggatgctgccccgcttcatccccgagaaccagcgcaccgtcgccgtatacagcttgaagatcgccgggtggcacgggcccaaggccccatacacgagcaccctgctgcccccggagctgtccgagacccccaacgccacgcagccagaactcgccccggaagaccccgaggattcggccctcttggaggaccccgtggggacggtggcgccgcaaatcccaccaaactggcacatcccgtcgatccaggacgccgcgacgccttaccatcccccggccaccccgaacaacatgggcctgatcgccggcgcggtgggcggcagtctcctggcagccctggtcatttgcggaattgtgtactggatgcaccgccgcactcggaaagccccaaagcgcatacgcctcccccacatccgggaagacgaccagccgtcctcgcaccagcccttgttttactagatacccccccttaatgggtgcgggggggtcaggtctgcggggttgggatgggaccttaactccatataaagcgagtctggaaggggggaaaggcggacagtcgataagtcggtagcgggggacgcgcacctgttccgcctgtcgcacccacagctttttcgcgaaccgtcccgtttcgggatgccgtgccgcccgttgcagggcctggtgctcgtgggcctctgggtctgtgccaccagcctggttgtccgtggccccacggtcagtctggtatcaaactcatttgtggacgccggggccttggggcccgacggcgtagtggaggaagacctgcttattctcggggagcttcgctttgtgggggaccaggtcccccacaccacctactacgatggggtcgtagagctgtggcactaccccatgggacacaaatgcccacgggtcgtgcatgtcgtcacggtgaccgcgtgcccacgtcgccccgccgtggcatttgccctgtgtcgcgcgaccgacagcactcacagccccgcatatcccaccctggagctgaatctggcccaacagccgcttttgcgggtccggagggcgacgcgtgactatgccggggtgtacgtgttacgcgtatgggtcggggacgcaccaaacgccagcctgtttgtcctggggatggccatagccgccgaaggtactctggcgtacaacggctcggcccatggctcctgcgacccgaaactgcttccgtcttcggccccgcgtctggccccggcgagcgtataccaacccgcccctaacccggcctccaccccctcgaccaccacctccaccccctcgaccaccatccccgctccccaagcatcgaccacacccttccccacgggagacccaaaaccccaacctcacggggtcaaccacgaacccccatcgaatgccacgcgagcgacccgcgactcgcgatatgcgctaacggtgacccagataatccagatagccatccccgcgtccattatagccctggtgtttctggggagctgtatttgctttatacacagatgtcaacgccgctaccgacgctcccgccgcccgatttacagcccccagatacccacgggcatctcatgcgcggtgaacgaagcggccatggcccgcctcggagccgagctcaaatcgcatccgagcaccccccccaaatcccggcgccggtcgtcacgcacgccaatgccctccctgacggccatcgccgaagagtcggagcccgcgggggcggctgggcttccgacgccccccgtggaccccacgacatccaccccaacgcctcccctgttggtataggtccacggccactggccgggggcaccacataaccgaccgcagtcactgagttgggaataaaccggtattatttacctatatccgtgtatgtccatttctttcttcccccccccccccggaaaccaaagaaggaagcaaagaatggatgggaggagttcaggaagccggggagagggcccgcggcgcatttaaggcgttgttgtgttgactttggctcttctggcgggttggtgcggtgctgtttgttgggctcccattttacccgaagatcggctgctatccccgggacatggatcgcggggcggtggtggggtttcttctcggtgtttgtgttgtatcgtgcttggcgggaacgcccaaaacgtcctggagacgggtgagtgtcggcgaggacgtttcgttgcttccagctccggggcctacggggcgcggcccgacccagaaactactatgggccgtggaacccctggatgggtgcggccccttacacccgtcgtgggtctcgctgatgccccccaagcaggtgcccgagacggtcgtggatgcggcgtgcatgcgcgctccggtcccgctggcgatggcgtacgcccccccggccccatctgcgaccgggggtctacgaacggacttcgtgtggcaggagcgcgcggccgtggttaaccggagtctggttattcacggggtccgagagacggacagcggcctgtataccctgtccgtgggcgacataaaggacccggctcgccaagtggcctcggtggtcctggtggtgcaaccggccccagttccgaccccacccccgaccccagccgattacgacgaggatgacaatgacgagggcgaggacgaaagtctcgccggcactcccgccagcgggaccccccggctcccgcctccccccgcccccccgaggtcttggcccagcgcccccgaagtctcacatgtgcgtggggtgaccgtgcgtatggagactccggaagctatcctgttttcccccggggagacgttcagcacgaacgtctccatccatgccatcgcccacgacgaccagacctactccatggacgtcgtctggttgaggttcgacgtgccgacctcgtgtgccgagatgcgaatatacgaatcgtgtctgtatcacccgcagctcccagaatgtctgtccccggccgacgcgccgtgcgccgcgagtacgtggacgtctcgcctggccgtccgcagctacgcggggtgttccagaacaaaccccccaccgcgctgttcggccgaggctcacatggagcccgtcccggggctggcgtggcaggcggcctccgtcaatctggagttccgggacgcgtccccacaacactccggcctgtatctgtgtgtggtgtacgtcaacgaccatattcacgcctggggccacattaccatcagcaccgcggcgcagtaccggaacgcggtggtggaacagcccctcccacagcgcggcgcggatttggccgagcccacccacccgcacgtcggggcccctccccacgcgcccccaacccacggcgccctgcggttaggggcggtgatgggggccgccctgctgctgtctgcgctggggttgtcggtgtgggcgtgtatgacctgttggcgcaggcgtgcctggcgggcggttaaaagcagggcctcgggtaaggggcccacgtacattcgcgtggccgacagcgagctgtacgcggactggagctcggacagcgagggagaacgcgaccaggtcccgtggctggcccccccggagagacccgactctccctccaccaatggatccggctttgagatcttatcaccaacggctccgtctgtatacccccgtagcgacgggcatcaatctcgccgccagctcacaacctttggatccggaaggcccgatcgccgttactcccaggcctccgattcgtccgtcttctggtaaggcgccccatcccgaggccccacgtcggtcgccgaactgggcgaccgccggcgaggtggacgtcggagacgagctaatcgcgatttccgacgaacgcggacccccccgacatgaccgcccgcccctcgccacgtcgaccgcgccctcgccacacccgcgacccccgggctacacggccgttgtctccccgatggccctccaggctgtcgacgccccctccctgtttgtcgcctggctggccgctcggtggctccggggggcttccggcctgggggccgtcctgtgtgggattgcgtggtatgtgacgtcaattgcccgaggcgcacaaagggccggtggtccgcctagccgcagcaaattaaaaatcgtgagtcacagcgaccgcaacttcccacccggagctttcttccggcctcgatgacgtcccggctctccgatcccaactcctcagcgcgatccgacatgtccgtgccgctttatcccacggcctcgccagtttcggtcgaagcctactactcggaaagcgaagacgaggcggccaacgacttcctcgtacgcatgggccgccaacagtcggtattaaggcgttgacgcagacgcacccgctgcgtcggcatggtgatcgcctgtctcctcgtggccgttctgtcgggcggatttggggcgctcctgatgtggctgctccgctaaaagaccgcatcgacacgcgcgtccttcttgtcgtctctcttcccccccatcaccccgcaatttgcacccagcctttaactacattaaattgggttcgattggcaatgttgtctcccggttgatttttgggtgggtggggagtgggtgggtggggagtgggtgggtggggagtgggtgggtggggagtgggtgggtggggagtgggtgggtggggagtgggtgggtggggagtgggtgggtggggagtgggtgggtggggagtgggtgggtggggagtggcaaggaagaaacaagcccgaccaccagacagaaaatgtaaccatacccaaaccgactctgggggctgtttgtggggtcggaaccataggatgaacaaaccaccccgtacctcccgcacccaagggtgcgggtggctcatcggcatctgtccggtatgggttgttccccacccactcgcgttcggacgtcttagaatcatggcggttttctatgccgacatcggttttctcccccgcaataagacacgatgcgataaaatctgtttgtaaaatttattaagggtacaaattgccctagcacaggggtggggttagggccgggtccccacacccaaacgcaccaaacagatgcaggcagtgggtcgagtacagccccgcgtacgaacacgtcgatgcgtgtgtcagacagcaccagaaagcacaggccatcaacaggtcgtgcatgtgtcggtgggtttggacgcggggggccatggtggtgataaagttaatggccgccgtccgccagggccacaggggcgacgtctcttggttggcccggagccactgggtgtggaccagccgcgcgtggcggcccaacatggcccctgtagccgggggcgggggatcgcgcacgtttgcagcgcacatgcgagacacctcgaccacggttcgaaagaaggcccggtggtccgcgggcaacatcaccaggtgcgcaagcgcccgggcgtccagagggtagagccctgagtcatccgaggttggctcatcgcccgggtcttgccgcaagtgcgtgtgggttgggcttccggtgggcgggacgcgaaccgcggtgtggatcccgacgcgggcccgagcgtatgctccatcttgtggggagaaggggtctgggctcgccaggggggcatacttgcccgggctatacagacccgcgagccgtacgtggttcgcggggggtgcgtggggtccggggctccctgggagaccggggttgtcgtggatccctggggtcacgcggtaccctggggtctctgggagctcgcggtactctgggttccctaggttctcggggtggtcgcggaacccggggctcccggggaacacgcggtgtcctggggattgttggcggtcggacggcttcagatggcttcgagatcgtagtgtccgcaccgactcgtagtagacccgaatctccacattgccccgccgcttgatcattatcaccccgttgcgggggtccggagatcatgcgcgggtgtcctcgaggtgcgtgaacacctctggggtgcatgccggcggacggcacgccttttaagtaaacatctgggtcgcccggcccaactggggccgggggttgggtctggctcatctcgagagacacgggggggaaccaccctccgcccagagactcgggtgatggtcgtacccgggactcaacgggttaccggattacggggactgtcggtcacggtcccgccggttcttcgatgtgccacacccaaggatgcgttgggggcgatttcgggcagcagcccgggagagcgcagcaggggacgctccgggtcgtgcacggcggttctggccgcctcccggtcctcacgcccccttttattgatctcatcgcgtacgtcggcgtacgtcctgggcccaacccgcatgttgtccaggaaggtgtccgccatttccagggcccacgacatgcttttccccccgacgagcaggaagcggtccacgcaacggtcgccgccggtcgcctcgacgagggcgttcctcctgcgggaaggcacgaacgcgggtgagccccctcctccgcccccgcgtcccccctcctccgcccccgcgtcccccctcctccgcccccgcgtcccccctcctccgcccccgcgtcccccctcctccgcccccgcgtcccccctcctctgcccacccaaggtgcttacccgtgcaaaaaaggcggaccggtgggtttctgtcgtcggaggcccccggggtgcgtcccctgtgtttcgtgggtggggtgggcgggtctttcccccccgcgtccgcgtgtccctttccgatgcgatcccgatcccgagccggggcgtcgcgatgccgacgccgtccgctccgacggccctctgcgactcccgctcccggtccgcgtgctccgcagccgctcccgtcgttcgtggctggcgccgtctgcgggcgtcggtcgcgccgggcctttatgtgcgccggagagacccgccccccgccgcccgggtccgcccccggggccggcgcggagtcgggcacggcgccagtgctcgcacttcgccctaataatatatatatattgggacgaagtgcgaacgcttcgcgttctcacttcttttacccggcggccccgcccccttggggcggtcccgcccgccggccaatgggggggcggcaaggcgggcggcccaagggccgcccgccgtcccgttggtcccggcgtccggcgggcgggaccgggggcccggggacggccaacgggcgcgcggggctcgtatctcattaccgccgaaccgggaagtcggggcccgggccccgccccctgcccgttcctcgttagcatgcggaacggaagcggaaaccgccggatcgggcggtaatgagatgccatgcggggcggggcgcggacccacccgccctcgcgccccgtccatggcagatggcgcggatgggcggggccgggggttcgaccaacgggccgcggccacgggcccccggcgtgccggcgtcggggcggggtcgtgcataatggaattccgttcggggtgggcccgccggggggcggggggccggcggcctccgctgctcctccttcccgccggcccctgggactatatgagcccgaggacgccccgatcgtccacacggagcgcggctgccgacacggatccacgacccgacgcgggaccgccagagacagaccgtcagacgctcgccgcgccgggacgccgatacgcggacgaagcgcgggagggggatcggccgtccctgtcctttttccccacccaagcatcgaccggtccgcgctagttccgcgtcgacggcgggggtcgtcggggtccgtgggtctcgccccctccccccatcgagagtccgtaggtgacctaccgtgctacgtccgccgtcgcagccgtatccccggaggatcgccccgcatcggcgatggcgtcggagaacaagcagcgccccggctccccgggccccaccgacgggccgccgcccaccccgagcccagaccgcgacgagcggggggccctcgggtggggcgcggagacggaggagggcggggacgaccccgaccacgaccccgaccacccccacgacctcgacgacgcccggcgggacgggagggcccccgcggcgggcaccgacgccggcgaggacgccggggacgccgtctcgtcgcgacagctggctctgctggcctccatggtagaggaggccgtccggacgatcccgacgcccgaccccgcggcctcgccgccccggacccccgcctttctagccgacgacgatgacggggacgagtacgacgacgcagccgacgccgccggcgaccgggccccggcccggggccgcgaacgggaggccccgctacgcggcgcgtatccggaccccacggaccgcctgtcgccgcgcccgccggcccagccgccgcggagacgtcgtcacggccggcggcggccatcggcgtcatcgacctcgtcggactccgggtcctcgtcctcgtcgtccgcatcctcttcgtcctcgtcgtccgacgaggacgaggacgacgacggcaacgacgcggccgaccacgcacgcgaggcgcgggccgtcgggcggggtccgtcgagcgcggcgccggaagcccccgggcggacgccgcccccgcccgggccaccccccctctccgaggccgcgcccaagccccgggcggcggcgaggacccccgcggcctccgcgggccgcatcgagcgccgccgggcccgcgcggcggtggccggccgcgacgccacgggccgcttcacggccgggcagccccggcgggtcgagctggacgccgacgcggcctccggcgccttctacgcgcgctatcgcgacgggtacgtcagcggggagccgtggcccggcgccgggcccccgcccccggggcgggtgctgtacggcggcctgggcgacagccgcccgggcctctggggggcgcccgaggcggaggaggcgcgacgccggttcgaggcctcgggcgccccggcggccgtgtgggcgcccgagctgggcgacgccgcgcagcagtacgccctgatcacgcggctgctgtacaccccggacgcggaggccatggggtggctccagaacccgcgcgtggtccccggggacgtggcgctggaccaggcctgcttccggatctcgggcgccgcgcgcaacagcagctccttcatcaccggcagcgtggcgcgggccgtgccccacctgggctacgccatggcggccggccgcttcggctggggcctggcgcacgcggcggccgccgtggccatgagccgccgatacgaccgcgcgcagaagggcttcctgctgaccagcctgcgccgcgcctacgcgcccctgttggcgcgcgagaacgcggcgctgacgggggccgcggggagccccggcgccggcgcagatgacgagggggtcgccgccgtcgccgccgccgcaccgggcgagcgcgcggtgcccgccgggtacggcgccgcggggatcctcgccgccctggggcggctgtccgccgcgcccgcctcccccgtggggggcgacgaccccgacgccgcccgccacgccgacgccgacgccgggcgccgcgcccaggccggccgcgtggccgtcgagtgcctggccgcctgccgcgggatcctggaggcgctggccgagggcttcgacggcgacctggcggccgtcccggggctggccggggcccggcccgccagccccccgcggccggagggacccgcgggccccgcttccccgccgccgccgcacgccgacgcgccccgcctgcgcgcgtggctgcgcgagctgcggttcgtgcgcgacgcgctggtgctcatgcgcctgcgcggggacctgcgcgtggccggcggcagcgaggccgccgtggccgccgtgcgcgccgtgagcctggtcgccggggccctgggccccgcgctgccgcgggacccgcgcctgccgagctccgcggccgccgccgccgcggacctgctgtttgagaaccagagcctccgccccctgctggcggcggcggccagcgcaccggacgccgccgacgcgctggcggccgccgccgcctccgccgcgccgcgggaggggcgcaagcgcaagagtcccggcccggcccggccgcccggaggcggcggcccgcgacccccgaagacgaagaagagcggcgcggacgcccccggctcggacgcccgcgcccccctccccgcgcccccctccacgcccccggggcccgagcccacccccgcccagcccgcggcggcccggggcgccgcggcgcaggcccgcccgcgccccgtggcgctgtcgcgccggcccgccgagggccccgaccccctgggcggctggcggcggcagccccgggggcccagccacacggcggcgcccgcggccgccgccctggaggcctactgctccccgcgcgccgtggccgagctcacggaccacccgctgttccccgtcccctggcgaccggccctcatgtttgacccgcgggccctggcctcgatcgccgcgcggtgcgccgggcccgcccccgccgcccaggccgcgtgcggcggcgacgacgacgagaacccccacccccacggggccgccgggggccgcctctttggccccctgcgcgcctcgggcccgctgcgccgcatggcggcctggatgcgccagatccccgaccccgaggacgtgcgcgtggtggtgctgtactcgccgctgccgggcgaggacctggccggcggcggggcctcgggggggccgccggagtggtccgccgagcgcggcgggctgtcctgcctgctggcggccctggccaaccggctgtgcgggccggacacggccgcctgggcgggcaactggaccggcgcccccgacgtgtcggcgctgggcgcgcagggcgtgctgctgctgtccacgcgggacctggccttcgccggggccgtggagtttctggggctgctcgccagcgccggcgaccggcggctcatcgtggtcaacaccgtgcgcgcctgcgactggcccgccgacgggcccgcggtgtcgcggcagcacgcctacctggcgtgcgacctgctgcccgccgtgcagtgcgccgtgcgctggccggcggcgcgggacctgcgccgcacggtgctggcctcgggccgcgtgttcggcccgggggtcttcgcgcgcgtggaggccgcgcacgcgcgcctgtaccccgacgcgccgccgctgcgcctgtgccgcggcggcaacgtgcgctaccgcgtgcgcacgcgcttcggcccggacacgccggtgcccatgtccccgcgcgagtaccgccgggccgtgctgccggcgctggacggccgggcggcggcctcggggaccaccgacgccatggcgcccggcgcgccggacttctgcgaggaggaggcccactcgcaccgcgcctgcgcgcgctggggcctgggcgcgccgctgcggcccgtgtacgtggcgctggggcgcgaggcggtgcgcgccggcccggcccggtggcgcgggccgcggagggacttttgcgcccgcgccctgctggagcccgacgacgacgcccccccgctggtgctgcgcggcgacgacgacgacggcccgggggccctgccgccggcgccgcccgggattcgctgggcctcggccacgggccgcagcggcaccgtgctggcggcggcgggggccgtggaggtgctgggggcggaggcgggcttggccacgcccccgcgacgggacgttgtggactgggaaggcgcctgggacgaagacgacggcggcgcgttcgagggggacggggtgctgtaacgggccgggacggggcggggcgcttgtgaaacccgaagacgcaataaacggcaacgacctgattaagttttgcagtagcgttgtttattcgaggggcgggagggggcgaggggcgggagggggcgaggggcgggagggggcgaggggcgggagggggcgaggggcgggagggggcgaggggcgggagggggcgaggggcgggagggggcgaggggcgggagggggcgaggggcgggagggggcgaggggcgggagggggcgaggggcgggagggggcgaggggcgggagggggcgaggggcgggagggggcgaggggcgggagggggcgaggggcgggagggggcgaggggcgggagggggcgaggggcgggagggggcgaggggcgggagggggcgaggggcgggagggggcgaggggcggtggtggtgcgcgggcgcccccggagggtttggatctctgacctgagattggcggcactgaggtagagatgcccgaacccccccgagggagcgcgggacgcggctggggagggctggggctggggagggctggggccggggagggctggggccggggagggctggggccggggagggctggggccggggagggctggggccggggagggctggggctggggagggctggggctggggaggggcggtggtgtgtagcaggagcggtgtgttgcgccggggtacgtctggaggagcgggaggtgcgcggtgacgtgtggatgaggaacaggagttgttgcgcggtgagttgtcgctgtgagttgtgttgttgggcaggtgtggtggatgacgtgacgtgtgacgtgcggattgcgccgtgctttgttggtgttgttttacctgtggcagcccgggccccccgcgggcgcgcgcgcgcgcaaaaaaggcgggcggcggtccgggcggcgtgcgcgcgcgcggcgggcgtggggggcggggccgcgggagcgggggaggagcgggggaggagcggggggaggagcggggggaggagcggggggaggagcggggggaggagcggggggaggagcggggggaggagcggggggaggagcggggggaggagcggggggaggagcggggggaggagcggggggaggagcggggggaggagcggggggaggagcggggggaggagcggggggaggagcgggggaggagcggccagaccccggaaacgggccccccccaaaacacaccccccgggggtcgcgcgcggccctttaaaggcgggcggcgg

SEQ ID NO: 30 - protein, 240 aa, Human alphaherpesvirus 1
MARRRHRGPRRPRPPGPTGAVPTAQSQVTSTPNSEPVVRSAPAAAPPPPPASGPPPSCSLLLRQWLHVPESASDDDDDDWPDSPPPEPAPEARPTAAAPRPRSPPPGAGPGGGANPSHPPSRPFRLPPRLALRLRVTAEHLARLRLRRAGGEGAPKPPATPATPATPTRVRFSPHVRVRHLVVWASAARLARRGSWARERADRARFRRRVAEAEAVIGPCLGPEARARALARGAGPANSV